European Patent Application EP 4 545 641 A1, published April 30, 2025. Title: siRNA for Inhibiting Apolipoprotein C3 Expression. Applicant: RONA BIOSCIENCE, LIMITED. The sequence listing filed with the application follows.

SEQUENCE LISTING (1681 sequences)

SEQ ID NO: 1 - RNA, 19 nt, synthetic construct
  source 1..19: mol_type = other RNA
aggcagctgctccaggaat

SEQ ID NO: 2 - RNA, 19 nt, synthetic construct
  source 1..19: mol_type = other RNA
ggcagctgctccaggaaca

SEQ ID NO: 3 - RNA, 19 nt, synthetic construct
  source 1..19: mol_type = other RNA
gcagctgctccaggaacaa

SEQ ID NO: 4 - RNA, 19 nt, synthetic construct
  source 1..19: mol_type = other RNA
cagctgctccaggaacaga

SEQ ID NO: 5 - RNA, 19 nt, synthetic construct
  source 1..19: mol_type = other RNA
agctgctccaggaacagaa

SEQ ID NO: 6 - RNA, 19 nt, synthetic construct
  source 1..19: mol_type = other RNA
gctgctccaggaacagaga

SEQ ID NO: 7 - RNA, 19 nt, synthetic construct
  source 1..19: mol_type = other RNA
tgctccaggaacagaggta

SEQ ID NO: 8 - RNA, 19 nt, synthetic construct
  source 1..19: mol_type = other RNA
caggaacagaggtgccata

SEQ ID NO: 9 - RNA, 19 nt, synthetic construct
  source 1..19: mol_type = other RNA
aggaacagaggtgccatgt

SEQ ID NO: 10 - RNA, 19 nt, synthetic construct
  source 1..19: mol_type = other RNA
ggaacagaggtgccatgca

SEQ ID NO: 11 - RNA, 19 nt, synthetic construct
  source 1..19: mol_type = other RNA
gaacagaggtgccatgcaa

SEQ ID NO: 12 - RNA, 19 nt, synthetic construct
  source 1..19: mol_type = other RNA
aacagaggtgccatgcagt

SEQ ID NO: 13 - RNA, 19 nt, synthetic construct
  source 1..19: mol_type = other RNA
catgcagccccgggtactt

SEQ ID NO: 14 - RNA, 19 nt, synthetic construct
  source 1..19: mol_type = other RNA
atgcagccccgggtactct

SEQ ID NO: 15 - RNA, 19 nt, synthetic construct
  source 1..19: mol_type = other RNA
tgcagccccgggtactcct

SEQ ID NO: 16 - RNA, 19 nt, synthetic construct
  source 1..19: mol_type = other RNA
gcagccccgggtactcctt

SEQ ID NO: 17 - RNA, 19 nt, synthetic construct
  source 1..19: mol_type = other RNA
cagccccgggtactcctta

SEQ ID NO: 18 - RNA, 19 nt, synthetic construct
  source 1..19: mol_type = other RNA
agccccgggtactccttgt

SEQ ID NO: 19 - RNA, 19 nt, synthetic construct
  source 1..19: mol_type = other RNA
gccccgggtactccttgtt

SEQ ID NO: 20 - RNA, 19 nt, synthetic construct
  source 1..19: mol_type = other RNA
ccccgggtactccttgtta

SEQ ID NO: 21 - RNA, 19 nt, synthetic construct
  source 1..19: mol_type = other RNA
cccgggtactccttgttgt

SEQ ID NO: 22 - RNA, 19 nt, synthetic construct
  source 1..19: mol_type = other RNA
ccgggtactccttgttgtt

SEQ ID NO: 23 - RNA, 19 nt, synthetic construct
  source 1..19: mol_type = other RNA
cgggtactccttgttgtta

SEQ ID NO: 24 - RNA, 19 nt, synthetic construct
  source 1..19: mol_type = other RNA
gggtactccttgttgttgt

SEQ ID NO: 25 - RNA, 19 nt, synthetic construct
  source 1..19: mol_type = other RNA
ggtactccttgttgttgct

SEQ ID NO: 26 - RNA, 19 nt, synthetic construct
  source 1..19: mol_type = other RNA
gtactccttgttgttgcct

SEQ ID NO: 27 - RNA, 19 nt, synthetic construct
  source 1..19: mol_type = other RNA
actccttgttgttgccctt

SEQ ID NO: 28 - RNA, 19 nt, synthetic construct
  source 1..19: mol_type = other RNA
ctccttgttgttgccctct

SEQ ID NO: 29 - RNA, 19 nt, synthetic construct
  source 1..19: mol_type = other RNA
tccttgttgttgccctcct

SEQ ID NO: 30 - RNA, 19 nt, synthetic construct
  source 1..19: mol_type = other RNA
ccttgttgttgccctccta

SEQ ID NO: 31 - RNA, 19 nt, synthetic construct
  source 1..19: mol_type = other RNA
cttgttgttgccctcctga

SEQ ID NO: 32 - RNA, 19 nt, synthetic construct
  source 1..19: mol_type = other RNA
ttgttgttgccctcctggt

SEQ ID NO: 33 - RNA, 19 nt, synthetic construct
  source 1..19: mol_type = other RNA
tgttgttgccctcctggca

SEQ ID NO: 34 - RNA, 19 nt, synthetic construct
  source 1..19: mol_type = other RNA
gccctcctggcgctcctga

SEQ ID NO: 35 - RNA, 19 nt, synthetic construct
  source 1..19: mol_type = other RNA
tcctggcgctcctggcctt

SEQ ID NO: 36 - RNA, 19 nt, synthetic construct
  source 1..19: mol_type = other RNA
ctggcgctcctggcctcta

SEQ ID NO: 37 - RNA, 19 nt, synthetic construct
  source 1..19: mol_type = other RNA
tggcgctcctggcctctgt

SEQ ID NO: 38 - RNA, 19 nt, synthetic construct
  source 1..19: mol_type = other RNA
ggcgctcctggcctctgct

SEQ ID NO: 39 - RNA, 19 nt, synthetic construct
  source 1..19: mol_type = other RNA
gcgctcctggcctctgcct

SEQ ID NO: 40 - RNA, 19 nt, synthetic construct
  source 1..19: mol_type = other RNA
ctggcctctgcccgagctt

SEQ ID NO: 41 - RNA, 19 nt, synthetic construct
  source 1..19: mol_type = other RNA
tggcctctgcccgagcttt

SEQ ID NO: 42 - RNA, 19 nt, synthetic construct
  source 1..19: mol_type = other RNA
ggcctctgcccgagcttca

SEQ ID NO: 43 - RNA, 19 nt, synthetic construct
  source 1..19: mol_type = other RNA
gcctctgcccgagcttcaa

SEQ ID NO: 44 - RNA, 19 nt, synthetic construct
  source 1..19: mol_type = other RNA
cctctgcccgagcttcaga

SEQ ID NO: 45 - RNA, 19 nt, synthetic construct
  source 1..19: mol_type = other RNA
ctctgcccgagcttcagaa

SEQ ID NO: 46 - RNA, 19 nt, synthetic construct
  source 1..19: mol_type = other RNA
tctgcccgagcttcagaga

SEQ ID NO: 47 - RNA, 19 nt, synthetic construct
  source 1..19: mol_type = other RNA
ctgcccgagcttcagaggt

SEQ ID NO: 48 - RNA, 19 nt, synthetic construct
  source 1..19: mol_type = other RNA
tgcccgagcttcagaggct

SEQ ID NO: 49 - RNA, 19 nt, synthetic construct
  source 1..19: mol_type = other RNA
agcttcagaggccgaggat

SEQ ID NO: 50 - RNA, 19 nt, synthetic construct
  source 1..19: mol_type = other RNA
gcttcagaggccgaggata

SEQ ID NO: 51 - RNA, 19 nt, synthetic construct
  source 1..19: mol_type = other RNA
cttcagaggccgaggatgt

SEQ ID NO: 52 - RNA, 19 nt, synthetic construct
  source 1..19: mol_type = other RNA
ttcagaggccgaggatgct

SEQ ID NO: 53 - RNA, 19 nt, synthetic construct
  source 1..19: mol_type = other RNA
tcagaggccgaggatgcct

SEQ ID NO: 54 - RNA, 19 nt, synthetic construct
  source 1..19: mol_type = other RNA
cagaggccgaggatgcctt

SEQ ID NO: 55 - RNA, 19 nt, synthetic construct
  source 1..19: mol_type = other RNA
agaggccgaggatgcctct

SEQ ID NO: 56 - RNA, 19 nt, synthetic construct
  source 1..19: mol_type = other RNA
gaggccgaggatgcctcct

SEQ ID NO: 57 - RNA, 19 nt, synthetic construct
  source 1..19: mol_type = other RNA
ggccgaggatgcctccctt

SEQ ID NO: 58 - RNA, 19 nt, synthetic construct
  source 1..19: mol_type = other RNA
gccgaggatgcctcccttt

SEQ ID NO: 59 - RNA, 19 nt, synthetic construct
  source 1..19: mol_type = other RNA
ccgaggatgcctcccttct

SEQ ID NO: 60 - RNA, 19 nt, synthetic construct
  source 1..19: mol_type = other RNA
cgaggatgcctcccttctt

SEQ ID NO: 61 - RNA, 19 nt, synthetic construct
  source 1..19: mol_type = other RNA
gaggatgcctcccttctca

SEQ ID NO: 62 - RNA, 19 nt, synthetic construct
  source 1..19: mol_type = other RNA
aggatgcctcccttctcaa

SEQ ID NO: 63 - RNA, 19 nt, synthetic construct
  source 1..19: mol_type = other RNA
ggatgcctcccttctcagt

SEQ ID NO: 64 - RNA, 19 nt, synthetic construct
  source 1..19: mol_type = other RNA
gatgcctcccttctcagct

SEQ ID NO: 65 - RNA, 19 nt, synthetic construct
  source 1..19: mol_type = other RNA
atgcctcccttctcagctt

SEQ ID NO: 66 - RNA, 19 nt, synthetic construct
  source 1..19: mol_type = other RNA
tgcctcccttctcagcttt

SEQ ID NO: 67 - RNA, 19 nt, synthetic construct
  source 1..19: mol_type = other RNA
gcctcccttctcagcttca

SEQ ID NO: 68 - RNA, 19 nt, synthetic construct
  source 1..19: mol_type = other RNA
cctcccttctcagcttcat

SEQ ID NO: 69 - RNA, 19 nt, synthetic construct
  source 1..19: mol_type = other RNA
ctcccttctcagcttcata

SEQ ID NO: 70 - RNA, 19 nt, synthetic construct
  source 1..19: mol_type = other RNA
tcccttctcagcttcatgt

SEQ ID NO: 71 - RNA, 19 nt, synthetic construct
  source 1..19: mol_type = other RNA
cccttctcagcttcatgca

SEQ ID NO: 72 - RNA, 19 nt, synthetic construct
  source 1..19: mol_type = other RNA
ccttctcagcttcatgcaa

SEQ ID NO: 73 - RNA, 19 nt, synthetic construct
  source 1..19: mol_type = other RNA
cttctcagcttcatgcaga

SEQ ID NO: 74 - RNA, 19 nt, synthetic construct
  source 1..19: mol_type = other RNA
ttctcagcttcatgcagga

SEQ ID NO: 75 - RNA, 19 nt, synthetic construct
  source 1..19: mol_type = other RNA
tctcagcttcatgcagggt

SEQ ID NO: 76 - RNA, 19 nt, synthetic construct
  source 1..19: mol_type = other RNA
ctcagcttcatgcagggtt

SEQ ID NO: 77 - RNA, 19 nt, synthetic construct
  source 1..19: mol_type = other RNA
tcagcttcatgcagggtta

SEQ ID NO: 78 - RNA, 19 nt, synthetic construct
  source 1..19: mol_type = other RNA
cagcttcatgcagggttat

SEQ ID NO: 79 - RNA, 19 nt, synthetic construct
  source 1..19: mol_type = other RNA
agcttcatgcagggttaca

SEQ ID NO: 80 - RNA, 19 nt, synthetic construct
  source 1..19: mol_type = other RNA
gcttcatgcagggttacat

SEQ ID NO: 81 - RNA, 19 nt, synthetic construct
  source 1..19: mol_type = other RNA
cttcatgcagggttacata

SEQ ID NO: 82 - RNA, 19 nt, synthetic construct
  source 1..19: mol_type = other RNA
ttcatgcagggttacatga

SEQ ID NO: 83 - RNA, 19 nt, synthetic construct
  source 1..19: mol_type = other RNA
tcatgcagggttacatgaa

SEQ ID NO: 84 - RNA, 19 nt, synthetic construct
  source 1..19: mol_type = other RNA
catgcagggttacatgaaa

SEQ ID NO: 85 - RNA, 19 nt, synthetic construct
  source 1..19: mol_type = other RNA
atgcagggttacatgaagt

SEQ ID NO: 86 - RNA, 19 nt, synthetic construct
  source 1..19: mol_type = other RNA
tgcagggttacatgaagca

SEQ ID NO: 87 - RNA, 19 nt, synthetic construct
  source 1..19: mol_type = other RNA
gcagggttacatgaagcat

SEQ ID NO: 88 - RNA, 19 nt, synthetic construct
  source 1..19: mol_type = other RNA
cagggttacatgaagcaca

SEQ ID NO: 89 - RNA, 19 nt, synthetic construct
  source 1..19: mol_type = other RNA
agggttacatgaagcacgt

SEQ ID NO: 90 - RNA, 19 nt, synthetic construct
  source 1..19: mol_type = other RNA
gggttacatgaagcacgct

SEQ ID NO: 91 - RNA, 19 nt, synthetic construct
  source 1..19: mol_type = other RNA
gttacatgaagcacgccat

SEQ ID NO: 92 - RNA, 19 nt, synthetic construct
  source 1..19: mol_type = other RNA
acatgaagcacgccaccaa

SEQ ID NO: 93 - RNA, 19 nt, synthetic construct
  source 1..19: mol_type = other RNA
catgaagcacgccaccaaa

SEQ ID NO: 94 - RNA, 19 nt, synthetic construct
  source 1..19: mol_type = other RNA
atgaagcacgccaccaaga

SEQ ID NO: 95 - RNA, 19 nt, synthetic construct
  source 1..19: mol_type = other RNA
tgaagcacgccaccaagat

SEQ ID NO: 96 - RNA, 19 nt, synthetic construct
  source 1..19: mol_type = other RNA
gaagcacgccaccaagact

SEQ ID NO: 97 - RNA, 19 nt, synthetic construct
  source 1..19: mol_type = other RNA
aagcacgccaccaagacca

SEQ ID NO: 98 - RNA, 19 nt, synthetic construct
  source 1..19: mol_type = other RNA
agcacgccaccaagaccgt

SEQ ID NO: 99 - RNA, 19 nt, synthetic construct
  source 1..19: mol_type = other RNA
gcacgccaccaagaccgct

SEQ ID NO: 100 - RNA, 19 nt, synthetic construct
  source 1..19: mol_type = other RNA
cgccaccaagaccgccaaa

SEQ ID NO: 101 - RNA, 19 nt, synthetic construct
  source 1..19: mol_type = other RNA
gccaccaagaccgccaaga

SEQ ID NO: 102 - RNA, 19 nt, synthetic construct
  source 1..19: mol_type = other RNA
ccaccaagaccgccaagga

SEQ ID NO: 103 - RNA, 19 nt, synthetic construct
  source 1..19: mol_type = other RNA
caccaagaccgccaaggat

SEQ ID NO: 104 - RNA, 19 nt, synthetic construct
  source 1..19: mol_type = other RNA
accaagaccgccaaggata

SEQ ID NO: 105 - RNA, 19 nt, synthetic construct
  source 1..19: mol_type = other RNA
ccaagaccgccaaggatgt

SEQ ID NO: 106 - RNA, 19 nt, synthetic construct
  source 1..19: mol_type = other RNA
caagaccgccaaggatgca

SEQ ID NO: 107 - RNA, 19 nt, synthetic construct
  source 1..19: mol_type = other RNA
aagaccgccaaggatgcat

SEQ ID NO: 108 - RNA, 19 nt, synthetic construct
  source 1..19: mol_type = other RNA
agaccgccaaggatgcact

SEQ ID NO: 109 - RNA, 19 nt, synthetic construct
  source 1..19: mol_type = other RNA
gaccgccaaggatgcacta

SEQ ID NO: 110 - RNA, 19 nt, synthetic construct
  source 1..19: mol_type = other RNA
accgccaaggatgcactga

SEQ ID NO: 111 - RNA, 19 nt, synthetic construct
  source 1..19: mol_type = other RNA
ccgccaaggatgcactgaa

SEQ ID NO: 112 - RNA, 19 nt, synthetic construct
  source 1..19: mol_type = other RNA
cgccaaggatgcactgagt

SEQ ID NO: 113 - RNA, 19 nt, synthetic construct
  source 1..19: mol_type = other RNA
gccaaggatgcactgagca

SEQ ID NO: 114 - RNA, 19 nt, synthetic construct
  source 1..19: mol_type = other RNA
ccaaggatgcactgagcaa

SEQ ID NO: 115 - RNA, 19 nt, synthetic construct
  source 1..19: mol_type = other RNA
caaggatgcactgagcagt

SEQ ID NO: 116 - RNA, 19 nt, synthetic construct
  source 1..19: mol_type = other RNA
aaggatgcactgagcagca

SEQ ID NO: 117 - RNA, 19 nt, synthetic construct
  source 1..19: mol_type = other RNA
aggatgcactgagcagcgt

SEQ ID NO: 118 - RNA, 19 nt, synthetic construct
  source 1..19: mol_type = other RNA
ggatgcactgagcagcgta

SEQ ID NO: 119 - RNA, 19 nt, synthetic construct
  source 1..19: mol_type = other RNA
gatgcactgagcagcgtgt

SEQ ID NO: 120 - RNA, 19 nt, synthetic construct
  source 1..19: mol_type = other RNA
atgcactgagcagcgtgca

SEQ ID NO: 121 - RNA, 19 nt, synthetic construct
  source 1..19: mol_type = other RNA
tgcactgagcagcgtgcaa

SEQ ID NO: 122 - RNA, 19 nt, synthetic construct
  source 1..19: mol_type = other RNA
gcactgagcagcgtgcaga

SEQ ID NO: 123 - RNA, 19 nt, synthetic construct
  source 1..19: mol_type = other RNA
cactgagcagcgtgcagga

SEQ ID NO: 124 - RNA, 19 nt, synthetic construct
  source 1..19: mol_type = other RNA
actgagcagcgtgcaggaa

SEQ ID NO: 125 - RNA, 19 nt, synthetic construct
  source 1..19: mol_type = other RNA
ctgagcagcgtgcaggagt

SEQ ID NO: 126 - RNA, 19 nt, synthetic construct
  source 1..19: mol_type = other RNA
tgagcagcgtgcaggagtt

SEQ ID NO: 127 - RNA, 19 nt, synthetic construct
  source 1..19: mol_type = other RNA
gagcagcgtgcaggagtct

SEQ ID NO: 128 - RNA, 19 nt, synthetic construct
  source 1..19: mol_type = other RNA
agcagcgtgcaggagtcct

SEQ ID NO: 129 - RNA, 19 nt, synthetic construct
  source 1..19: mol_type = other RNA
gcagcgtgcaggagtccca

SEQ ID NO: 130 - RNA, 19 nt, synthetic construct
  source 1..19: mol_type = other RNA
cagcgtgcaggagtcccaa

SEQ ID NO: 131 - RNA, 19 nt, synthetic construct
  source 1..19: mol_type = other RNA
agcgtgcaggagtcccaga

SEQ ID NO: 132 - RNA, 19 nt, synthetic construct
  source 1..19: mol_type = other RNA
gcgtgcaggagtcccaggt

SEQ ID NO: 133 - RNA, 19 nt, synthetic construct
  source 1..19: mol_type = other RNA
cgtgcaggagtcccaggta

SEQ ID NO: 134 - RNA, 19 nt, synthetic construct
  source 1..19: mol_type = other RNA
gtgcaggagtcccaggtga

SEQ ID NO: 135 - RNA, 19 nt, synthetic construct
  source 1..19: mol_type = other RNA
tgcaggagtcccaggtggt

SEQ ID NO: 136 - RNA, 19 nt, synthetic construct
  source 1..19: mol_type = other RNA
gtcccaggtggcccagcaa

SEQ ID NO: 137 - RNA, 19 nt, synthetic construct
  source 1..19: mol_type = other RNA
tcccaggtggcccagcaga

SEQ ID NO: 138 - RNA, 19 nt, synthetic construct
  source 1..19: mol_type = other RNA
cccaggtggcccagcaggt

SEQ ID NO: 139 - RNA, 19 nt, synthetic construct
  source 1..19: mol_type = other RNA
ccaggtggcccagcaggct

SEQ ID NO: 140 - RNA, 19 nt, synthetic construct
  source 1..19: mol_type = other RNA
caggtggcccagcaggcca

SEQ ID NO: 141 - RNA, 19 nt, synthetic construct
  source 1..19: mol_type = other RNA
aggtggcccagcaggccaa

SEQ ID NO: 142 - RNA, 19 nt, synthetic construct
  source 1..19: mol_type = other RNA
ggtggcccagcaggccaga

SEQ ID NO: 143 - RNA, 19 nt, synthetic construct
  source 1..19: mol_type = other RNA
gtggcccagcaggccagga

SEQ ID NO: 144 - RNA, 19 nt, synthetic construct
  source 1..19: mol_type = other RNA
gcaggccaggggctgggta

SEQ ID NO: 145 - RNA, 19 nt, synthetic construct
  source 1..19: mol_type = other RNA
caggccaggggctgggtga

SEQ ID NO: 146 - RNA, 19 nt, synthetic construct
  source 1..19: mol_type = other RNA
aggccaggggctgggtgat

SEQ ID NO: 147 - RNA, 19 nt, synthetic construct
  source 1..19: mol_type = other RNA
ggccaggggctgggtgact

SEQ ID NO: 148 - RNA, 19 nt, synthetic construct
  source 1..19: mol_type = other RNA
gccaggggctgggtgacca

SEQ ID NO: 149 - RNA, 19 nt, synthetic construct
  source 1..19: mol_type = other RNA
ccaggggctgggtgaccga

SEQ ID NO: 150 - RNA, 19 nt, synthetic construct
  source 1..19: mol_type = other RNA
caggggctgggtgaccgat

SEQ ID NO: 151 - RNA, 19 nt, synthetic construct
  source 1..19: mol_type = other RNA
aggggctgggtgaccgata

SEQ ID NO: 152 - RNA, 19 nt, synthetic construct
  source 1..19: mol_type = other RNA
ggggctgggtgaccgatga

SEQ ID NO: 153 - RNA, 19 nt, synthetic construct
  source 1..19: mol_type = other RNA
gggctgggtgaccgatggt

SEQ ID NO: 154 - RNA, 19 nt, synthetic construct
  source 1..19: mol_type = other RNA
ggctgggtgaccgatggct

SEQ ID NO: 155 - RNA, 19 nt, synthetic construct
  source 1..19: mol_type = other RNA
gctgggtgaccgatggctt

SEQ ID NO: 156 - RNA, 19 nt, synthetic construct
  source 1..19: mol_type = other RNA
ctgggtgaccgatggcttt

SEQ ID NO: 157 - RNA, 19 nt, synthetic construct
  source 1..19: mol_type = other RNA
tgggtgaccgatggcttca

SEQ ID NO: 158 - RNA, 19 nt, synthetic construct
  source 1..19: mol_type = other RNA
gggtgaccgatggcttcaa

SEQ ID NO: 159 - RNA, 19 nt, synthetic construct
  source 1..19: mol_type = other RNA
ggtgaccgatggcttcagt

SEQ ID NO: 160 - RNA, 19 nt, synthetic construct
  source 1..19: mol_type = other RNA
gtgaccgatggcttcagtt

SEQ ID NO: 161 - RNA, 19 nt, synthetic construct
  source 1..19: mol_type = other RNA
tgaccgatggcttcagttt

SEQ ID NO: 162 - RNA, 19 nt, synthetic construct
  source 1..19: mol_type = other RNA
gaccgatggcttcagttct

SEQ ID NO: 163 - RNA, 19 nt, synthetic construct
  source 1..19: mol_type = other RNA
accgatggcttcagttcct

SEQ ID NO: 164 - RNA, 19 nt, synthetic construct
  source 1..19: mol_type = other RNA
ccgatggcttcagttccct

SEQ ID NO: 165 - RNA, 19 nt, synthetic construct
  source 1..19: mol_type = other RNA
cgatggcttcagttcccta

SEQ ID NO: 166 - RNA, 19 nt, synthetic construct
  source 1..19: mol_type = other RNA
gatggcttcagttccctga

SEQ ID NO: 167 - RNA, 19 nt, synthetic construct
  source 1..19: mol_type = other RNA
atggcttcagttccctgaa

SEQ ID NO: 168 - RNA, 19 nt, synthetic construct
  source 1..19: mol_type = other RNA
tggcttcagttccctgaaa

SEQ ID NO: 169 - RNA, 19 nt, synthetic construct
  source 1..19: mol_type = other RNA
ggcttcagttccctgaaaa

SEQ ID NO: 170 - RNA, 19 nt, synthetic construct
  source 1..19: mol_type = other RNA
gcttcagttccctgaaaga

SEQ ID NO: 171 - RNA, 19 nt, synthetic construct
  source 1..19: mol_type = other RNA
cttcagttccctgaaagat

SEQ ID NO: 172 - RNA, 19 nt, synthetic construct
  source 1..19: mol_type = other RNA
ttcagttccctgaaagact

SEQ ID NO: 173 - RNA, 19 nt, synthetic construct
  source 1..19: mol_type = other RNA
tcagttccctgaaagacta

SEQ ID NO: 174 - RNA, 19 nt, synthetic construct
  source 1..19: mol_type = other RNA
cagttccctgaaagactat

SEQ ID NO: 175 - RNA, 19 nt, synthetic construct
  source 1..19: mol_type = other RNA
agttccctgaaagactact

SEQ ID NO: 176 - RNA, 19 nt, synthetic construct
  source 1..19: mol_type = other RNA
gttccctgaaagactacta

SEQ ID NO: 177 - RNA, 19 nt, synthetic construct
  source 1..19: mol_type = other RNA
ttccctgaaagactactga

SEQ ID NO: 178 - RNA, 19 nt, synthetic construct
  source 1..19: mol_type = other RNA
tccctgaaagactactgga

SEQ ID NO: 179 - RNA, 19 nt, synthetic construct
  source 1..19: mol_type = other RNA
ccctgaaagactactggaa

SEQ ID NO: 180 - RNA, 19 nt, synthetic construct
  source 1..19: mol_type = other RNA
cctgaaagactactggagt

SEQ ID NO: 181 - RNA, 19 nt, synthetic construct
  source 1..19: mol_type = other RNA
ctgaaagactactggagca

SEQ ID NO: 182 - RNA, 19 nt, synthetic construct
  source 1..19: mol_type = other RNA
tgaaagactactggagcat

SEQ ID NO: 183 - RNA, 19 nt, synthetic construct
  source 1..19: mol_type = other RNA
gaaagactactggagcact

SEQ ID NO: 184 - RNA, 19 nt, synthetic construct
  source 1..19: mol_type = other RNA
aaagactactggagcacca

SEQ ID NO: 185 - RNA, 19 nt, synthetic construct
  source 1..19: mol_type = other RNA
agactactggagcaccgtt

SEQ ID NO: 186 - RNA, 19 nt, synthetic construct
  source 1..19: mol_type = other RNA
gactactggagcaccgtta

SEQ ID NO: 187 - RNA, 19 nt, synthetic construct
  source 1..19: mol_type = other RNA
actactggagcaccgttaa

SEQ ID NO: 188 - RNA, 19 nt, synthetic construct
  source 1..19: mol_type = other RNA
ctactggagcaccgttaaa

SEQ ID NO: 189 - RNA, 19 nt, synthetic construct
  source 1..19: mol_type = other RNA
tactggagcaccgttaaga

SEQ ID NO: 190 - RNA, 19 nt, synthetic construct
  source 1..19: mol_type = other RNA
actggagcaccgttaagga

SEQ ID NO: 191 - RNA, 19 nt, synthetic construct
  source 1..19: mol_type = other RNA
ctggagcaccgttaaggat

SEQ ID NO: 192 - RNA, 19 nt, synthetic construct
  source 1..19: mol_type = other RNA
tggagcaccgttaaggaca

SEQ ID NO: 193 - RNA, 19 nt, synthetic construct
  source 1..19: mol_type = other RNA
ggagcaccgttaaggacaa

SEQ ID NO: 194 - RNA, 19 nt, synthetic construct
  source 1..19: mol_type = other RNA
gagcaccgttaaggacaaa

SEQ ID NO: 195 - RNA, 19 nt, synthetic construct
  source 1..19: mol_type = other RNA
agcaccgttaaggacaagt

SEQ ID NO: 196 - RNA, 19 nt, synthetic construct
  source 1..19: mol_type = other RNA
gcaccgttaaggacaagtt

SEQ ID NO: 197 - RNA, 19 nt, synthetic construct
  source 1..19: mol_type = other RNA
caccgttaaggacaagttt

SEQ ID NO: 198 - RNA, 19 nt, synthetic construct
  source 1..19: mol_type = other RNA
accgttaaggacaagttct

SEQ ID NO: 199 - RNA, 19 nt, synthetic construct
  source 1..19: mol_type = other RNA
ccgttaaggacaagttctt

SEQ ID NO: 200 - RNA, 19 nt, synthetic construct
  source 1..19: mol_type = other RNA
cgttaaggacaagttctct

SEQ ID NO: 201 - RNA, 19 nt, synthetic construct
  source 1..19: mol_type = other RNA
gttaaggacaagttctcta

SEQ ID NO: 202 - RNA, 19 nt, synthetic construct
  source 1..19: mol_type = other RNA
ttaaggacaagttctctga

SEQ ID NO: 203 - RNA, 19 nt, synthetic construct
  source 1..19: mol_type = other RNA
taaggacaagttctctgaa

SEQ ID NO: 204 - RNA, 19 nt, synthetic construct
  source 1..19: mol_type = other RNA
aaggacaagttctctgagt

SEQ ID NO: 205 - RNA, 19 nt, synthetic construct
  source 1..19: mol_type = other RNA
aggacaagttctctgagtt

SEQ ID NO: 206 - RNA, 19 nt, synthetic construct
  source 1..19: mol_type = other RNA
ggacaagttctctgagttt

SEQ ID NO: 207 - RNA, 19 nt, synthetic construct
  source 1..19: mol_type = other RNA
gacaagttctctgagttct

SEQ ID NO: 208 - RNA, 19 nt, synthetic construct
  source 1..19: mol_type = other RNA
acaagttctctgagttcta

SEQ ID NO: 209 - RNA, 19 nt, synthetic construct
  source 1..19: mol_type = other RNA
caagttctctgagttctga

SEQ ID NO: 210 - RNA, 19 nt, synthetic construct
  source 1..19: mol_type = other RNA
aagttctctgagttctgga

SEQ ID NO: 211 - RNA, 19 nt, synthetic construct
  source 1..19: mol_type = other RNA
agttctctgagttctggga

SEQ ID NO: 212 - RNA, 19 nt, synthetic construct
  source 1..19: mol_type = other RNA
gttctctgagttctgggat

SEQ ID NO: 213 - RNA, 19 nt, synthetic construct
  source 1..19: mol_type = other RNA
ttctctgagttctgggatt

SEQ ID NO: 214 - RNA, 19 nt, synthetic construct
  source 1..19: mol_type = other RNA
tctctgagttctgggattt

SEQ ID NO: 215 - RNA, 19 nt, synthetic construct
  source 1..19: mol_type = other RNA
ctctgagttctgggattta

SEQ ID NO: 216 - RNA, 19 nt, synthetic construct
  source 1..19: mol_type = other RNA
tctgagttctgggatttga

SEQ ID NO: 217 - RNA, 19 nt, synthetic construct
  source 1..19: mol_type = other RNA
ctgagttctgggatttgga

SEQ ID NO: 218 - RNA, 19 nt, synthetic construct
  source 1..19: mol_type = other RNA
tgagttctgggatttggat

SEQ ID NO: 219 - RNA, 19 nt, synthetic construct
  source 1..19: mol_type = other RNA
gagttctgggatttggact

SEQ ID NO: 220 - RNA, 19 nt, synthetic construct
  source 1..19: mol_type = other RNA
agttctgggatttggacct

SEQ ID NO: 221 - RNA, 19 nt, synthetic construct
  source 1..19: mol_type = other RNA
ttctgggatttggacccta

SEQ ID NO: 222 - RNA, 19 nt, synthetic construct
  source 1..19: mol_type = other RNA
tctgggatttggaccctga

SEQ ID NO: 223 - RNA, 19 nt, synthetic construct
  source 1..19: mol_type = other RNA
ctgggatttggaccctgaa

SEQ ID NO: 224 - RNA, 19 nt, synthetic construct
  source 1..19: mol_type = other RNA
tgggatttggaccctgaga

SEQ ID NO: 225 - RNA, 19 nt, synthetic construct
  source 1..19: mol_type = other RNA
gggatttggaccctgaggt

SEQ ID NO: 226 - RNA, 19 nt, synthetic construct
  source 1..19: mol_type = other RNA
ggatttggaccctgaggtt

SEQ ID NO: 227 - RNA, 19 nt, synthetic construct
  source 1..19: mol_type = other RNA
gatttggaccctgaggtca

SEQ ID NO: 228 - RNA, 19 nt, synthetic construct
  source 1..19: mol_type = other RNA
atttggaccctgaggtcaa

SEQ ID NO: 229 - RNA, 19 nt, synthetic construct
  source 1..19: mol_type = other RNA
tttggaccctgaggtcaga

SEQ ID NO: 230 - RNA, 19 nt, synthetic construct
  source 1..19: mol_type = other RNA
ttggaccctgaggtcagat

SEQ ID NO: 231 - RNA, 19 nt, synthetic construct
  source 1..19: mol_type = other RNA
tggaccctgaggtcagact

SEQ ID NO: 232 - RNA, 19 nt, synthetic construct
  source 1..19: mol_type = other RNA
ggaccctgaggtcagacca

SEQ ID NO: 233 - RNA, 19 nt, synthetic construct
  source 1..19: mol_type = other RNA
gaccctgaggtcagaccaa

SEQ ID NO: 234 - RNA, 19 nt, synthetic construct
  source 1..19: mol_type = other RNA
accctgaggtcagaccaat

SEQ ID NO: 235 - RNA, 19 nt, synthetic construct
  source 1..19: mol_type = other RNA
ccctgaggtcagaccaact

SEQ ID NO: 236 - RNA, 19 nt, synthetic construct
  source 1..19: mol_type = other RNA
cctgaggtcagaccaactt

SEQ ID NO: 237 - RNA, 19 nt, synthetic construct
  source 1..19: mol_type = other RNA
ctgaggtcagaccaacttt

SEQ ID NO: 238 - RNA, 19 nt, synthetic construct
  source 1..19: mol_type = other RNA
tgaggtcagaccaacttca

SEQ ID NO: 239 - RNA, 19 nt, synthetic construct
  source 1..19: mol_type = other RNA
gaggtcagaccaacttcaa

SEQ ID NO: 240 - RNA, 19 nt, synthetic construct
  source 1..19: mol_type = other RNA
aggtcagaccaacttcagt

SEQ ID NO: 241 - RNA, 19 nt, synthetic construct
  source 1..19: mol_type = other RNA
ggtcagaccaacttcagct

SEQ ID NO: 242 - RNA, 19 nt, synthetic construct
  source 1..19: mol_type = other RNA
gtcagaccaacttcagcca

SEQ ID NO: 243 - RNA, 19 nt, synthetic construct
  source 1..19: mol_type = other RNA
ccaacttcagccgtggcta

SEQ ID NO: 244 - RNA, 19 nt, synthetic construct
  source 1..19: mol_type = other RNA
caacttcagccgtggctgt

SEQ ID NO: 245 - RNA, 19 nt, synthetic construct
  source 1..19: mol_type = other RNA
aacttcagccgtggctgct

SEQ ID NO: 246 - RNA, 19 nt, synthetic construct
  source 1..19: mol_type = other RNA
acttcagccgtggctgcct

SEQ ID NO: 247 - RNA, 19 nt, synthetic construct
  source 1..19: mol_type = other RNA
cttcagccgtggctgccta

SEQ ID NO: 248 - RNA, 19 nt, synthetic construct
  source 1..19: mol_type = other RNA
ttcagccgtggctgcctga

SEQ ID NO: 249 - RNA, 19 nt, synthetic construct
  source 1..19: mol_type = other RNA
tcagccgtggctgcctgaa

SEQ ID NO: 250 - RNA, 19 nt, synthetic construct
  source 1..19: mol_type = other RNA
cagccgtggctgcctgaga

SEQ ID NO: 251 - RNA, 19 nt, synthetic construct
  source 1..19: mol_type = other RNA
agccgtggctgcctgagat

SEQ ID NO: 252 - RNA, 19 nt, synthetic construct
  source 1..19: mol_type = other RNA
gccgtggctgcctgagact

SEQ ID NO: 253 - RNA, 19 nt, synthetic construct
  source 1..19: mol_type = other RNA
ccgtggctgcctgagacct

SEQ ID NO: 254 - RNA, 19 nt, synthetic construct
  source 1..19: mol_type = other RNA
cgtggctgcctgagacctt

SEQ ID NO: 255 - RNA, 19 nt, synthetic construct
  source 1..19: mol_type = other RNA
gtggctgcctgagacctca

SEQ ID NO: 256 - RNA, 19 nt, synthetic construct
  source 1..19: mol_type = other RNA
tggctgcctgagacctcaa

SEQ ID NO: 257 - RNA, 19 nt, synthetic construct
  source 1..19: mol_type = other RNA
ggctgcctgagacctcaat

SEQ ID NO: 258 - RNA, 19 nt, synthetic construct
  source 1..19: mol_type = other RNA
gctgcctgagacctcaata

SEQ ID NO: 259 - RNA, 19 nt, synthetic construct
  source 1..19: mol_type = other RNA
ctgcctgagacctcaatat

SEQ ID NO: 260 - RNA, 19 nt, synthetic construct
  source 1..19: mol_type = other RNA
tgcctgagacctcaatact

SEQ ID NO: 261 - RNA, 19 nt, synthetic construct
  source 1..19: mol_type = other RNA
gcctgagacctcaatacct

SEQ ID NO: 262 - RNA, 19 nt, synthetic construct
  source 1..19: mol_type = other RNA
cctgagacctcaataccct

SEQ ID NO: 263 - RNA, 19 nt, synthetic construct
  source 1..19: mol_type = other RNA
tgagacctcaataccccaa

SEQ ID NO: 264 - RNA, 19 nt, synthetic construct
  source 1..19: mol_type = other RNA
gagacctcaataccccaaa

SEQ ID NO: 265 - RNA, 19 nt, synthetic construct
  source 1..19: mol_type = other RNA
agacctcaataccccaagt

SEQ ID NO: 266 - RNA, 19 nt, synthetic construct
  source 1..19: mol_type = other RNA
gacctcaataccccaagtt

SEQ ID NO: 267 - RNA, 19 nt, synthetic construct
  source 1..19: mol_type = other RNA
acctcaataccccaagtct

SEQ ID NO: 268 - RNA, 19 nt, synthetic construct
  source 1..19: mol_type = other RNA
cctcaataccccaagtcca

SEQ ID NO: 269 - RNA, 19 nt, synthetic construct
  source 1..19: mol_type = other RNA
ctcaataccccaagtccat

SEQ ID NO: 270 - RNA, 19 nt, synthetic construct
  source 1..19: mol_type = other RNA
tcaataccccaagtccact

SEQ ID NO: 271 - RNA, 19 nt, synthetic construct
  source 1..19: mol_type = other RNA
caataccccaagtccacct

SEQ ID NO: 272 - RNA, 19 nt, synthetic construct
  source 1..19: mol_type = other RNA
aataccccaagtccaccta

SEQ ID NO: 273 - RNA, 19 nt, synthetic construct
  source 1..19: mol_type = other RNA
ataccccaagtccacctgt

SEQ ID NO: 274 - RNA, 19 nt, synthetic construct
  source 1..19: mol_type = other RNA
taccccaagtccacctgct

SEQ ID NO: 275 - RNA, 19 nt, synthetic construct
  source 1..19: mol_type = other RNA
ccccaagtccacctgccta

SEQ ID NO: 276 - RNA, 19 nt, synthetic construct
  source 1..19: mol_type = other RNA
cccaagtccacctgcctat

SEQ ID NO: 277 - RNA, 19 nt, synthetic construct
  source 1..19: mol_type = other RNA
ccaagtccacctgcctatt

SEQ ID NO: 278 - RNA, 19 nt, synthetic construct
  source 1..19: mol_type = other RNA
caagtccacctgcctatct

SEQ ID NO: 279 - RNA, 19 nt, synthetic construct
  source 1..19: mol_type = other RNA
aagtccacctgcctatcca

SEQ ID NO: 280 - RNA, 19 nt, synthetic construct
  source 1..19: mol_type = other RNA
agtccacctgcctatccat

SEQ ID NO: 281 - RNA, 19 nt, synthetic construct
  source 1..19: mol_type = other RNA
gtccacctgcctatccatt

SEQ ID NO: 282 - RNA, 19 nt, synthetic construct
  source 1..19: mol_type = other RNA
tccacctgcctatccatct

SEQ ID NO: 283 - RNA, 19 nt, synthetic construct
  source 1..19: mol_type = other RNA
ccacctgcctatccatcct

SEQ ID NO: 284 - RNA, 19 nt, synthetic construct
  source 1..19: mol_type = other RNA
cacctgcctatccatccta

SEQ ID NO: 285 - RNA, 19 nt, synthetic construct
  source 1..19: mol_type = other RNA
acctgcctatccatcctgt

SEQ ID NO: 286 - RNA, 19 nt, synthetic construct
  source 1..19: mol_type = other RNA
cctgcctatccatcctgca

SEQ ID NO: 287 - RNA, 19 nt, synthetic construct
  source 1..19: mol_type = other RNA
ctgcctatccatcctgcga

SEQ ID NO: 288 - RNA, 19 nt, synthetic construct
  source 1..19: mol_type = other RNA
tgcctatccatcctgcgaa

SEQ ID NO: 289 - RNA, 19 nt, synthetic construct
  source 1..19: mol_type = other RNA
gcctatccatcctgcgagt

SEQ ID NO: 290 - RNA, 19 nt, synthetic construct
  source 1..19: mol_type = other RNA
cctatccatcctgcgagct

SEQ ID NO: 291 - RNA, 19 nt, synthetic construct
  source 1..19: mol_type = other RNA
ctatccatcctgcgagctt

SEQ ID NO: 292 - RNA, 19 nt, synthetic construct
  source 1..19: mol_type = other RNA
tatccatcctgcgagctct

SEQ ID NO: 293 - RNA, 19 nt, synthetic construct
  source 1..19: mol_type = other RNA
atccatcctgcgagctcct

SEQ ID NO: 294 - RNA, 19 nt, synthetic construct
  source 1..19: mol_type = other RNA
tccatcctgcgagctcctt

SEQ ID NO: 295 - RNA, 19 nt, synthetic construct
  source 1..19: mol_type = other RNA
ccatcctgcgagctcctta

SEQ ID NO: 296 - RNA, 19 nt, synthetic construct
  source 1..19: mol_type = other RNA
catcctgcgagctccttga

SEQ ID NO: 297 - RNA, 19 nt, synthetic construct
  source 1..19: mol_type = other RNA
atcctgcgagctccttgga

SEQ ID NO: 298 - RNA, 19 nt, synthetic construct
  source 1..19: mol_type = other RNA
tcctgcgagctccttgggt

SEQ ID NO: 299 - RNA, 19 nt, synthetic construct
  source 1..19: mol_type = other RNA
cctgcgagctccttgggtt

SEQ ID NO: 300 - RNA, 19 nt, synthetic construct
  source 1..19: mol_type = other RNA
ctgcgagctccttgggtct

SEQ ID NO: 301 - RNA, 19 nt, synthetic construct
  source 1..19: mol_type = other RNA
tgcgagctccttgggtcct

SEQ ID NO: 302 - RNA, 19 nt, synthetic construct
  source 1..19: mol_type = other RNA
gcgagctccttgggtccta

SEQ ID NO: 303 - RNA, 19 nt, synthetic construct
  source 1..19: mol_type = other RNA
cgagctccttgggtcctgt

SEQ ID NO: 304 - RNA, 19 nt, synthetic construct
  source 1..19: mol_type = other RNA
gagctccttgggtcctgca

SEQ ID NO: 305 - RNA, 19 nt, synthetic construct
  source 1..19: mol_type = other RNA
agctccttgggtcctgcaa

SEQ ID NO: 306 - RNA, 19 nt, synthetic construct
  source 1..19: mol_type = other RNA
gctccttgggtcctgcaat

SEQ ID NO: 307 - RNA, 19 nt, synthetic construct
  source 1..19: mol_type = other RNA
ctccttgggtcctgcaatt

SEQ ID NO: 308 - RNA, 19 nt, synthetic construct
  source 1..19: mol_type = other RNA
tccttgggtcctgcaatct

SEQ ID NO: 309 - RNA, 19 nt, synthetic construct
  source 1..19: mol_type = other RNA
ccttgggtcctgcaatctt

SEQ ID NO: 310 - RNA, 19 nt, synthetic construct
  source 1..19: mol_type = other RNA
cttgggtcctgcaatctct

SEQ ID NO: 311 - RNA, 19 nt, synthetic construct
  source 1..19: mol_type = other RNA
ttgggtcctgcaatctcca

SEQ ID NO: 312 - RNA, 19 nt, synthetic construct
  source 1..19: mol_type = other RNA
tgggtcctgcaatctccaa

SEQ ID NO: 313 - RNA, 19 nt, synthetic construct
  source 1..19: mol_type = other RNA
gggtcctgcaatctccaga

SEQ ID NO: 314 - RNA, 19 nt, synthetic construct
  source 1..19: mol_type = other RNA
ggtcctgcaatctccagga

SEQ ID NO: 315 - RNA, 19 nt, synthetic construct
  source 1..19: mol_type = other RNA
gtcctgcaatctccagggt

SEQ ID NO: 316 - RNA, 19 nt, synthetic construct
  source 1..19: mol_type = other RNA
cctgcaatctccagggcta

SEQ ID NO: 317 - RNA, 19 nt, synthetic construct
  source 1..19: mol_type = other RNA
ctgcaatctccagggctgt

SEQ ID NO: 318 - RNA, 19 nt, synthetic construct
  source 1..19: mol_type = other RNA
tgcaatctccagggctgct

SEQ ID NO: 319 - RNA, 19 nt, synthetic construct
  source 1..19: mol_type = other RNA
ctccagggctgcccctgta

SEQ ID NO: 320 - RNA, 19 nt, synthetic construct
  source 1..19: mol_type = other RNA
tccagggctgcccctgtaa

SEQ ID NO: 321 - RNA, 19 nt, synthetic construct
  source 1..19: mol_type = other RNA
ccagggctgcccctgtaga

SEQ ID NO: 322 - RNA, 19 nt, synthetic construct
  source 1..19: mol_type = other RNA
cagggctgcccctgtaggt

SEQ ID NO: 323 - RNA, 19 nt, synthetic construct
  source 1..19: mol_type = other RNA
agggctgcccctgtaggtt

SEQ ID NO: 324 - RNA, 19 nt, synthetic construct
  source 1..19: mol_type = other RNA
gggctgcccctgtaggtta

SEQ ID NO: 325 - RNA, 19 nt, synthetic construct
  source 1..19: mol_type = other RNA
ggctgcccctgtaggttgt

SEQ ID NO: 326 - RNA, 19 nt, synthetic construct
  source 1..19: mol_type = other RNA
gctgcccctgtaggttgct

SEQ ID NO: 327 - RNA, 19 nt, synthetic construct
  source 1..19: mol_type = other RNA
ctgcccctgtaggttgctt

SEQ ID NO: 328 - RNA, 19 nt, synthetic construct
  source 1..19: mol_type = other RNA
tgcccctgtaggttgctta

SEQ ID NO: 329 - RNA, 19 nt, synthetic construct
  source 1..19: mol_type = other RNA
gcccctgtaggttgcttaa

SEQ ID NO: 330 - RNA, 19 nt, synthetic construct
  source 1..19: mol_type = other RNA
cccctgtaggttgcttaaa

SEQ ID NO: 331 - RNA, 19 nt, synthetic construct
  source 1..19: mol_type = other RNA
ccctgtaggttgcttaaaa

SEQ ID NO: 332 - RNA, 19 nt, synthetic construct
  source 1..19: mol_type = other RNA
cctgtaggttgcttaaaaa

SEQ ID NO: 333 - RNA, 19 nt, synthetic construct
  source 1..19: mol_type = other RNA
ctgtaggttgcttaaaaga

SEQ ID NO: 334 - RNA, 19 nt, synthetic construct
  source 1..19: mol_type = other RNA
tgtaggttgcttaaaagga

SEQ ID NO: 335 - RNA, 19 nt, synthetic construct
  source 1..19: mol_type = other RNA
gtaggttgcttaaaaggga

SEQ ID NO: 336 - RNA, 19 nt, synthetic construct
  source 1..19: mol_type = other RNA
taggttgcttaaaagggat

SEQ ID NO: 337 - RNA, 19 nt, synthetic construct
  source 1..19: mol_type = other RNA
aggttgcttaaaagggaca

SEQ ID NO: 338 - RNA, 19 nt, synthetic construct
  source 1..19: mol_type = other RNA
ggttgcttaaaagggacaa

SEQ ID NO: 339 - RNA, 19 nt, synthetic construct
  source 1..19: mol_type = other RNA
gttgcttaaaagggacagt

SEQ ID NO: 340 - RNA, 19 nt, synthetic construct
  source 1..19: mol_type = other RNA
ttgcttaaaagggacagta

SEQ ID NO: 341 - RNA, 19 nt, synthetic construct
  source 1..19: mol_type = other RNA
tgcttaaaagggacagtat

SEQ ID NO: 342 - RNA, 19 nt, synthetic construct
  source 1..19: mol_type = other RNA
gcttaaaagggacagtatt

SEQ ID NO: 343 - RNA, 19 nt, synthetic construct
  source 1..19: mol_type = other RNA
cttaaaagggacagtattt

SEQ ID NO: 344 - RNA, 19 nt, synthetic construct
  source 1..19: mol_type = other RNA
ttaaaagggacagtattct

SEQ ID NO: 345 - RNA, 19 nt, synthetic construct
  source 1..19: mol_type = other RNA
taaaagggacagtattctt

SEQ ID NO: 346 - RNA, 19 nt, synthetic construct
  source 1..19: mol_type = other RNA
aaaagggacagtattctca

SEQ ID NO: 347 - RNA, 19 nt, synthetic construct
  source 1..19: mol_type = other RNA
aaagggacagtattctcaa

SEQ ID NO: 348 - RNA, 19 nt, synthetic construct
  source 1..19: mol_type = other RNA
aagggacagtattctcagt

SEQ ID NO: 349 - RNA, 19 nt, synthetic construct
  source 1..19: mol_type = other RNA
agggacagtattctcagta

SEQ ID NO: 350 - RNA, 19 nt, synthetic construct
  source 1..19: mol_type = other RNA
gggacagtattctcagtgt

SEQ ID NO: 351 - RNA, 19 nt, synthetic construct
  source 1..19: mol_type = other RNA
ggacagtattctcagtgct

SEQ ID NO: 352 - RNA, 19 nt, synthetic construct
  source 1..19: mol_type = other RNA
gacagtattctcagtgctt

SEQ ID NO: 353 - RNA, 19 nt, synthetic construct
  source 1..19: mol_type = other RNA
acagtattctcagtgctct

SEQ ID NO: 354 - RNA, 19 nt, synthetic construct
  source 1..19: mol_type = other RNA
cagtattctcagtgctctt

SEQ ID NO: 355 - RNA, 19 nt, synthetic construct
  source 1..19: mol_type = other RNA
agtattctcagtgctctct

SEQ ID NO: 356 - RNA, 19 nt, synthetic construct
  source 1..19: mol_type = other RNA
gtattctcagtgctctcct

SEQ ID NO: 357 - RNA, 19 nt, synthetic construct
  source 1..19: mol_type = other RNA
tattctcagtgctctccta

SEQ ID NO: 358 - RNA, 19 nt, synthetic construct
  source 1..19: mol_type = other RNA
attctcagtgctctcctat

SEQ ID NO: 359 - RNA, 19 nt, synthetic construct
  source 1..19: mol_type = other RNA
ttctcagtgctctcctact

SEQ ID NO: 360 - RNA, 19 nt, synthetic construct
  source 1..19: mol_type = other RNA
tctcagtgctctcctacct

SEQ ID NO: 361 - RNA, 19 nt, synthetic construct
  source 1..19: mol_type = other RNA
ctcagtgctctcctaccct

SEQ ID NO: 362 - RNA, 19 nt, synthetic construct
  source 1..19: mol_type = other RNA
gctctcctaccccacctca

SEQ ID NO: 363 - RNA, 19 nt, synthetic construct
  source 1..19: mol_type = other RNA
ctctcctaccccacctcat

SEQ ID NO: 364 - RNA, 19 nt, synthetic construct
  source 1..19: mol_type = other RNA
tctcctaccccacctcata

SEQ ID NO: 365 - RNA, 19 nt, synthetic construct
  source 1..19: mol_type = other RNA
ctcctaccccacctcatgt

SEQ ID NO: 366 - RNA, 19 nt, synthetic construct
  source 1..19: mol_type = other RNA
tcctaccccacctcatgct

SEQ ID NO: 367 - RNA, 19 nt, synthetic construct
  source 1..19: mol_type = other RNA
cctaccccacctcatgcct

SEQ ID NO: 368 - RNA, 19 nt, synthetic construct
  source 1..19: mol_type = other RNA
ctaccccacctcatgccta

SEQ ID NO: 369 - RNA, 19 nt, synthetic construct
  source 1..19: mol_type = other RNA
taccccacctcatgcctga

SEQ ID NO: 370 - RNA, 19 nt, synthetic construct
  source 1..19: mol_type = other RNA
cccctccaggcatgctggt

SEQ ID NO: 371 - RNA, 19 nt, synthetic construct
  source 1..19: mol_type = other RNA
ccctccaggcatgctggct

SEQ ID NO: 372 - RNA, 19 nt, synthetic construct
  source 1..19: mol_type = other RNA
cctccaggcatgctggcct

SEQ ID NO: 373 - RNA, 19 nt, synthetic construct
  source 1..19: mol_type = other RNA
ctccaggcatgctggcctt

SEQ ID NO: 374 - RNA, 19 nt, synthetic construct
  source 1..19: mol_type = other RNA
aggcatgctggcctcccaa

SEQ ID NO: 375 - RNA, 19 nt, synthetic construct
  source 1..19: mol_type = other RNA
ggcatgctggcctcccaat

SEQ ID NO: 376 - RNA, 19 nt, synthetic construct
  source 1..19: mol_type = other RNA
gcatgctggcctcccaata

SEQ ID NO: 377 - RNA, 19 nt, synthetic construct
  source 1..19: mol_type = other RNA
catgctggcctcccaataa

SEQ ID NO: 378 - RNA, 19 nt, synthetic construct
  source 1..19: mol_type = other RNA
atgctggcctcccaataaa

SEQ ID NO: 379 - RNA, 19 nt, synthetic construct
  source 1..19: mol_type = other RNA
tgctggcctcccaataaaa

SEQ ID NO: 380 - RNA, 19 nt, synthetic construct
  source 1..19: mol_type = other RNA
gctggcctcccaataaagt

SEQ ID NO: 381 - RNA, 19 nt, synthetic construct
  source 1..19: mol_type = other RNA
ctggcctcccaataaagct

SEQ ID NO: 382 - RNA, 19 nt, synthetic construct
  source 1..19: mol_type = other RNA
tggcctcccaataaagcta

SEQ ID NO: 383 - RNA, 19 nt, synthetic construct
  source 1..19: mol_type = other RNA
ggcctcccaataaagctga

SEQ ID NO: 384 - RNA, 19 nt, synthetic construct
  source 1..19: mol_type = other RNA
gcctcccaataaagctgga

SEQ ID NO: 385 - RNA, 19 nt, synthetic construct
  source 1..19: mol_type = other RNA
cctcccaataaagctggat

SEQ ID NO: 386 - RNA, 19 nt, synthetic construct
  source 1..19: mol_type = other RNA
ctcccaataaagctggaca

SEQ ID NO: 387 - RNA, 19 nt, synthetic construct
  source 1..19: mol_type = other RNA
tcccaataaagctggacaa

SEQ ID NO: 388 - RNA, 19 nt, synthetic construct
  source 1..19: mol_type = other RNA
cccaataaagctggacaaa

SEQ ID NO: 389 - RNA, 19 nt, synthetic construct
  source 1..19: mol_type = other RNA
ccaataaagctggacaaga

SEQ ID NO: 390 - RNA, 19 nt, synthetic construct
  source 1..19: mol_type = other RNA
caataaagctggacaagaa

SEQ ID NO: 391 - RNA, 19 nt, synthetic construct
  source 1..19: mol_type = other RNA
aataaagctggacaagaaa

SEQ ID NO: 392 - RNA, 19 nt, synthetic construct
  source 1..19: mol_type = other RNA
ataaagctggacaagaagt

SEQ ID NO: 393 - RNA, 19 nt, synthetic construct
  source 1..19: mol_type = other RNA
taaagctggacaagaagct

SEQ ID NO: 394 - RNA, 19 nt, synthetic construct
  source 1..19: mol_type = other RNA
aaagctggacaagaagcta

SEQ ID NO: 395 - RNA, 19 nt, synthetic construct
  source 1..19: mol_type = other RNA
aagctggacaagaagctgt

SEQ ID NO: 396 - RNA, 19 nt, synthetic construct
  source 1..19: mol_type = other RNA
agctggacaagaagctgct

SEQ ID NO: 397 - RNA, 19 nt, synthetic construct
  source 1..19: mol_type = other RNA
gctggacaagaagctgcta

SEQ ID NO: 398 - RNA, 19 nt, synthetic construct
  source 1..19: mol_type = other RNA
ctggacaagaagctgctat

SEQ ID NO: 399 - RNA, 19 nt, synthetic construct
  source 1..19: mol_type = other RNA
tggacaagaagctgctata

SEQ ID NO: 400 - RNA, 19 nt, synthetic construct
  source 1..19: mol_type = other RNA
ggacaagaagctgctatga

SEQ ID NO: 401 - RNA, 21 nt, synthetic construct
  source 1..21: mol_type = other RNA
acgggacagtattctcagtga

SEQ ID NO: 402 - RNA, 21 nt, synthetic construct
  source 1..21: mol_type = other RNA
aagggacagtattctcagtgc

SEQ ID NO: 403 - RNA, 19 nt, synthetic construct
  source 1..19: mol_type = other RNA
ttaaaagggacagtattct

SEQ ID NO: 404 - RNA, 19 nt, synthetic construct
  source 1..19: mol_type = other RNA
aagggacagtattctcagt

SEQ ID NO: 405 - RNA, 19 nt, synthetic construct
  source 1..19: mol_type = other RNA
ccaagtccacctgcctatt

SEQ ID NO: 406 - RNA, 19 nt, synthetic construct
  source 1..19: mol_type = other RNA
ccgttaaggacaagttctt

SEQ ID NO: 407 - RNA, 19 nt, synthetic construct
  source 1..19: mol_type = other RNA
cgaggatgcctcccttctt

SEQ ID NO: 408 - RNA, 19 nt, synthetic construct
  source 1..19: mol_type = other RNA
aagggacagtattctcaga

SEQ ID NO: 409 - RNA, 21 nt, synthetic construct
  source 1..21: mol_type = other RNA
aaaagggacagtattctcagt

SEQ ID NO: 410 - RNA, 21 nt, synthetic construct
  source 1..21: mol_type = other RNA
aaaagggacagtattctcagt

SEQ ID NO: 411 - RNA, 21 nt, synthetic construct
  source 1..21: mol_type = other RNA
aaaagggacagtattctcagt

SEQ ID NO: 412 - RNA, 19 nt, synthetic construct
  source 1..19: mol_type = other RNA
aagggacagtattctcaga

SEQ ID NO: 413 - RNA, 19 nt, synthetic construct
  source 1..19: mol_type = other RNA
aagggacagtattctcaga

SEQ ID NO: 414 - RNA, 21 nt, synthetic construct
  source 1..21: mol_type = other RNA
attcctggagcagctgccttt

SEQ ID NO: 415 - RNA, 21 nt, synthetic construct
  source 1..21: mol_type = other RNA
tgttcctggagcagctgcctt

SEQ ID NO: 416 - RNA, 21 nt, synthetic construct
  source 1..21: mol_type = other RNA
ttgttcctggagcagctgctt

SEQ ID NO: 417 - RNA, 21 nt, synthetic construct
  source 1..21: mol_type = other RNA
tctgttcctggagcagctgtt

SEQ ID NO: 418 - RNA, 21 nt, synthetic construct
  source 1..21: mol_type = other RNA
ttctgttcctggagcagcttt

SEQ ID NO: 419 - RNA, 21 nt, synthetic construct
  source 1..21: mol_type = other RNA
tctctgttcctggagcagctt

SEQ ID NO: 420 - RNA, 21 nt, synthetic construct
  source 1..21: mol_type = other RNA
tacctctgttcctggagcatt

SEQ ID NO: 421 - RNA, 21 nt, synthetic construct
  source 1..21: mol_type = other RNA
tatggcacctctgttcctgtt

SEQ ID NO: 422 - RNA, 21 nt, synthetic construct
  source 1..21: mol_type = other RNA
acatggcacctctgttccttt

SEQ ID NO: 423 - RNA, 21 nt, synthetic construct
  source 1..21: mol_type = other RNA
tgcatggcacctctgttcctt

SEQ ID NO: 424 - RNA, 21 nt, synthetic construct
  source 1..21: mol_type = other RNA
ttgcatggcacctctgttctt

SEQ ID NO: 425 - RNA, 21 nt, synthetic construct
  source 1..21: mol_type = other RNA
actgcatggcacctctgtttt

SEQ ID NO: 426 - RNA, 21 nt, synthetic construct
  source 1..21: mol_type = other RNA
aagtacccggggctgcatgtt

SEQ ID NO: 427 - RNA, 21 nt, synthetic construct
  source 1..21: mol_type = other RNA
agagtacccggggctgcattt

SEQ ID NO: 428 - RNA, 21 nt, synthetic construct
  source 1..21: mol_type = other RNA
aggagtacccggggctgcatt

SEQ ID NO: 429 - RNA, 21 nt, synthetic construct
  source 1..21: mol_type = other RNA
aaggagtacccggggctgctt

SEQ ID NO: 430 - RNA, 21 nt, synthetic construct
  source 1..21: mol_type = other RNA
taaggagtacccggggctgtt

SEQ ID NO: 431 - RNA, 21 nt, synthetic construct
  source 1..21: mol_type = other RNA
acaaggagtacccggggcttt

SEQ ID NO: 432 - RNA, 21 nt, synthetic construct
  source 1..21: mol_type = other RNA
aacaaggagtacccggggctt

SEQ ID NO: 433 - RNA, 21 nt, synthetic construct
  source 1..21: mol_type = other RNA
taacaaggagtacccggggtt

SEQ ID NO: 434 - RNA, 21 nt, synthetic construct
  source 1..21: mol_type = other RNA
acaacaaggagtacccgggtt

SEQ ID NO: 435 - RNA, 21 nt, synthetic construct
  source 1..21: mol_type = other RNA
aacaacaaggagtacccggtt

SEQ ID NO: 436 - RNA, 21 nt, synthetic construct
  source 1..21: mol_type = other RNA
taacaacaaggagtacccgtt

SEQ ID NO: 437 - RNA, 21 nt, synthetic construct
  source 1..21: mol_type = other RNA
acaacaacaaggagtaccctt

SEQ ID NO: 438 - RNA, 21 nt, synthetic construct
  source 1..21: mol_type = other RNA
agcaacaacaaggagtacctt

SEQ ID NO: 439 - RNA, 21 nt, synthetic construct
  source 1..21: mol_type = other RNA
aggcaacaacaaggagtactt

SEQ ID NO: 440 - RNA, 21 nt, synthetic construct
  source 1..21: mol_type = other RNA
aagggcaacaacaaggagttt

SEQ ID NO: 441 - RNA, 21 nt, synthetic construct
  source 1..21: mol_type = other RNA
agagggcaacaacaaggagtt

SEQ ID NO: 442 - RNA, 21 nt, synthetic construct
  source 1..21: mol_type = other RNA
aggagggcaacaacaaggatt

SEQ ID NO: 443 - RNA, 21 nt, synthetic construct
  source 1..21: mol_type = other RNA
taggagggcaacaacaaggtt

SEQ ID NO: 444 - RNA, 21 nt, synthetic construct
  source 1..21: mol_type = other RNA
tcaggagggcaacaacaagtt

SEQ ID NO: 445 - RNA, 21 nt, synthetic construct
  source 1..21: mol_type = other RNA
accaggagggcaacaacaatt

SEQ ID NO: 446 - RNA, 21 nt, synthetic construct
  source 1..21: mol_type = other RNA
tgccaggagggcaacaacatt

SEQ ID NO: 447 - RNA, 21 nt, synthetic construct
  source 1..21: mol_type = other RNA
tcaggagcgccaggagggctt

SEQ ID NO: 448 - RNA, 21 nt, synthetic construct
  source 1..21: mol_type = other RNA
aaggccaggagcgccaggatt

SEQ ID NO: 449 - RNA, 21 nt, synthetic construct
  source 1..21: mol_type = other RNA
tagaggccaggagcgccagtt

SEQ ID NO: 450 - RNA, 21 nt, synthetic construct
  source 1..21: mol_type = other RNA
acagaggccaggagcgccatt

SEQ ID NO: 451 - RNA, 21 nt, synthetic construct
  source 1..21: mol_type = other RNA
agcagaggccaggagcgcctt

SEQ ID NO: 452 - RNA, 21 nt, synthetic construct
  source 1..21: mol_type = other RNA
aggcagaggccaggagcgctt

SEQ ID NO: 453 - RNA, 21 nt, synthetic construct
  source 1..21: mol_type = other RNA
aagctcgggcagaggccagtt

SEQ ID NO: 454 - RNA, 21 nt, synthetic construct
  source 1..21: mol_type = other RNA
aaagctcgggcagaggccatt

SEQ ID NO: 455 - RNA, 21 nt, synthetic construct
  source 1..21: mol_type = other RNA
tgaagctcgggcagaggcctt

SEQ ID NO: 456 - RNA, 21 nt, synthetic construct
  source 1..21: mol_type = other RNA
ttgaagctcgggcagaggctt

SEQ ID NO: 457 - RNA, 21 nt, synthetic construct
  source 1..21: mol_type = other RNA
tctgaagctcgggcagaggtt

SEQ ID NO: 458 - RNA, 21 nt, synthetic construct
  source 1..21: mol_type = other RNA
ttctgaagctcgggcagagtt

SEQ ID NO: 459 - RNA, 21 nt, synthetic construct
  source 1..21: mol_type = other RNA
tctctgaagctcgggcagatt

SEQ ID NO: 460 - RNA, 21 nt, synthetic construct
  source 1..21: mol_type = other RNA
acctctgaagctcgggcagtt

SEQ ID NO: 461 - RNA, 21 nt, synthetic construct
  source 1..21: mol_type = other RNA
agcctctgaagctcgggcatt

SEQ ID NO: 462 - RNA, 21 nt, synthetic construct
  source 1..21: mol_type = other RNA
atcctcggcctctgaagcttt

SEQ ID NO: 463 - RNA, 21 nt, synthetic construct
  source 1..21: mol_type = other RNA
tatcctcggcctctgaagctt

SEQ ID NO: 464 - RNA, 21 nt, synthetic construct
  source 1..21: mol_type = other RNA
acatcctcggcctctgaagtt

SEQ ID NO: 465 - RNA, 21 nt, synthetic construct
  source 1..21: mol_type = other RNA
agcatcctcggcctctgaatt

SEQ ID NO: 466 - RNA, 21 nt, synthetic construct
  source 1..21: mol_type = other RNA
aggcatcctcggcctctgatt

SEQ ID NO: 467 - RNA, 21 nt, synthetic construct
  source 1..21: mol_type = other RNA
aaggcatcctcggcctctgtt

SEQ ID NO: 468 - RNA, 21 nt, synthetic construct
  source 1..21: mol_type = other RNA
agaggcatcctcggcctcttt

SEQ ID NO: 469 - RNA, 21 nt, synthetic construct
  source 1..21: mol_type = other RNA
aggaggcatcctcggcctctt

SEQ ID NO: 470 - RNA, 21 nt, synthetic construct
  source 1..21: mol_type = other RNA
aagggaggcatcctcggcctt

SEQ ID NO: 471 - RNA, 21 nt, synthetic construct
  source 1..21: mol_type = other RNA
aaagggaggcatcctcggctt

SEQ ID NO: 472 - RNA, 21 nt, synthetic construct
  source 1..21: mol_type = other RNA
agaagggaggcatcctcggtt

SEQ ID NO: 473 - RNA, 21 nt, synthetic construct
  source 1..21: mol_type = other RNA
aagaagggaggcatcctcgtt

SEQ ID NO: 474 - RNA, 21 nt, synthetic construct
  source 1..21: mol_type = other RNA
tgagaagggaggcatcctctt

SEQ ID NO: 475 - RNA, 21 nt, synthetic construct
  source 1..21: mol_type = other RNA
ttgagaagggaggcatccttt

SEQ ID NO: 476 - RNA, 21 nt, synthetic construct
  source 1..21: mol_type = other RNA
actgagaagggaggcatcctt

SEQ ID NO: 477 - RNA, 21 nt, synthetic construct
  source 1..21: mol_type = other RNA
agctgagaagggaggcatctt

SEQ ID NO: 478 - RNA, 21 nt, synthetic construct
  source 1..21: mol_type = other RNA
aagctgagaagggaggcattt

SEQ ID NO: 479 - RNA, 21 nt, synthetic construct
  source 1..21: mol_type = other RNA
aaagctgagaagggaggcatt

SEQ ID NO: 480 - RNA, 21 nt, synthetic construct
  source 1..21: mol_type = other RNA
tgaagctgagaagggaggctt

SEQ ID NO: 481 - RNA, 21 nt, synthetic construct
  source 1..21: mol_type = other RNA
atgaagctgagaagggaggtt

SEQ ID NO: 482 - RNA, 21 nt, synthetic construct
  source 1..21: mol_type = other RNA
tatgaagctgagaagggagtt

SEQ ID NO: 483 - RNA, 21 nt, synthetic construct
  source 1..21: mol_type = other RNA
acatgaagctgagaagggatt

SEQ ID NO: 484 - RNA, 21 nt, synthetic construct
  source 1..21: mol_type = other RNA
tgcatgaagctgagaagggtt

SEQ ID NO: 485 - RNA, 21 nt, synthetic construct
  source 1..21: mol_type = other RNA
ttgcatgaagctgagaaggtt

SEQ ID NO: 486 - RNA, 21 nt, synthetic construct
  source 1..21: mol_type = other RNA
tctgcatgaagctgagaagtt

SEQ ID NO: 487 - RNA, 21 nt, synthetic construct
  source 1..21: mol_type = other RNA
tcctgcatgaagctgagaatt

SEQ ID NO: 488 - RNA, 21 nt, synthetic construct
  source 1..21: mol_type = other RNA
accctgcatgaagctgagatt

SEQ ID NO: 489 - RNA, 21 nt, synthetic construct
  source 1..21: mol_type = other RNA
aaccctgcatgaagctgagtt

SEQ ID NO: 490 - RNA, 21 nt, synthetic construct
  source 1..21: mol_type = other RNA
taaccctgcatgaagctgatt

SEQ ID NO: 491 - RNA, 21 nt, synthetic construct
  source 1..21: mol_type = other RNA
ataaccctgcatgaagctgtt

SEQ ID NO: 492 - RNA, 21 nt, synthetic construct
  source 1..21: mol_type = other RNA
tgtaaccctgcatgaagcttt

SEQ ID NO: 493 - RNA, 21 nt, synthetic construct
  source 1..21: mol_type = other RNA
atgtaaccctgcatgaagctt

SEQ ID NO: 494 - RNA, 21 nt, synthetic construct
  source 1..21: mol_type = other RNA
tatgtaaccctgcatgaagtt

SEQ ID NO: 495 - RNA, 21 nt, synthetic construct
  source 1..21: mol_type = other RNA
tcatgtaaccctgcatgaatt

SEQ ID NO: 496 - RNA, 21 nt, synthetic construct
  source 1..21: mol_type = other RNA
ttcatgtaaccctgcatgatt

SEQ ID NO: 497 - RNA, 21 nt, synthetic construct
  source 1..21: mol_type = other RNA
tttcatgtaaccctgcatgtt

SEQ ID NO: 498 - RNA, 21 nt, synthetic construct
  source 1..21: mol_type = other RNA
acttcatgtaaccctgcattt

SEQ ID NO: 499 - RNA, 21 nt, synthetic construct
  source 1..21: mol_type = other RNA
tgcttcatgtaaccctgcatt

SEQ ID NO: 500 - RNA, 21 nt, synthetic construct
  source 1..21: mol_type = other RNA
atgcttcatgtaaccctgctt

SEQ ID NO: 501 - RNA, 21 nt, synthetic construct
  source 1..21: mol_type = other RNA
tgtgcttcatgtaaccctgtt

SEQ ID NO: 502 - RNA, 21 nt, synthetic construct
  source 1..21: mol_type = other RNA
acgtgcttcatgtaacccttt

SEQ ID NO: 503 - RNA, 21 nt, synthetic construct
  source 1..21: mol_type = other RNA
agcgtgcttcatgtaaccctt

SEQ ID NO: 504 - RNA, 21 nt, synthetic construct
  source 1..21: mol_type = other RNA
atggcgtgcttcatgtaactt

SEQ ID NO: 505 - RNA, 21 nt, synthetic construct
  source 1..21: mol_type = other RNA
ttggtggcgtgcttcatgttt

SEQ ID NO: 506 - RNA, 21 nt, synthetic construct
  source 1..21: mol_type = other RNA
tttggtggcgtgcttcatgtt

SEQ ID NO: 507 - RNA, 21 nt, synthetic construct
  source 1..21: mol_type = other RNA
tcttggtggcgtgcttcattt

SEQ ID NO: 508 - RNA, 21 nt, synthetic construct
  source 1..21: mol_type = other RNA
atcttggtggcgtgcttcatt

SEQ ID NO: 509 - RNA, 21 nt, synthetic construct
  source 1..21: mol_type = other RNA
agtcttggtggcgtgcttctt

SEQ ID NO: 510 - RNA, 21 nt, synthetic construct
  source 1..21: mol_type = other RNA
tggtcttggtggcgtgctttt

SEQ ID NO: 511 - RNA, 21 nt, synthetic construct
  source 1..21: mol_type = other RNA
acggtcttggtggcgtgcttt

SEQ ID NO: 512 - RNA, 21 nt, synthetic construct
  source 1..21: mol_type = other RNA
agcggtcttggtggcgtgctt

SEQ ID NO: 513 - RNA, 21 nt, synthetic construct
  source 1..21: mol_type = other RNA
tttggcggtcttggtggcgtt

SEQ ID NO: 514 - RNA, 21 nt, synthetic construct
  source 1..21: mol_type = other RNA
tcttggcggtcttggtggctt

SEQ ID NO: 515 - RNA, 21 nt, synthetic construct
  source 1..21: mol_type = other RNA
tccttggcggtcttggtggtt

SEQ ID NO: 516 - RNA, 21 nt, synthetic construct
  source 1..21: mol_type = other RNA
atccttggcggtcttggtgtt

SEQ ID NO: 517 - RNA, 21 nt, synthetic construct
  source 1..21: mol_type = other RNA
tatccttggcggtcttggttt

SEQ ID NO: 518 - RNA, 21 nt, synthetic construct
  source 1..21: mol_type = other RNA
acatccttggcggtcttggtt

SEQ ID NO: 519 - RNA, 21 nt, synthetic construct
  source 1..21: mol_type = other RNA
tgcatccttggcggtcttgtt

SEQ ID NO: 520 - RNA, 21 nt, synthetic construct
  source 1..21: mol_type = other RNA
atgcatccttggcggtctttt

SEQ ID NO: 521 - RNA, 21 nt, synthetic construct
  source 1..21: mol_type = other RNA
agtgcatccttggcggtcttt

SEQ ID NO: 522 - RNA, 21 nt, synthetic construct
  source 1..21: mol_type = other RNA
tagtgcatccttggcggtctt

SEQ ID NO: 523 - RNA, 21 nt, synthetic construct
  source 1..21: mol_type = other RNA
tcagtgcatccttggcggttt

SEQ ID NO: 524 - RNA, 21 nt, synthetic construct
  source 1..21: mol_type = other RNA
ttcagtgcatccttggcggtt

SEQ ID NO: 525 - RNA, 21 nt, synthetic construct
  source 1..21: mol_type = other RNA
actcagtgcatccttggcgtt

SEQ ID NO: 526 - RNA, 21 nt, synthetic construct
  source 1..21: mol_type = other RNA
tgctcagtgcatccttggctt

SEQ ID NO: 527 - RNA, 21 nt, synthetic construct
  source 1..21: mol_type = other RNA
ttgctcagtgcatccttggtt

SEQ ID NO: 528 - RNA, 21 nt, synthetic construct
  source 1..21: mol_type = other RNA
actgctcagtgcatccttgtt

SEQ ID NO: 529 - RNA, 21 nt, synthetic construct
  source 1..21: mol_type = other RNA
tgctgctcagtgcatcctttt

SEQ ID NO: 530 - RNA, 21 nt, synthetic construct
  source 1..21: mol_type = other RNA
acgctgctcagtgcatccttt

SEQ ID NO: 531 - RNA, 21 nt, synthetic construct
  source 1..21: mol_type = other RNA
tacgctgctcagtgcatcctt

SEQ ID NO: 532 - RNA, 21 nt, synthetic construct
  source 1..21: mol_type = other RNA
acacgctgctcagtgcatctt

SEQ ID NO: 533 - RNA, 21 nt, synthetic construct
  source 1..21: mol_type = other RNA
tgcacgctgctcagtgcattt

SEQ ID NO: 534 - RNA, 21 nt, synthetic construct
  source 1..21: mol_type = other RNA
ttgcacgctgctcagtgcatt

SEQ ID NO: 535 - RNA, 21 nt, synthetic construct
  source 1..21: mol_type = other RNA
tctgcacgctgctcagtgctt

SEQ ID NO: 536 - RNA, 21 nt, synthetic construct
  source 1..21: mol_type = other RNA
tcctgcacgctgctcagtgtt

SEQ ID NO: 537 - RNA, 21 nt, synthetic construct
  source 1..21: mol_type = other RNA
ttcctgcacgctgctcagttt

SEQ ID NO: 538 - RNA, 21 nt, synthetic construct
  source 1..21: mol_type = other RNA
actcctgcacgctgctcagtt

SEQ ID NO: 539 - RNA, 21 nt, synthetic construct
  source 1..21: mol_type = other RNA
aactcctgcacgctgctcatt

SEQ ID NO: 540 - RNA, 21 nt, synthetic construct
  source 1..21: mol_type = other RNA
agactcctgcacgctgctctt

SEQ ID NO: 541 - RNA, 21 nt, synthetic construct
  source 1..21: mol_type = other RNA
aggactcctgcacgctgcttt

SEQ ID NO: 542 - RNA, 21 nt, synthetic construct
  source 1..21: mol_type = other RNA
tgggactcctgcacgctgctt

SEQ ID NO: 543 - RNA, 21 nt, synthetic construct
  source 1..21: mol_type = other RNA
ttgggactcctgcacgctgtt

SEQ ID NO: 544 - RNA, 21 nt, synthetic construct
  source 1..21: mol_type = other RNA
tctgggactcctgcacgcttt

SEQ ID NO: 545 - RNA, 21 nt, synthetic construct
  source 1..21: mol_type = other RNA
acctgggactcctgcacgctt

SEQ ID NO: 546 - RNA, 21 nt, synthetic construct
  source 1..21: mol_type = other RNA
tacctgggactcctgcacgtt

SEQ ID NO: 547 - RNA, 21 nt, synthetic construct
  source 1..21: mol_type = other RNA
tcacctgggactcctgcactt

SEQ ID NO: 548 - RNA, 21 nt, synthetic construct
  source 1..21: mol_type = other RNA
accacctgggactcctgcatt

SEQ ID NO: 549 - RNA, 21 nt, synthetic construct
  source 1..21: mol_type = other RNA
ttgctgggccacctgggactt

SEQ ID NO: 550 - RNA, 21 nt, synthetic construct
  source 1..21: mol_type = other RNA
tctgctgggccacctgggatt

SEQ ID NO: 551 - RNA, 21 nt, synthetic construct
  source 1..21: mol_type = other RNA
acctgctgggccacctgggtt

SEQ ID NO: 552 - RNA, 21 nt, synthetic construct
  source 1..21: mol_type = other RNA
agcctgctgggccacctggtt

SEQ ID NO: 553 - RNA, 21 nt, synthetic construct
  source 1..21: mol_type = other RNA
tggcctgctgggccacctgtt

SEQ ID NO: 554 - RNA, 21 nt, synthetic construct
  source 1..21: mol_type = other RNA
ttggcctgctgggccaccttt

SEQ ID NO: 555 - RNA, 21 nt, synthetic construct
  source 1..21: mol_type = other RNA
tctggcctgctgggccacctt

SEQ ID NO: 556 - RNA, 21 nt, synthetic construct
  source 1..21: mol_type = other RNA
tcctggcctgctgggccactt

SEQ ID NO: 557 - RNA, 21 nt, synthetic construct
  source 1..21: mol_type = other RNA
tacccagcccctggcctgctt

SEQ ID NO: 558 - RNA, 21 nt, synthetic construct
  source 1..21: mol_type = other RNA
tcacccagcccctggcctgtt

SEQ ID NO: 559 - RNA, 21 nt, synthetic construct
  source 1..21: mol_type = other RNA
atcacccagcccctggccttt

SEQ ID NO: 560 - RNA, 21 nt, synthetic construct
  source 1..21: mol_type = other RNA
agtcacccagcccctggcctt

SEQ ID NO: 561 - RNA, 21 nt, synthetic construct
  source 1..21: mol_type = other RNA
tggtcacccagcccctggctt

SEQ ID NO: 562 - RNA, 21 nt, synthetic construct
  source 1..21: mol_type = other RNA
tcggtcacccagcccctggtt

SEQ ID NO: 563 - RNA, 21 nt, synthetic construct
  source 1..21: mol_type = other RNA
atcggtcacccagcccctgtt

SEQ ID NO: 564 - RNA, 21 nt, synthetic construct
  source 1..21: mol_type = other RNA
tatcggtcacccagccccttt

SEQ ID NO: 565 - RNA, 21 nt, synthetic construct
  source 1..21: mol_type = other RNA
tcatcggtcacccagcccctt

SEQ ID NO: 566 - RNA, 21 nt, synthetic construct
  source 1..21: mol_type = other RNA
accatcggtcacccagccctt

SEQ ID NO: 567 - RNA, 21 nt, synthetic construct
  source 1..21: mol_type = other RNA
agccatcggtcacccagcctt

SEQ ID NO: 568 - RNA, 21 nt, synthetic construct
  source 1..21: mol_type = other RNA
aagccatcggtcacccagctt

SEQ ID NO: 569 - RNA, 21 nt, synthetic construct
  source 1..21: mol_type = other RNA
aaagccatcggtcacccagtt

SEQ ID NO: 570 - RNA, 21 nt, synthetic construct
  source 1..21: mol_type = other RNA
tgaagccatcggtcacccatt

SEQ ID NO: 571 - RNA, 21 nt, synthetic construct
  source 1..21: mol_type = other RNA
ttgaagccatcggtcaccctt

SEQ ID NO: 572 - RNA, 21 nt, synthetic construct
  source 1..21: mol_type = other RNA
actgaagccatcggtcacctt

SEQ ID NO: 573 - RNA, 21 nt, synthetic construct
  source 1..21: mol_type = other RNA
aactgaagccatcggtcactt

SEQ ID NO: 574 - RNA, 21 nt, synthetic construct
  source 1..21: mol_type = other RNA
aaactgaagccatcggtcatt

SEQ ID NO: 575 - RNA, 21 nt, synthetic construct
  source 1..21: mol_type = other RNA
agaactgaagccatcggtctt

SEQ ID NO: 576 - RNA, 21 nt, synthetic construct
  source 1..21: mol_type = other RNA
aggaactgaagccatcggttt

SEQ ID NO: 577 - RNA, 21 nt, synthetic construct
  source 1..21: mol_type = other RNA
agggaactgaagccatcggtt

SEQ ID NO: 578 - RNA, 21 nt, synthetic construct
  source 1..21: mol_type = other RNA
tagggaactgaagccatcgtt

SEQ ID NO: 579 - RNA, 21 nt, synthetic construct
  source 1..21: mol_type = other RNA
tcagggaactgaagccatctt

SEQ ID NO: 580 - RNA, 21 nt, synthetic construct
  source 1..21: mol_type = other RNA
ttcagggaactgaagccattt

SEQ ID NO: 581 - RNA, 21 nt, synthetic construct
  source 1..21: mol_type = other RNA
tttcagggaactgaagccatt

SEQ ID NO: 582 - RNA, 21 nt, synthetic construct
  source 1..21: mol_type = other RNA
ttttcagggaactgaagcctt

SEQ ID NO: 583 - RNA, 21 nt, synthetic construct
  source 1..21: mol_type = other RNA
tctttcagggaactgaagctt

SEQ ID NO: 584 - RNA, 21 nt, synthetic construct
  source 1..21: mol_type = other RNA
atctttcagggaactgaagtt

SEQ ID NO: 585 - RNA, 21 nt, synthetic construct
  source 1..21: mol_type = other RNA
agtctttcagggaactgaatt

SEQ ID NO: 586 - RNA, 21 nt, synthetic construct
  source 1..21: mol_type = other RNA
tagtctttcagggaactgatt

SEQ ID NO: 587 - RNA, 21 nt, synthetic construct
  source 1..21: mol_type = other RNA
atagtctttcagggaactgtt

SEQ ID NO: 588 - RNA, 21 nt, synthetic construct
  source 1..21: mol_type = other RNA
agtagtctttcagggaacttt

SEQ ID NO: 589 - RNA, 21 nt, synthetic construct
  source 1..21: mol_type = other RNA
tagtagtctttcagggaactt

SEQ ID NO: 590 - RNA, 21 nt, synthetic construct
  source 1..21: mol_type = other RNA
tcagtagtctttcagggaatt

SEQ ID NO: 591 - RNA, 21 nt, synthetic construct
  source 1..21: mol_type = other RNA
tccagtagtctttcagggatt

SEQ ID NO: 592 - RNA, 21 nt, synthetic construct
  source 1..21: mol_type = other RNA
ttccagtagtctttcagggtt

SEQ ID NO: 593 - RNA, 21 nt, synthetic construct
  source 1..21: mol_type = other RNA
actccagtagtctttcaggtt

SEQ ID NO: 594 - RNA, 21 nt, synthetic construct
  source 1..21: mol_type = other RNA
tgctccagtagtctttcagtt

SEQ ID NO: 595 - RNA, 21 nt, synthetic construct
  source 1..21: mol_type = other RNA
atgctccagtagtctttcatt

SEQ ID NO: 596 - RNA, 21 nt, synthetic construct
  source 1..21: mol_type = other RNA
agtgctccagtagtctttctt

SEQ ID NO: 597 - RNA, 21 nt, synthetic construct
  source 1..21: mol_type = other RNA
tggtgctccagtagtcttttt

SEQ ID NO: 598 - RNA, 21 nt, synthetic construct
  source 1..21: mol_type = other RNA
aacggtgctccagtagtcttt

SEQ ID NO: 599 - RNA, 21 nt, synthetic construct
  source 1..21: mol_type = other RNA
taacggtgctccagtagtctt

SEQ ID NO: 600 - RNA, 21 nt, synthetic construct
  source 1..21: mol_type = other RNA
ttaacggtgctccagtagttt

SEQ ID NO: 601 - RNA, 21 nt, synthetic construct
  source 1..21: mol_type = other RNA
tttaacggtgctccagtagtt

SEQ ID NO: 602 - RNA, 21 nt, synthetic construct
  source 1..21: mol_type = other RNA
tcttaacggtgctccagtatt

SEQ ID NO: 603 - RNA, 21 nt, synthetic construct
  source 1..21: mol_type = other RNA
tccttaacggtgctccagttt

SEQ ID NO: 604 - RNA, 21 nt, synthetic construct
  source 1..21: mol_type = other RNA
atccttaacggtgctccagtt

SEQ ID NO: 605 - RNA, 21 nt, synthetic construct
  source 1..21: mol_type = other RNA
tgtccttaacggtgctccatt

SEQ ID NO: 606 - RNA, 21 nt, synthetic construct
  source 1..21: mol_type = other RNA
ttgtccttaacggtgctcctt

SEQ ID NO: 607 - RNA, 21 nt, synthetic construct
  source 1..21: mol_type = other RNA
tttgtccttaacggtgctctt

SEQ ID NO: 608 - RNA, 21 nt, synthetic construct
  source 1..21: mol_type = other RNA
acttgtccttaacggtgcttt

SEQ ID NO: 609 - RNA, 21 nt, synthetic construct
  source 1..21: mol_type = other RNA
aacttgtccttaacggtgctt

SEQ ID NO: 610 - RNA, 21 nt, synthetic construct
  source 1..21: mol_type = other RNA
aaacttgtccttaacggtgtt

SEQ ID NO: 611 - RNA, 21 nt, synthetic construct
  source 1..21: mol_type = other RNA
agaacttgtccttaacggttt

SEQ ID NO: 612 - RNA, 21 nt, synthetic construct
  source 1..21: mol_type = other RNA
aagaacttgtccttaacggtt

SEQ ID NO: 613 - RNA, 21 nt, synthetic construct
  source 1..21: mol_type = other RNA
agagaacttgtccttaacgtt

SEQ ID NO: 614 - RNA, 21 nt, synthetic construct
  source 1..21: mol_type = other RNA
tagagaacttgtccttaactt

SEQ ID NO: 615 - RNA, 21 nt, synthetic construct
  source 1..21: mol_type = other RNA
tcagagaacttgtccttaatt

SEQ ID NO: 616 - RNA, 21 nt, synthetic construct
  source 1..21: mol_type = other RNA
ttcagagaacttgtccttatt

SEQ ID NO: 617 - RNA, 21 nt, synthetic construct
  source 1..21: mol_type = other RNA
actcagagaacttgtcctttt

SEQ ID NO: 618 - RNA, 21 nt, synthetic construct
  source 1..21: mol_type = other RNA
aactcagagaacttgtccttt

SEQ ID NO: 619 - RNA, 21 nt, synthetic construct
  source 1..21: mol_type = other RNA
aaactcagagaacttgtcctt

SEQ ID NO: 620 - RNA, 21 nt, synthetic construct
  source 1..21: mol_type = other RNA
agaactcagagaacttgtctt

SEQ ID NO: 621 - RNA, 21 nt, synthetic construct
  source 1..21: mol_type = other RNA
tagaactcagagaacttgttt

SEQ ID NO: 622 - RNA, 21 nt, synthetic construct
  source 1..21: mol_type = other RNA
tcagaactcagagaacttgtt

SEQ ID NO: 623 - RNA, 21 nt, synthetic construct
  source 1..21: mol_type = other RNA
tccagaactcagagaactttt

SEQ ID NO: 624 - RNA, 21 nt, synthetic construct
  source 1..21: mol_type = other RNA
tcccagaactcagagaacttt

SEQ ID NO: 625 - RNA, 21 nt, synthetic construct
  source 1..21: mol_type = other RNA
atcccagaactcagagaactt

SEQ ID NO: 626 - RNA, 21 nt, synthetic construct
  source 1..21: mol_type = other RNA
aatcccagaactcagagaatt

SEQ ID NO: 627 - RNA, 21 nt, synthetic construct
  source 1..21: mol_type = other RNA
aaatcccagaactcagagatt

SEQ ID NO: 628 - RNA, 21 nt, synthetic construct
  source 1..21: mol_type = other RNA
taaatcccagaactcagagtt

SEQ ID NO: 629 - RNA, 21 nt, synthetic construct
  source 1..21: mol_type = other RNA
tcaaatcccagaactcagatt

SEQ ID NO: 630 - RNA, 21 nt, synthetic construct
  source 1..21: mol_type = other RNA
tccaaatcccagaactcagtt

SEQ ID NO: 631 - RNA, 21 nt, synthetic construct
  source 1..21: mol_type = other RNA
atccaaatcccagaactcatt

SEQ ID NO: 632 - RNA, 21 nt, synthetic construct
  source 1..21: mol_type = other RNA
agtccaaatcccagaactctt

SEQ ID NO: 633 - RNA, 21 nt, synthetic construct
  source 1..21: mol_type = other RNA
aggtccaaatcccagaacttt

SEQ ID NO: 634 - RNA, 21 nt, synthetic construct
  source 1..21: mol_type = other RNA
tagggtccaaatcccagaatt

SEQ ID NO: 635 - RNA, 21 nt, synthetic construct
  source 1..21: mol_type = other RNA
tcagggtccaaatcccagatt

SEQ ID NO: 636 - RNA, 21 nt, synthetic construct
  source 1..21: mol_type = other RNA
ttcagggtccaaatcccagtt

SEQ ID NO: 637 - RNA, 21 nt, synthetic construct
  source 1..21: mol_type = other RNA
tctcagggtccaaatcccatt

SEQ ID NO: 638 - RNA, 21 nt, synthetic construct
  source 1..21: mol_type = other RNA
acctcagggtccaaatccctt

SEQ ID NO: 639 - RNA, 21 nt, synthetic construct
  source 1..21: mol_type = other RNA
aacctcagggtccaaatcctt

SEQ ID NO: 640 - RNA, 21 nt, synthetic construct
  source 1..21: mol_type = other RNA
tgacctcagggtccaaatctt

SEQ ID NO: 641 - RNA, 21 nt, synthetic construct
  source 1..21: mol_type = other RNA
ttgacctcagggtccaaattt

SEQ ID NO: 642 - RNA, 21 nt, synthetic construct
  source 1..21: mol_type = other RNA
tctgacctcagggtccaaatt

SEQ ID NO: 643 - RNA, 21 nt, synthetic construct
  source 1..21: mol_type = other RNA
atctgacctcagggtccaatt

SEQ ID NO: 644 - RNA, 21 nt, synthetic construct
  source 1..21: mol_type = other RNA
agtctgacctcagggtccatt

SEQ ID NO: 645 - RNA, 21 nt, synthetic construct
  source 1..21: mol_type = other RNA
tggtctgacctcagggtcctt

SEQ ID NO: 646 - RNA, 21 nt, synthetic construct
  source 1..21: mol_type = other RNA
ttggtctgacctcagggtctt

SEQ ID NO: 647 - RNA, 21 nt, synthetic construct
  source 1..21: mol_type = other RNA
attggtctgacctcagggttt

SEQ ID NO: 648 - RNA, 21 nt, synthetic construct
  source 1..21: mol_type = other RNA
agttggtctgacctcagggtt

SEQ ID NO: 649 - RNA, 21 nt, synthetic construct
  source 1..21: mol_type = other RNA
aagttggtctgacctcaggtt

SEQ ID NO: 650 - RNA, 21 nt, synthetic construct
  source 1..21: mol_type = other RNA
aaagttggtctgacctcagtt

SEQ ID NO: 651 - RNA, 21 nt, synthetic construct
  source 1..21: mol_type = other RNA
tgaagttggtctgacctcatt

SEQ ID NO: 652 - RNA, 21 nt, synthetic construct
  source 1..21: mol_type = other RNA
ttgaagttggtctgacctctt

SEQ ID NO: 653 - RNA, 21 nt, synthetic construct
  source 1..21: mol_type = other RNA
actgaagttggtctgaccttt

SEQ ID NO: 654 - RNA, 21 nt, synthetic construct
  source 1..21: mol_type = other RNA
agctgaagttggtctgacctt

SEQ ID NO: 655 - RNA, 21 nt, synthetic construct
  source 1..21: mol_type = other RNA
tggctgaagttggtctgactt

SEQ ID NO: 656 - RNA, 21 nt, synthetic construct
  source 1..21: mol_type = other RNA
tagccacggctgaagttggtt

SEQ ID NO: 657 - RNA, 21 nt, synthetic construct
  source 1..21: mol_type = other RNA
acagccacggctgaagttgtt

SEQ ID NO: 658 - RNA, 21 nt, synthetic construct
  source 1..21: mol_type = other RNA
agcagccacggctgaagtttt

SEQ ID NO: 659 - RNA, 21 nt, synthetic construct
  source 1..21: mol_type = other RNA
aggcagccacggctgaagttt

SEQ ID NO: 660 - RNA, 21 nt, synthetic construct
  source 1..21: mol_type = other RNA
taggcagccacggctgaagtt

SEQ ID NO: 661 - RNA, 21 nt, synthetic construct
  source 1..21: mol_type = other RNA
tcaggcagccacggctgaatt

SEQ ID NO: 662 - RNA, 21 nt, synthetic construct
  source 1..21: mol_type = other RNA
ttcaggcagccacggctgatt

SEQ ID NO: 663 - RNA, 21 nt, synthetic construct
  source 1..21: mol_type = other RNA
tctcaggcagccacggctgtt

SEQ ID NO: 664 - RNA, 21 nt, synthetic construct
  source 1..21: mol_type = other RNA
atctcaggcagccacggcttt

SEQ ID NO: 665 - RNA, 21 nt, synthetic construct
  source 1..21: mol_type = other RNA
agtctcaggcagccacggctt

SEQ ID NO: 666 - RNA, 21 nt, synthetic construct
  source 1..21: mol_type = other RNA
aggtctcaggcagccacggtt

SEQ ID NO: 667 - RNA, 21 nt, synthetic construct
  source 1..21: mol_type = other RNA
aaggtctcaggcagccacgtt

SEQ ID NO: 668 - RNA, 21 nt, synthetic construct
  source 1..21: mol_type = other RNA
tgaggtctcaggcagccactt

SEQ ID NO: 669 - RNA, 21 nt, synthetic construct
  source 1..21: mol_type = other RNA
ttgaggtctcaggcagccatt

SEQ ID NO: 670 - RNA, 21 nt, synthetic construct
  source 1..21: mol_type = other RNA
attgaggtctcaggcagcctt

SEQ ID NO: 671 - RNA, 21 nt, synthetic construct
  source 1..21: mol_type = other RNA
tattgaggtctcaggcagctt

SEQ ID NO: 672 - RNA, 21 nt, synthetic construct
  source 1..21: mol_type = other RNA
atattgaggtctcaggcagtt

SEQ ID NO: 673 - RNA, 21 nt, synthetic construct
  source 1..21: mol_type = other RNA
agtattgaggtctcaggcatt

SEQ ID NO: 674 - RNA, 21 nt, synthetic construct
  source 1..21: mol_type = other RNA
aggtattgaggtctcaggctt

SEQ ID NO: 675 - RNA, 21 nt, synthetic construct
  source 1..21: mol_type = other RNA
agggtattgaggtctcaggtt

SEQ ID NO: 676 - RNA, 21 nt, synthetic construct
  source 1..21: mol_type = other RNA
ttggggtattgaggtctcatt

SEQ ID NO: 677 - RNA, 21 nt, synthetic construct
  source 1..21: mol_type = other RNA
tttggggtattgaggtctctt

SEQ ID NO: 678 - RNA, 21 nt, synthetic construct
  source 1..21: mol_type = other RNA
acttggggtattgaggtcttt

SEQ ID NO: 679 - RNA, 21 nt, synthetic construct
  source 1..21: mol_type = other RNA
aacttggggtattgaggtctt

SEQ ID NO: 680 - RNA, 21 nt, synthetic construct
  source 1..21: mol_type = other RNA
agacttggggtattgaggttt

SEQ ID NO: 681 - RNA, 21 nt, synthetic construct
  source 1..21: mol_type = other RNA
tggacttggggtattgaggtt

SEQ ID NO: 682 - RNA, 21 nt, synthetic construct
  source 1..21: mol_type = other RNA
atggacttggggtattgagtt

SEQ ID NO: 683 - RNA, 21 nt, synthetic construct
  source 1..21: mol_type = other RNA
agtggacttggggtattgatt

SEQ ID NO: 684 - RNA, 21 nt, synthetic construct
  source 1..21: mol_type = other RNA
aggtggacttggggtattgtt

SEQ ID NO: 685 - RNA, 21 nt, synthetic construct
  source 1..21: mol_type = other RNA
taggtggacttggggtatttt

SEQ ID NO: 686 - RNA, 21 nt, synthetic construct
  source 1..21: mol_type = other RNA
acaggtggacttggggtattt

SEQ ID NO: 687 - RNA, 21 nt, synthetic construct
  source 1..21: mol_type = other RNA
agcaggtggacttggggtatt

SEQ ID NO: 688 - RNA, 21 nt, synthetic construct
  source 1..21: mol_type = other RNA
taggcaggtggacttggggtt

SEQ ID NO: 689 - RNA, 21 nt, synthetic construct
  source 1..21: mol_type = other RNA
ataggcaggtggacttgggtt

SEQ ID NO: 690 - RNA, 21 nt, synthetic construct
  source 1..21: mol_type = other RNA
aataggcaggtggacttggtt

SEQ ID NO: 691 - RNA, 21 nt, synthetic construct
  source 1..21: mol_type = other RNA
agataggcaggtggacttgtt

SEQ ID NO: 692 - RNA, 21 nt, synthetic construct
  source 1..21: mol_type = other RNA
tggataggcaggtggactttt

SEQ ID NO: 693 - RNA, 21 nt, synthetic construct
  source 1..21: mol_type = other RNA
atggataggcaggtggacttt

SEQ ID NO: 694 - RNA, 21 nt, synthetic construct
  source 1..21: mol_type = other RNA
aatggataggcaggtggactt

SEQ ID NO: 695 - RNA, 21 nt, synthetic construct
  source 1..21: mol_type = other RNA
agatggataggcaggtggatt

SEQ ID NO: 696 - RNA, 21 nt, synthetic construct
  source 1..21: mol_type = other RNA
aggatggataggcaggtggtt

SEQ ID NO: 697 - RNA, 21 nt, synthetic construct
  source 1..21: mol_type = other RNA
taggatggataggcaggtgtt

SEQ ID NO: 698 - RNA, 21 nt, synthetic construct
  source 1..21: mol_type = other RNA
acaggatggataggcaggttt

SEQ ID NO: 699 - RNA, 21 nt, synthetic construct
  source 1..21: mol_type = other RNA
tgcaggatggataggcaggtt

SEQ ID NO: 700 - RNA, 21 nt, synthetic construct
  source 1..21: mol_type = other RNA
tcgcaggatggataggcagtt

SEQ ID NO: 701 - RNA, 21 nt, synthetic construct
  source 1..21: mol_type = other RNA
ttcgcaggatggataggcatt

SEQ ID NO: 702 - RNA, 21 nt, synthetic construct
  source 1..21: mol_type = other RNA
actcgcaggatggataggctt

SEQ ID NO: 703 - RNA, 21 nt, synthetic construct
  source 1..21: mol_type = other RNA
agctcgcaggatggataggtt

SEQ ID NO: 704 - RNA, 21 nt, synthetic construct
  source 1..21: mol_type = other RNA
aagctcgcaggatggatagtt

SEQ ID NO: 705 - RNA, 21 nt, synthetic construct
  source 1..21: mol_type = other RNA
agagctcgcaggatggatatt

SEQ ID NO: 706 - RNA, 21 nt, synthetic construct
  source 1..21: mol_type = other RNA
aggagctcgcaggatggattt

SEQ ID NO: 707 - RNA, 21 nt, synthetic construct
  source 1..21: mol_type = other RNA
aaggagctcgcaggatggatt

SEQ ID NO: 708 - RNA, 21 nt, synthetic construct
  source 1..21: mol_type = other RNA
taaggagctcgcaggatggtt

SEQ ID NO: 709 - RNA, 21 nt, synthetic construct
  source 1..21: mol_type = other RNA
tcaaggagctcgcaggatgtt

SEQ ID NO: 710 - RNA, 21 nt, synthetic construct
  source 1..21: mol_type = other RNA
tccaaggagctcgcaggattt

SEQ ID NO: 711 - RNA, 21 nt, synthetic construct
  source 1..21: mol_type = other RNA
acccaaggagctcgcaggatt

SEQ ID NO: 712 - RNA, 21 nt, synthetic construct
  source 1..21: mol_type = other RNA
aacccaaggagctcgcaggtt

SEQ ID NO: 713 - RNA, 21 nt, synthetic construct
  source 1..21: mol_type = other RNA
agacccaaggagctcgcagtt

SEQ ID NO: 714 - RNA, 21 nt, synthetic construct
  source 1..21: mol_type = other RNA
aggacccaaggagctcgcatt

SEQ ID NO: 715 - RNA, 21 nt, synthetic construct
  source 1..21: mol_type = other RNA
taggacccaaggagctcgctt

SEQ ID NO: 716 - RNA, 21 nt, synthetic construct
  source 1..21: mol_type = other RNA
acaggacccaaggagctcgtt

SEQ ID NO: 717 - RNA, 21 nt, synthetic construct
  source 1..21: mol_type = other RNA
tgcaggacccaaggagctctt

SEQ ID NO: 718 - RNA, 21 nt, synthetic construct
  source 1..21: mol_type = other RNA
ttgcaggacccaaggagcttt

SEQ ID NO: 719 - RNA, 21 nt, synthetic construct
  source 1..21: mol_type = other RNA
attgcaggacccaaggagctt

SEQ ID NO: 720 - RNA, 21 nt, synthetic construct
  source 1..21: mol_type = other RNA
aattgcaggacccaaggagtt

SEQ ID NO: 721 - RNA, 21 nt, synthetic construct
  source 1..21: mol_type = other RNA
agattgcaggacccaaggatt

SEQ ID NO: 722 - RNA, 21 nt, synthetic construct
  source 1..21: mol_type = other RNA
aagattgcaggacccaaggtt

SEQ ID NO: 723 - RNA, 21 nt, synthetic construct
  source 1..21: mol_type = other RNA
agagattgcaggacccaagtt

SEQ ID NO: 724 - RNA, 21 nt, synthetic construct
  source 1..21: mol_type = other RNA
tggagattgcaggacccaatt

SEQ ID NO: 725 - RNA, 21 nt, synthetic construct
  source 1..21: mol_type = other RNA
ttggagattgcaggacccatt

SEQ ID NO: 726 - RNA, 21 nt, synthetic construct
  source 1..21: mol_type = other RNA
tctggagattgcaggaccctt

SEQ ID NO: 727 - RNA, 21 nt, synthetic construct
  source 1..21: mol_type = other RNA
tcctggagattgcaggacctt

SEQ ID NO: 728 - RNA, 21 nt, synthetic construct
  source 1..21: mol_type = other RNA
accctggagattgcaggactt

SEQ ID NO: 729 - RNA, 21 nt, synthetic construct
  source 1..21: mol_type = other RNA
tagccctggagattgcaggtt

SEQ ID NO: 730 - RNA, 21 nt, synthetic construct
  source 1..21: mol_type = other RNA
acagccctggagattgcagtt

SEQ ID NO: 731 - RNA, 21 nt, synthetic construct
  source 1..21: mol_type = other RNA
agcagccctggagattgcatt

SEQ ID NO: 732 - RNA, 21 nt, synthetic construct
  source 1..21: mol_type = other RNA
tacaggggcagccctggagtt

SEQ ID NO: 733 - RNA, 21 nt, synthetic construct
  source 1..21: mol_type = other RNA
ttacaggggcagccctggatt

SEQ ID NO: 734 - RNA, 21 nt, synthetic construct
  source 1..21: mol_type = other RNA
tctacaggggcagccctggtt

SEQ ID NO: 735 - RNA, 21 nt, synthetic construct
  source 1..21: mol_type = other RNA
acctacaggggcagccctgtt

SEQ ID NO: 736 - RNA, 21 nt, synthetic construct
  source 1..21: mol_type = other RNA
aacctacaggggcagcccttt

SEQ ID NO: 737 - RNA, 21 nt, synthetic construct
  source 1..21: mol_type = other RNA
taacctacaggggcagccctt

SEQ ID NO: 738 - RNA, 21 nt, synthetic construct
  source 1..21: mol_type = other RNA
acaacctacaggggcagcctt

SEQ ID NO: 739 - RNA, 21 nt, synthetic construct
  source 1..21: mol_type = other RNA
agcaacctacaggggcagctt

SEQ ID NO: 740 - RNA, 21 nt, synthetic construct
  source 1..21: mol_type = other RNA
aagcaacctacaggggcagtt

SEQ ID NO: 741 - RNA, 21 nt, synthetic construct
  source 1..21: mol_type = other RNA
taagcaacctacaggggcatt

SEQ ID NO: 742 - RNA, 21 nt, synthetic construct
  source 1..21: mol_type = other RNA
ttaagcaacctacaggggctt

SEQ ID NO: 743 - RNA, 21 nt, synthetic construct
  source 1..21: mol_type = other RNA
tttaagcaacctacaggggtt

SEQ ID NO: 744 - RNA, 21 nt, synthetic construct
  source 1..21: mol_type = other RNA
ttttaagcaacctacagggtt

SEQ ID NO: 745 - RNA, 21 nt, synthetic construct
  source 1..21: mol_type = other RNA
tttttaagcaacctacaggtt

SEQ ID NO: 746 - RNA, 21 nt, synthetic construct
  source 1..21: mol_type = other RNA
tcttttaagcaacctacagtt

SEQ ID NO: 747 - RNA, 21 nt, synthetic construct
  source 1..21: mol_type = other RNA
tccttttaagcaacctacatt

SEQ ID NO: 748 - RNA, 21 nt, synthetic construct
  source 1..21: mol_type = other RNA
tcccttttaagcaacctactt

SEQ ID NO: 749 - RNA, 21 nt, synthetic construct
  source 1..21: mol_type = other RNA
atcccttttaagcaacctatt

SEQ ID NO: 750 - RNA, 21 nt, synthetic construct
  source 1..21: mol_type = other RNA
tgtcccttttaagcaaccttt

SEQ ID NO: 751 - RNA, 21 nt, synthetic construct
  source 1..21: mol_type = other RNA
ttgtcccttttaagcaacctt

SEQ ID NO: 752 - RNA, 21 nt, synthetic construct
  source 1..21: mol_type = other RNA
actgtcccttttaagcaactt

SEQ ID NO: 753 - RNA, 21 nt, synthetic construct
  source 1..21: mol_type = other RNA
tactgtcccttttaagcaatt

SEQ ID NO: 754 - RNA, 21 nt, synthetic construct
  source 1..21: mol_type = other RNA
atactgtcccttttaagcatt

SEQ ID NO: 755 - RNA, 21 nt, synthetic construct
  source 1..21: mol_type = other RNA
aatactgtcccttttaagctt

SEQ ID NO: 756 - RNA, 21 nt, synthetic construct
  source 1..21: mol_type = other RNA
aaatactgtcccttttaagtt

SEQ ID NO: 757 - RNA, 21 nt, synthetic construct
  source 1..21: mol_type = other RNA
agaatactgtcccttttaatt

SEQ ID NO: 758 - RNA, 21 nt, synthetic construct
  source 1..21: mol_type = other RNA
aagaatactgtcccttttatt

SEQ ID NO: 759 - RNA, 21 nt, synthetic construct
  source 1..21: mol_type = other RNA
tgagaatactgtccctttttt

SEQ ID NO: 760 - RNA, 21 nt, synthetic construct
  source 1..21: mol_type = other RNA
ttgagaatactgtcccttttt

SEQ ID NO: 761 - RNA, 21 nt, synthetic construct
  source 1..21: mol_type = other RNA
actgagaatactgtccctttt

SEQ ID NO: 762 - RNA, 21 nt, synthetic construct
  source 1..21: mol_type = other RNA
tactgagaatactgtcccttt

SEQ ID NO: 763 - RNA, 21 nt, synthetic construct
  source 1..21: mol_type = other RNA
acactgagaatactgtccctt

SEQ ID NO: 764 - RNA, 21 nt, synthetic construct
  source 1..21: mol_type = other RNA
agcactgagaatactgtcctt

SEQ ID NO: 765 - RNA, 21 nt, synthetic construct
  source 1..21: mol_type = other RNA
aagcactgagaatactgtctt

SEQ ID NO: 766 - RNA, 21 nt, synthetic construct
  source 1..21: mol_type = other RNA
agagcactgagaatactgttt

SEQ ID NO: 767 - RNA, 21 nt, synthetic construct
  source 1..21: mol_type = other RNA
aagagcactgagaatactgtt

SEQ ID NO: 768 - RNA, 21 nt, synthetic construct
  source 1..21: mol_type = other RNA
agagagcactgagaatacttt

SEQ ID NO: 769 - RNA, 21 nt, synthetic construct
  source 1..21: mol_type = other RNA
aggagagcactgagaatactt

SEQ ID NO: 770 - RNA, 21 nt, synthetic construct
  source 1..21: mol_type = other RNA
taggagagcactgagaatatt

SEQ ID NO: 771 - RNA, 21 nt, synthetic construct
  source 1..21: mol_type = other RNA
ataggagagcactgagaattt

SEQ ID NO: 772 - RNA, 21 nt, synthetic construct
  source 1..21: mol_type = other RNA
agtaggagagcactgagaatt

SEQ ID NO: 773 - RNA, 21 nt, synthetic construct
  source 1..21: mol_type = other RNA
aggtaggagagcactgagatt

SEQ ID NO: 774 - RNA, 21 nt, synthetic construct
  source 1..21: mol_type = other RNA
agggtaggagagcactgagtt

SEQ ID NO: 775 - RNA, 21 nt, synthetic construct
  source 1..21: mol_type = other RNA
tgaggtggggtaggagagctt

SEQ ID NO: 776 - RNA, 21 nt, synthetic construct
  source 1..21: mol_type = other RNA
atgaggtggggtaggagagtt

SEQ ID NO: 777 - RNA, 21 nt, synthetic construct
  source 1..21: mol_type = other RNA
tatgaggtggggtaggagatt

SEQ ID NO: 778 - RNA, 21 nt, synthetic construct
  source 1..21: mol_type = other RNA
acatgaggtggggtaggagtt

SEQ ID NO: 779 - RNA, 21 nt, synthetic construct
  source 1..21: mol_type = other RNA
agcatgaggtggggtaggatt

SEQ ID NO: 780 - RNA, 21 nt, synthetic construct
  source 1..21: mol_type = other RNA
aggcatgaggtggggtaggtt

SEQ ID NO: 781 - RNA, 21 nt, synthetic construct
  source 1..21: mol_type = other RNA
taggcatgaggtggggtagtt

SEQ ID NO: 782 - RNA, 21 nt, synthetic construct
  source 1..21: mol_type = other RNA
tcaggcatgaggtggggtatt

SEQ ID NO: 783 - RNA, 21 nt, synthetic construct
  source 1..21: mol_type = other RNA
accagcatgcctggaggggtt

SEQ ID NO: 784 - RNA, 21 nt, synthetic construct
  source 1..21: mol_type = other RNA
agccagcatgcctggagggtt

SEQ ID NO: 785 - RNA, 21 nt, synthetic construct
  source 1..21: mol_type = other RNA
aggccagcatgcctggaggtt

SEQ ID NO: 786 - RNA, 21 nt, synthetic construct
  source 1..21: mol_type = other RNA
aaggccagcatgcctggagtt

SEQ ID NO: 787 - RNA, 21 nt, synthetic construct
  source 1..21: mol_type = other RNA
ttgggaggccagcatgccttt

SEQ ID NO: 788 - RNA, 21 nt, synthetic construct
  source 1..21: mol_type = other RNA
attgggaggccagcatgcctt

SEQ ID NO: 789 - RNA, 21 nt, synthetic construct
  source 1..21: mol_type = other RNA
tattgggaggccagcatgctt

SEQ ID NO: 790 - RNA, 21 nt, synthetic construct
  source 1..21: mol_type = other RNA
ttattgggaggccagcatgtt

SEQ ID NO: 791 - RNA, 21 nt, synthetic construct
  source 1..21: mol_type = other RNA
tttattgggaggccagcattt

SEQ ID NO: 792 - RNA, 21 nt, synthetic construct
  source 1..21: mol_type = other RNA
ttttattgggaggccagcatt

SEQ ID NO: 793 - RNA, 21 nt, synthetic construct
  source 1..21: mol_type = other RNA
actttattgggaggccagctt

SEQ ID NO: 794 - RNA, 21 nt, synthetic construct
  source 1..21: mol_type = other RNA
agctttattgggaggccagtt

SEQ ID NO: 795 - RNA, 21 nt, synthetic construct
  source 1..21: mol_type = other RNA
tagctttattgggaggccatt

SEQ ID NO: 796 - RNA, 21 nt, synthetic construct
  source 1..21: mol_type = other RNA
tcagctttattgggaggcctt

SEQ ID NO: 797 - RNA, 21 nt, synthetic construct
  source 1..21: mol_type = other RNA
tccagctttattgggaggctt

SEQ ID NO: 798 - RNA, 21 nt, synthetic construct
  source 1..21: mol_type = other RNA
atccagctttattgggaggtt

SEQ ID NO: 799 - RNA, 21 nt, synthetic construct
  source 1..21: mol_type = other RNA
tgtccagctttattgggagtt

SEQ ID NO: 800 - RNA, 21 nt, synthetic construct
  source 1..21: mol_type = other RNA
ttgtccagctttattgggatt

SEQ ID NO: 801 - RNA, 21 nt, synthetic construct
  source 1..21: mol_type = other RNA
tttgtccagctttattgggtt

SEQ ID NO: 802 - RNA, 21 nt, synthetic construct
  source 1..21: mol_type = other RNA
tcttgtccagctttattggtt

SEQ ID NO: 803 - RNA, 21 nt, synthetic construct
  source 1..21: mol_type = other RNA
ttcttgtccagctttattgtt

SEQ ID NO: 804 - RNA, 21 nt, synthetic construct
  source 1..21: mol_type = other RNA
tttcttgtccagctttatttt

SEQ ID NO: 805 - RNA, 21 nt, synthetic construct
  source 1..21: mol_type = other RNA
acttcttgtccagctttattt

SEQ ID NO: 806 - RNA, 21 nt, synthetic construct
  source 1..21: mol_type = other RNA
agcttcttgtccagctttatt

SEQ ID NO: 807 - RNA, 21 nt, synthetic construct
  source 1..21: mol_type = other RNA
tagcttcttgtccagcttttt

SEQ ID NO: 808 - RNA, 21 nt, synthetic construct
  source 1..21: mol_type = other RNA
acagcttcttgtccagctttt

SEQ ID NO: 809 - RNA, 21 nt, synthetic construct
  source 1..21: mol_type = other RNA
agcagcttcttgtccagcttt

SEQ ID NO: 810 - RNA, 21 nt, synthetic construct
  source 1..21: mol_type = other RNA
tagcagcttcttgtccagctt

SEQ ID NO: 811 - RNA, 21 nt, synthetic construct
  source 1..21: mol_type = other RNA
atagcagcttcttgtccagtt

SEQ ID NO: 812 - RNA, 21 nt, synthetic construct
  source 1..21: mol_type = other RNA
tatagcagcttcttgtccatt

SEQ ID NO: 813 - RNA, 21 nt, synthetic construct
  source 1..21: mol_type = other RNA
tcatagcagcttcttgtcctt

SEQ ID NO: 814 - RNA, 21 nt, synthetic construct
  source 1..21: mol_type = other RNA
tcactgagaatactgtcccgt

SEQ ID NO: 815 - RNA, 23 nt, synthetic construct
  source 1..23: mol_type = other RNA
gcactgagaatactgtccctttt

SEQ ID NO: 816 - RNA, 21 nt, synthetic construct
  source 1..21: mol_type = other RNA
agaatactgtcccttttaatt

SEQ ID NO: 817 - RNA, 21 nt, synthetic construct
  source 1..21: mol_type = other RNA
actgagaatactgtccctttt

SEQ ID NO: 818 - RNA, 21 nt, synthetic construct
  source 1..21: mol_type = other RNA
aataggcaggtggacttggtt

SEQ ID NO: 819 - RNA, 21 nt, synthetic construct
  source 1..21: mol_type = other RNA
aagaacttgtccttaacggtt

SEQ ID NO: 820 - RNA, 21 nt, synthetic construct
  source 1..21: mol_type = other RNA
aagaagggaggcatcctcgtt

SEQ ID NO: 821 - RNA, 21 nt, synthetic construct
  source 1..21: mol_type = other RNA
tctgagaatactgtccctttt

SEQ ID NO: 822 - RNA, 21 nt, synthetic construct
  source 1..21: mol_type = other RNA
actgagaatactgtccctttt

SEQ ID NO: 823 - RNA, 21 nt, synthetic construct
  source 1..21: mol_type = other RNA
actgagaatactgtccctttt

SEQ ID NO: 824 - RNA, 23 nt, synthetic construct
  source 1..23: mol_type = other RNA
actgagaatactgtcccttttaa

SEQ ID NO: 825 - RNA, 21 nt, synthetic construct
  source 1..21: mol_type = other RNA
tctgagaatactgtccctttt

SEQ ID NO: 826 - RNA, 21 nt, synthetic construct
  source 1..21: mol_type = other RNA
tctgagaatactgtccctttt

SEQ ID NO: 827 - RNA, 19 nt, synthetic construct
  source 1..19: mol_type = other RNA
aggcagctgctccaggaat

SEQ ID NO: 828 - RNA, 19 nt, synthetic construct
  source 1..19: mol_type = other RNA
ggcagctgctccaggaaca

SEQ ID NO: 829 - RNA, 19 nt, synthetic construct
  source 1..19: mol_type = other RNA
gcagctgctccaggaacaa

SEQ ID NO: 830 - RNA, 19 nt, synthetic construct
  source 1..19: mol_type = other RNA
cagctgctccaggaacaga

SEQ ID NO: 831 - RNA, 19 nt, synthetic construct
  source 1..19: mol_type = other RNA
agctgctccaggaacagaa

SEQ ID NO: 832 - RNA, 19 nt, synthetic construct
  source 1..19: mol_type = other RNA
gctgctccaggaacagaga

SEQ ID NO: 833 - RNA, 19 nt, synthetic construct
  source 1..19: mol_type = other RNA
tgctccaggaacagaggta

SEQ ID NO: 834 - RNA, 19 nt, synthetic construct
  source 1..19: mol_type = other RNA
caggaacagaggtgccata

SEQ ID NO: 835 - RNA, 19 nt, synthetic construct
  source 1..19: mol_type = other RNA
aggaacagaggtgccatgt

SEQ ID NO: 836 - RNA, 19 nt, synthetic construct
  source 1..19: mol_type = other RNA
ggaacagaggtgccatgca

SEQ ID NO: 837 - RNA, 19 nt, synthetic construct
  source 1..19: mol_type = other RNA
gaacagaggtgccatgcaa

SEQ ID NO: 838 - RNA, 19 nt, synthetic construct
  source 1..19: mol_type = other RNA
aacagaggtgccatgcagt

SEQ ID NO: 839 - RNA, 19 nt, synthetic construct
  source 1..19: mol_type = other RNA
catgcagccccgggtactt

SEQ ID NO: 840 - RNA, 19 nt, synthetic construct
  source 1..19: mol_type = other RNA
atgcagccccgggtactct

SEQ ID NO: 841 - RNA, 19 nt, synthetic construct
  source 1..19: mol_type = other RNA
tgcagccccgggtactcct

SEQ ID NO: 842 - RNA, 19 nt, synthetic construct
  source 1..19: mol_type = other RNA
gcagccccgggtactcctt

SEQ ID NO: 843 - RNA, 19 nt, synthetic construct
  source 1..19: mol_type = other RNA
cagccccgggtactcctta

SEQ ID NO: 844 - RNA, 19 nt, synthetic construct
  source 1..19: mol_type = other RNA
agccccgggtactccttgt

SEQ ID NO: 845 - RNA, 19 nt, synthetic construct
  source 1..19: mol_type = other RNA
gccccgggtactccttgtt

SEQ ID NO: 846 - RNA, 19 nt, synthetic construct
  source 1..19: mol_type = other RNA
ccccgggtactccttgtta

SEQ ID NO: 847 - RNA, 19 nt, synthetic construct
  source 1..19: mol_type = other RNA
cccgggtactccttgttgt

SEQ ID NO: 848 - RNA, 19 nt, synthetic construct
  source 1..19: mol_type = other RNA
ccgggtactccttgttgtt

SEQ ID NO: 849 - RNA, 19 nt, synthetic construct
  source 1..19: mol_type = other RNA
cgggtactccttgttgtta

SEQ ID NO: 850 - RNA, 19 nt, synthetic construct
  source 1..19: mol_type = other RNA
gggtactccttgttgttgt

SEQ ID NO: 851 - RNA, 19 nt, synthetic construct
  source 1..19: mol_type = other RNA
ggtactccttgttgttgct

SEQ ID NO: 852 - RNA, 19 nt, synthetic construct
  source 1..19: mol_type = other RNA
gtactccttgttgttgcct

SEQ ID NO: 853 - RNA, 19 nt, synthetic construct
  source 1..19: mol_type = other RNA
actccttgttgttgccctt

SEQ ID NO: 854 - RNA, 19 nt, synthetic construct
  source 1..19: mol_type = other RNA
ctccttgttgttgccctct

SEQ ID NO: 855 - RNA, 19 nt, synthetic construct
  source 1..19: mol_type = other RNA
tccttgttgttgccctcct

SEQ ID NO: 856 - RNA, 19 nt, synthetic construct
  source 1..19: mol_type = other RNA
ccttgttgttgccctccta

SEQ ID NO: 857 - RNA, 19 nt, synthetic construct
  source 1..19: mol_type = other RNA
cttgttgttgccctcctga

SEQ ID NO: 858 - RNA, 19 nt, synthetic construct
  source 1..19: mol_type = other RNA
ttgttgttgccctcctggt

SEQ ID NO: 859 - RNA, 19 nt, synthetic construct
  source 1..19: mol_type = other RNA
tgttgttgccctcctggca

SEQ ID NO: 860 - RNA, 19 nt, synthetic construct
  source 1..19: mol_type = other RNA
gccctcctggcgctcctga

SEQ ID NO: 861 - RNA, 19 nt, synthetic construct
  source 1..19: mol_type = other RNA
tcctggcgctcctggcctt

SEQ ID NO: 862 - RNA, 19 nt, synthetic construct
  source 1..19: mol_type = other RNA
ctggcgctcctggcctcta

SEQ ID NO: 863 - RNA, 19 nt, synthetic construct
  source 1..19: mol_type = other RNA
tggcgctcctggcctctgt

SEQ ID NO: 864 - RNA, 19 nt, synthetic construct
  source 1..19: mol_type = other RNA
ggcgctcctggcctctgct

SEQ ID NO: 865 - RNA, 19 nt, synthetic construct
  source 1..19: mol_type = other RNA
gcgctcctggcctctgcct

SEQ ID NO: 866 - RNA, 19 nt, synthetic construct
  source 1..19: mol_type = other RNA
ctggcctctgcccgagctt

SEQ ID NO: 867 - RNA, 19 nt, synthetic construct
  source 1..19: mol_type = other RNA
tggcctctgcccgagcttt

SEQ ID NO: 868 - RNA, 19 nt, synthetic construct
  source 1..19: mol_type = other RNA
ggcctctgcccgagcttca

SEQ ID NO: 869 - RNA, 19 nt, synthetic construct
  source 1..19: mol_type = other RNA
gcctctgcccgagcttcaa

SEQ ID NO: 870 - RNA, 19 nt, synthetic construct
  source 1..19: mol_type = other RNA
cctctgcccgagcttcaga

SEQ ID NO: 871 - RNA, 19 nt, synthetic construct
  source 1..19: mol_type = other RNA
ctctgcccgagcttcagaa

SEQ ID NO: 872 - RNA, 19 nt, synthetic construct
  source 1..19: mol_type = other RNA
tctgcccgagcttcagaga

SEQ ID NO: 873 - RNA, 19 nt, synthetic construct
  source 1..19: mol_type = other RNA
ctgcccgagcttcagaggt

SEQ ID NO: 874 - RNA, 19 nt, synthetic construct
  source 1..19: mol_type = other RNA
tgcccgagcttcagaggct

SEQ ID NO: 875 - RNA, 19 nt, synthetic construct
  source 1..19: mol_type = other RNA
agcttcagaggccgaggat

SEQ ID NO: 876 - RNA, 19 nt, synthetic construct
  source 1..19: mol_type = other RNA
gcttcagaggccgaggata

SEQ ID NO: 877 - RNA, 19 nt, synthetic construct
  source 1..19: mol_type = other RNA
cttcagaggccgaggatgt

SEQ ID NO: 878 - RNA, 19 nt, synthetic construct
  source 1..19: mol_type = other RNA
ttcagaggccgaggatgct

SEQ ID NO: 879 - RNA, 19 nt, synthetic construct
  source 1..19: mol_type = other RNA
tcagaggccgaggatgcct

SEQ ID NO: 880 - RNA, 19 nt, synthetic construct
  source 1..19: mol_type = other RNA
cagaggccgaggatgcctt

SEQ ID NO: 881 - RNA, 19 nt, synthetic construct
  source 1..19: mol_type = other RNA
agaggccgaggatgcctct

SEQ ID NO: 882 - RNA, 19 nt, synthetic construct
  source 1..19: mol_type = other RNA
gaggccgaggatgcctcct

SEQ ID NO: 883 - RNA, 19 nt, synthetic construct
  source 1..19: mol_type = other RNA
ggccgaggatgcctccctt

SEQ ID NO: 884 - RNA, 19 nt, synthetic construct
  source 1..19: mol_type = other RNA
gccgaggatgcctcccttt

SEQ ID NO: 885 - RNA, 19 nt, synthetic construct
  source 1..19: mol_type = other RNA
ccgaggatgcctcccttct

SEQ ID NO: 886 - RNA, 19 nt, synthetic construct
  source 1..19: mol_type = other RNA
cgaggatgcctcccttctt

SEQ ID NO: 887 - RNA, 19 nt, synthetic construct
  source 1..19: mol_type = other RNA
gaggatgcctcccttctca

SEQ ID NO: 888 - RNA, 19 nt, synthetic construct
  source 1..19: mol_type = other RNA
aggatgcctcccttctcaa

SEQ ID NO: 889 - RNA, 19 nt, synthetic construct
  source 1..19: mol_type = other RNA
ggatgcctcccttctcagt

SEQ ID NO: 890 - RNA, 19 nt, synthetic construct
  source 1..19: mol_type = other RNA
gatgcctcccttctcagct

SEQ ID NO: 891 - RNA, 19 nt, synthetic construct
  source 1..19: mol_type = other RNA
atgcctcccttctcagctt

SEQ ID NO: 892 - RNA, 19 nt, synthetic construct
  source 1..19: mol_type = other RNA
tgcctcccttctcagcttt

SEQ ID NO: 893 - RNA, 19 nt, synthetic construct
  source 1..19: mol_type = other RNA
gcctcccttctcagcttca

SEQ ID NO: 894 - RNA, 19 nt, synthetic construct
  source 1..19: mol_type = other RNA
cctcccttctcagcttcat

SEQ ID NO: 895 - RNA, 19 nt, synthetic construct
  source 1..19: mol_type = other RNA
ctcccttctcagcttcata

SEQ ID NO: 896 - RNA, 19 nt, synthetic construct
  source 1..19: mol_type = other RNA
tcccttctcagcttcatgt

SEQ ID NO: 897 - RNA, 19 nt, synthetic construct
  source 1..19: mol_type = other RNA
cccttctcagcttcatgca

SEQ ID NO: 898 - RNA, 19 nt, synthetic construct
  source 1..19: mol_type = other RNA
ccttctcagcttcatgcaa

SEQ ID NO: 899 - RNA, 19 nt, synthetic construct
  source 1..19: mol_type = other RNA
cttctcagcttcatgcaga

SEQ ID NO: 900 - RNA, 19 nt, synthetic construct
  source 1..19: mol_type = other RNA
ttctcagcttcatgcagga

SEQ ID NO: 901 - RNA, 19 nt, synthetic construct
  source 1..19: mol_type = other RNA
tctcagcttcatgcagggt

SEQ ID NO: 902 - RNA, 19 nt, synthetic construct
  source 1..19: mol_type = other RNA
ctcagcttcatgcagggtt

SEQ ID NO: 903 - RNA, 19 nt, synthetic construct
  source 1..19: mol_type = other RNA
tcagcttcatgcagggtta

SEQ ID NO: 904 - RNA, 19 nt, synthetic construct
  source 1..19: mol_type = other RNA
cagcttcatgcagggttat

SEQ ID NO: 905 - RNA, 19 nt, synthetic construct
  source 1..19: mol_type = other RNA
agcttcatgcagggttaca

SEQ ID NO: 906 - RNA, 19 nt, synthetic construct
  source 1..19: mol_type = other RNA
gcttcatgcagggttacat

SEQ ID NO: 907 - RNA, 19 nt, synthetic construct
  source 1..19: mol_type = other RNA
cttcatgcagggttacata

SEQ ID NO: 908 - RNA, 19 nt, synthetic construct
  source 1..19: mol_type = other RNA
ttcatgcagggttacatga

SEQ ID NO: 909 - RNA, 19 nt, synthetic construct
  source 1..19: mol_type = other RNA
tcatgcagggttacatgaa

SEQ ID NO: 910 - RNA, 19 nt, synthetic construct
  source 1..19: mol_type = other RNA
catgcagggttacatgaaa

SEQ ID NO: 911 - RNA, 19 nt, synthetic construct
  source 1..19: mol_type = other RNA
atgcagggttacatgaagt

SEQ ID NO: 912 - RNA, 19 nt, synthetic construct
  source 1..19: mol_type = other RNA
tgcagggttacatgaagca

SEQ ID NO: 913 - RNA, 19 nt, synthetic construct
  source 1..19: mol_type = other RNA
gcagggttacatgaagcat

SEQ ID NO: 914 - RNA, 19 nt, synthetic construct
  source 1..19: mol_type = other RNA
cagggttacatgaagcaca

SEQ ID NO: 915 - RNA, 19 nt, synthetic construct
  source 1..19: mol_type = other RNA
agggttacatgaagcacgt

SEQ ID NO: 916 - RNA, 19 nt, synthetic construct
  source 1..19: mol_type = other RNA
gggttacatgaagcacgct

SEQ ID NO: 917 - RNA, 19 nt, synthetic construct
  source 1..19: mol_type = other RNA
gttacatgaagcacgccat

SEQ ID NO: 918 - RNA, 19 nt, synthetic construct
  source 1..19: mol_type = other RNA
acatgaagcacgccaccaa

SEQ ID NO: 919 - RNA, 19 nt, synthetic construct
  source 1..19: mol_type = other RNA
catgaagcacgccaccaaa

SEQ ID NO: 920 - RNA, 19 nt, synthetic construct
  source 1..19: mol_type = other RNA
atgaagcacgccaccaaga

SEQ ID NO: 921 - RNA, 19 nt, synthetic construct
  source 1..19: mol_type = other RNA
tgaagcacgccaccaagat

SEQ ID NO: 922 - RNA, 19 nt, synthetic construct
  source 1..19: mol_type = other RNA
gaagcacgccaccaagact

SEQ ID NO: 923 - RNA, 19 nt, synthetic construct
  source 1..19: mol_type = other RNA
aagcacgccaccaagacca

SEQ ID NO: 924 - RNA, 19 nt, synthetic construct
  source 1..19: mol_type = other RNA
agcacgccaccaagaccgt

SEQ ID NO: 925 - RNA, 19 nt, synthetic construct
  source 1..19: mol_type = other RNA
gcacgccaccaagaccgct

SEQ ID NO: 926 - RNA, 19 nt, synthetic construct
  source 1..19: mol_type = other RNA
cgccaccaagaccgccaaa

SEQ ID NO: 927 - RNA, 19 nt, synthetic construct
  source 1..19: mol_type = other RNA
gccaccaagaccgccaaga

SEQ ID NO: 928 - RNA, 19 nt, synthetic construct
  source 1..19: mol_type = other RNA
ccaccaagaccgccaagga

SEQ ID NO: 929 - RNA, 19 nt, synthetic construct
  source 1..19: mol_type = other RNA
caccaagaccgccaaggat

SEQ ID NO: 930 - RNA, 19 nt, synthetic construct
  source 1..19: mol_type = other RNA
accaagaccgccaaggata

SEQ ID NO: 931 - RNA, 19 nt, synthetic construct
  source 1..19: mol_type = other RNA
ccaagaccgccaaggatgt

SEQ ID NO: 932 - RNA, 19 nt, synthetic construct
  source 1..19: mol_type = other RNA
caagaccgccaaggatgca

SEQ ID NO: 933 - RNA, 19 nt, synthetic construct
  source 1..19: mol_type = other RNA
aagaccgccaaggatgcat

SEQ ID NO: 934 - RNA, 19 nt, synthetic construct
  source 1..19: mol_type = other RNA
agaccgccaaggatgcact

SEQ ID NO: 935 - RNA, 19 nt, synthetic construct
  source 1..19: mol_type = other RNA
gaccgccaaggatgcacta

SEQ ID NO: 936 - RNA, 19 nt, synthetic construct
  source 1..19: mol_type = other RNA
accgccaaggatgcactga

SEQ ID NO: 937 - RNA, 19 nt, synthetic construct
  source 1..19: mol_type = other RNA
ccgccaaggatgcactgaa

SEQ ID NO: 938 - RNA, 19 nt, synthetic construct
  source 1..19: mol_type = other RNA
cgccaaggatgcactgagt

SEQ ID NO: 939 - RNA, 19 nt, synthetic construct
  source 1..19: mol_type = other RNA
gccaaggatgcactgagca

SEQ ID NO: 940 - RNA, 19 nt, synthetic construct
  source 1..19: mol_type = other RNA
ccaaggatgcactgagcaa

SEQ ID NO: 941 - RNA, 19 nt, synthetic construct
  source 1..19: mol_type = other RNA
caaggatgcactgagcagt

SEQ ID NO: 942 - RNA, 19 nt, synthetic construct
  source 1..19: mol_type = other RNA
aaggatgcactgagcagca

SEQ ID NO: 943 - RNA, 19 nt, synthetic construct
  source 1..19: mol_type = other RNA
aggatgcactgagcagcgt

SEQ ID NO: 944 - RNA, 19 nt, synthetic construct
  source 1..19: mol_type = other RNA
ggatgcactgagcagcgta

SEQ ID NO: 945 - RNA, 19 nt, synthetic construct
  source 1..19: mol_type = other RNA
gatgcactgagcagcgtgt

SEQ ID NO: 946 - RNA, 19 nt, synthetic construct
  source 1..19: mol_type = other RNA
atgcactgagcagcgtgca

SEQ ID NO: 947 - RNA, 19 nt, synthetic construct
  source 1..19: mol_type = other RNA
tgcactgagcagcgtgcaa

SEQ ID NO: 948 - RNA, 19 nt, synthetic construct
  source 1..19: mol_type = other RNA
gcactgagcagcgtgcaga

SEQ ID NO: 949 - RNA, 19 nt, synthetic construct
  source 1..19: mol_type = other RNA
cactgagcagcgtgcagga

SEQ ID NO: 950 - RNA, 19 nt, synthetic construct
  source 1..19: mol_type = other RNA
actgagcagcgtgcaggaa

SEQ ID NO: 951 - RNA, 19 nt, synthetic construct
  source 1..19: mol_type = other RNA
ctgagcagcgtgcaggagt

SEQ ID NO: 952 - RNA, 19 nt, synthetic construct
  source 1..19: mol_type = other RNA
tgagcagcgtgcaggagtt

SEQ ID NO: 953 - RNA, 19 nt, synthetic construct
  source 1..19: mol_type = other RNA
gagcagcgtgcaggagtct

SEQ ID NO: 954 - RNA, 19 nt, synthetic construct
  source 1..19: mol_type = other RNA
agcagcgtgcaggagtcct

SEQ ID NO: 955 - RNA, 19 nt, synthetic construct
  source 1..19: mol_type = other RNA
gcagcgtgcaggagtccca

SEQ ID NO: 956 - RNA, 19 nt, synthetic construct
  source 1..19: mol_type = other RNA
cagcgtgcaggagtcccaa

SEQ ID NO: 957 - RNA, 19 nt, synthetic construct
  source 1..19: mol_type = other RNA
agcgtgcaggagtcccaga

SEQ ID NO: 958 - RNA, 19 nt, synthetic construct
  source 1..19: mol_type = other RNA
gcgtgcaggagtcccaggt

SEQ ID NO: 959 - RNA, 19 nt, synthetic construct
  source 1..19: mol_type = other RNA
cgtgcaggagtcccaggta

SEQ ID NO: 960 - RNA, 19 nt, synthetic construct
  source 1..19: mol_type = other RNA
gtgcaggagtcccaggtga

SEQ ID NO: 961 - RNA, 19 nt, synthetic construct
  source 1..19: mol_type = other RNA
tgcaggagtcccaggtggt

SEQ ID NO: 962 - RNA, 19 nt, synthetic construct
  source 1..19: mol_type = other RNA
gtcccaggtggcccagcaa

SEQ ID NO: 963 - RNA, 19 nt, synthetic construct
  source 1..19: mol_type = other RNA
tcccaggtggcccagcaga

SEQ ID NO: 964 - RNA, 19 nt, synthetic construct
  source 1..19: mol_type = other RNA
cccaggtggcccagcaggt

SEQ ID NO: 965 - RNA, 19 nt, synthetic construct
  source 1..19: mol_type = other RNA
ccaggtggcccagcaggct

SEQ ID NO: 966 - RNA, 19 nt, synthetic construct
  source 1..19: mol_type = other RNA
caggtggcccagcaggcca

SEQ ID NO: 967 - RNA, 19 nt, synthetic construct
  source 1..19: mol_type = other RNA
aggtggcccagcaggccaa

SEQ ID NO: 968 - RNA, 19 nt, synthetic construct
  source 1..19: mol_type = other RNA
ggtggcccagcaggccaga

SEQ ID NO: 969 - RNA, 19 nt, synthetic construct
  source 1..19: mol_type = other RNA
gtggcccagcaggccagga

SEQ ID NO: 970 - RNA, 19 nt, synthetic construct
  source 1..19: mol_type = other RNA
gcaggccaggggctgggta

SEQ ID NO: 971 - RNA, 19 nt, synthetic construct
  source 1..19: mol_type = other RNA
caggccaggggctgggtga

SEQ ID NO: 972 - RNA, 19 nt, synthetic construct
  source 1..19: mol_type = other RNA
aggccaggggctgggtgat

SEQ ID NO: 973 - RNA, 19 nt, synthetic construct
  source 1..19: mol_type = other RNA
ggccaggggctgggtgact

SEQ ID NO: 974 - RNA, 19 nt, synthetic construct
  source 1..19: mol_type = other RNA
gccaggggctgggtgacca

SEQ ID NO: 975 - RNA, 19 nt, synthetic construct
  source 1..19: mol_type = other RNA
ccaggggctgggtgaccga

SEQ ID NO: 976 - RNA, 19 nt, synthetic construct
  source 1..19: mol_type = other RNA
caggggctgggtgaccgat

SEQ ID NO: 977 - RNA, 19 nt, synthetic construct
  source 1..19: mol_type = other RNA
aggggctgggtgaccgata

SEQ ID NO: 978 - RNA, 19 nt, synthetic construct
  source 1..19: mol_type = other RNA
ggggctgggtgaccgatga

SEQ ID NO: 979 - RNA, 19 nt, synthetic construct
  source 1..19: mol_type = other RNA
gggctgggtgaccgatggt

SEQ ID NO: 980 - RNA, 19 nt, synthetic construct
  source 1..19: mol_type = other RNA
ggctgggtgaccgatggct

SEQ ID NO: 981 - RNA, 19 nt, synthetic construct
  source 1..19: mol_type = other RNA
gctgggtgaccgatggctt

SEQ ID NO: 982 - RNA, 19 nt, synthetic construct
  source 1..19: mol_type = other RNA
ctgggtgaccgatggcttt

SEQ ID NO: 983 - RNA, 19 nt, synthetic construct
  source 1..19: mol_type = other RNA
tgggtgaccgatggcttca

SEQ ID NO: 984 - RNA, 19 nt, synthetic construct
  source 1..19: mol_type = other RNA
gggtgaccgatggcttcaa

SEQ ID NO: 985 - RNA, 19 nt, synthetic construct
  source 1..19: mol_type = other RNA
ggtgaccgatggcttcagt

SEQ ID NO: 986 - RNA, 19 nt, synthetic construct
  source 1..19: mol_type = other RNA
gtgaccgatggcttcagtt

SEQ ID NO: 987 - RNA, 19 nt, synthetic construct
  source 1..19: mol_type = other RNA
tgaccgatggcttcagttt

SEQ ID NO: 988 - RNA, 19 nt, synthetic construct
  source 1..19: mol_type = other RNA
gaccgatggcttcagttct

SEQ ID NO: 989 - RNA, 19 nt, synthetic construct
  source 1..19: mol_type = other RNA
accgatggcttcagttcct

SEQ ID NO: 990 - RNA, 19 nt, synthetic construct
  source 1..19: mol_type = other RNA
ccgatggcttcagttccct

SEQ ID NO: 991 - RNA, 19 nt, synthetic construct
  source 1..19: mol_type = other RNA
cgatggcttcagttcccta

SEQ ID NO: 992 - RNA, 19 nt, synthetic construct
  source 1..19: mol_type = other RNA
gatggcttcagttccctga

SEQ ID NO: 993 - RNA, 19 nt, synthetic construct
  source 1..19: mol_type = other RNA
atggcttcagttccctgaa

SEQ ID NO: 994 - RNA, 19 nt, synthetic construct
  source 1..19: mol_type = other RNA
tggcttcagttccctgaaa

SEQ ID NO: 995 - RNA, 19 nt, synthetic construct
  source 1..19: mol_type = other RNA
ggcttcagttccctgaaaa

SEQ ID NO: 996 - RNA, 19 nt, synthetic construct
  source 1..19: mol_type = other RNA
gcttcagttccctgaaaga

SEQ ID NO: 997 - RNA, 19 nt, synthetic construct
  source 1..19: mol_type = other RNA
cttcagttccctgaaagat

SEQ ID NO: 998 - RNA, 19 nt, synthetic construct
  source 1..19: mol_type = other RNA
ttcagttccctgaaagact

SEQ ID NO: 999 - RNA, 19 nt, synthetic construct
  source 1..19: mol_type = other RNA
tcagttccctgaaagacta

SEQ ID NO: 1000 - RNA, 19 nt, synthetic construct
  source 1..19: mol_type = other RNA
cagttccctgaaagactat

SEQ ID NO: 1001 - RNA, 19 nt, synthetic construct
  source 1..19: mol_type = other RNA
agttccctgaaagactact

SEQ ID NO: 1002 - RNA, 19 nt, synthetic construct
  source 1..19: mol_type = other RNA
gttccctgaaagactacta

SEQ ID NO: 1003 - RNA, 19 nt, synthetic construct
  source 1..19: mol_type = other RNA
ttccctgaaagactactga

SEQ ID NO: 1004 - RNA, 19 nt, synthetic construct
  source 1..19: mol_type = other RNA
tccctgaaagactactgga

SEQ ID NO: 1005 - RNA, 19 nt, synthetic construct
  source 1..19: mol_type = other RNA
ccctgaaagactactggaa

SEQ ID NO: 1006 - RNA, 19 nt, synthetic construct
  source 1..19: mol_type = other RNA
cctgaaagactactggagt

SEQ ID NO: 1007 - RNA, 19 nt, synthetic construct
  source 1..19: mol_type = other RNA
ctgaaagactactggagca

SEQ ID NO: 1008 - RNA, 19 nt, synthetic construct
  source 1..19: mol_type = other RNA
tgaaagactactggagcat

SEQ ID NO: 1009 - RNA, 19 nt, synthetic construct
  source 1..19: mol_type = other RNA
gaaagactactggagcact

SEQ ID NO: 1010 - RNA, 19 nt, synthetic construct
  source 1..19: mol_type = other RNA
aaagactactggagcacca

SEQ ID NO: 1011 - RNA, 19 nt, synthetic construct
  source 1..19: mol_type = other RNA
agactactggagcaccgtt

SEQ ID NO: 1012 - RNA, 19 nt, synthetic construct
  source 1..19: mol_type = other RNA
gactactggagcaccgtta

SEQ ID NO: 1013 - RNA, 19 nt, synthetic construct
  source 1..19: mol_type = other RNA
actactggagcaccgttaa

SEQ ID NO: 1014 - RNA, 19 nt, synthetic construct
  source 1..19: mol_type = other RNA
ctactggagcaccgttaaa

SEQ ID NO: 1015 - RNA, 19 nt, synthetic construct
  source 1..19: mol_type = other RNA
tactggagcaccgttaaga

SEQ ID NO: 1016 - RNA, 19 nt, synthetic construct
  source 1..19: mol_type = other RNA
actggagcaccgttaagga

SEQ ID NO: 1017 - RNA, 19 nt, synthetic construct
  source 1..19: mol_type = other RNA
ctggagcaccgttaaggat

SEQ ID NO: 1018 - RNA, 19 nt, synthetic construct
  source 1..19: mol_type = other RNA
tggagcaccgttaaggaca

SEQ ID NO: 1019 - RNA, 19 nt, synthetic construct
  source 1..19: mol_type = other RNA
ggagcaccgttaaggacaa

SEQ ID NO: 1020 - RNA, 19 nt, synthetic construct
  source 1..19: mol_type = other RNA
gagcaccgttaaggacaaa

SEQ ID NO: 1021 - RNA, 19 nt, synthetic construct
  source 1..19: mol_type = other RNA
agcaccgttaaggacaagt

SEQ ID NO: 1022 - RNA, 19 nt, synthetic construct
  source 1..19: mol_type = other RNA
gcaccgttaaggacaagtt

SEQ ID NO: 1023 - RNA, 19 nt, synthetic construct
  source 1..19: mol_type = other RNA
caccgttaaggacaagttt

SEQ ID NO: 1024 - RNA, 19 nt, synthetic construct
  source 1..19: mol_type = other RNA
accgttaaggacaagttct

SEQ ID NO: 1025 - RNA, 19 nt, synthetic construct
  source 1..19: mol_type = other RNA
ccgttaaggacaagttctt

SEQ ID NO: 1026 - RNA, 19 nt, synthetic construct
  source 1..19: mol_type = other RNA
cgttaaggacaagttctct

SEQ ID NO: 1027 - RNA, 19 nt, synthetic construct
  source 1..19: mol_type = other RNA
gttaaggacaagttctcta

SEQ ID NO: 1028 - RNA, 19 nt, synthetic construct
  source 1..19: mol_type = other RNA
ttaaggacaagttctctga

SEQ ID NO: 1029 - RNA, 19 nt, synthetic construct
  source 1..19: mol_type = other RNA
taaggacaagttctctgaa

SEQ ID NO: 1030 - RNA, 19 nt, synthetic construct
  source 1..19: mol_type = other RNA
aaggacaagttctctgagt

SEQ ID NO: 1031 - RNA, 19 nt, synthetic construct
  source 1..19: mol_type = other RNA
aggacaagttctctgagtt

SEQ ID NO: 1032 - RNA, 19 nt, synthetic construct
  source 1..19: mol_type = other RNA
ggacaagttctctgagttt

SEQ ID NO: 1033 - RNA, 19 nt, synthetic construct
  source 1..19: mol_type = other RNA
gacaagttctctgagttct

SEQ ID NO: 1034 - RNA, 19 nt, synthetic construct
  source 1..19: mol_type = other RNA
acaagttctctgagttcta

SEQ ID NO: 1035 - RNA, 19 nt, synthetic construct
  source 1..19: mol_type = other RNA
caagttctctgagttctga

SEQ ID NO: 1036 - RNA, 19 nt, synthetic construct
  source 1..19: mol_type = other RNA
aagttctctgagttctgga

SEQ ID NO: 1037 - RNA, 19 nt, synthetic construct
  source 1..19: mol_type = other RNA
agttctctgagttctggga

SEQ ID NO: 1038 - RNA, 19 nt, synthetic construct
  source 1..19: mol_type = other RNA
gttctctgagttctgggat

SEQ ID NO: 1039 - RNA, 19 nt, synthetic construct
  source 1..19: mol_type = other RNA
ttctctgagttctgggatt

SEQ ID NO: 1040 - RNA, 19 nt, synthetic construct
  source 1..19: mol_type = other RNA
tctctgagttctgggattt

SEQ ID NO: 1041 - RNA, 19 nt, synthetic construct
  source 1..19: mol_type = other RNA
ctctgagttctgggattta

SEQ ID NO: 1042 - RNA, 19 nt, synthetic construct
  source 1..19: mol_type = other RNA
tctgagttctgggatttga

SEQ ID NO: 1043 - RNA, 19 nt, synthetic construct
  source 1..19: mol_type = other RNA
ctgagttctgggatttgga

SEQ ID NO: 1044 - RNA, 19 nt, synthetic construct
  source 1..19: mol_type = other RNA
tgagttctgggatttggat

SEQ ID NO: 1045 - RNA, 19 nt, synthetic construct
  source 1..19: mol_type = other RNA
gagttctgggatttggact

SEQ ID NO: 1046 - RNA, 19 nt, synthetic construct
  source 1..19: mol_type = other RNA
agttctgggatttggacct

SEQ ID NO: 1047 - RNA, 19 nt, synthetic construct
  source 1..19: mol_type = other RNA
ttctgggatttggacccta

SEQ ID NO: 1048 - RNA, 19 nt, synthetic construct
  source 1..19: mol_type = other RNA
tctgggatttggaccctga

SEQ ID NO: 1049 - RNA, 19 nt, synthetic construct
  source 1..19: mol_type = other RNA
ctgggatttggaccctgaa

SEQ ID NO: 1050 - RNA, 19 nt, synthetic construct
  source 1..19: mol_type = other RNA
tgggatttggaccctgaga

SEQ ID NO: 1051 - RNA, 19 nt, synthetic construct
  source 1..19: mol_type = other RNA
gggatttggaccctgaggt

SEQ ID NO: 1052 - RNA, 19 nt, synthetic construct
  source 1..19: mol_type = other RNA
ggatttggaccctgaggtt

SEQ ID NO: 1053 - RNA, 19 nt, synthetic construct
  source 1..19: mol_type = other RNA
gatttggaccctgaggtca

SEQ ID NO: 1054 - RNA, 19 nt, synthetic construct
  source 1..19: mol_type = other RNA
atttggaccctgaggtcaa

SEQ ID NO: 1055 - RNA, 19 nt, synthetic construct
  source 1..19: mol_type = other RNA
tttggaccctgaggtcaga

SEQ ID NO: 1056 - RNA, 19 nt, synthetic construct
  source 1..19: mol_type = other RNA
ttggaccctgaggtcagat

SEQ ID NO: 1057 - RNA, 19 nt, synthetic construct
  source 1..19: mol_type = other RNA
tggaccctgaggtcagact

SEQ ID NO: 1058 - RNA, 19 nt, synthetic construct
  source 1..19: mol_type = other RNA
ggaccctgaggtcagacca

SEQ ID NO: 1059 - RNA, 19 nt, synthetic construct
  source 1..19: mol_type = other RNA
gaccctgaggtcagaccaa

SEQ ID NO: 1060 - RNA, 19 nt, synthetic construct
  source 1..19: mol_type = other RNA
accctgaggtcagaccaat

SEQ ID NO: 1061 - RNA, 19 nt, synthetic construct
  source 1..19: mol_type = other RNA
ccctgaggtcagaccaact

SEQ ID NO: 1062 - RNA, 19 nt, synthetic construct
  source 1..19: mol_type = other RNA
cctgaggtcagaccaactt

SEQ ID NO: 1063 - RNA, 19 nt, synthetic construct
  source 1..19: mol_type = other RNA
ctgaggtcagaccaacttt

SEQ ID NO: 1064 - RNA, 19 nt, synthetic construct
  source 1..19: mol_type = other RNA
tgaggtcagaccaacttca

SEQ ID NO: 1065 - RNA, 19 nt, synthetic construct
  source 1..19: mol_type = other RNA
gaggtcagaccaacttcaa

SEQ ID NO: 1066 - RNA, 19 nt, synthetic construct
  source 1..19: mol_type = other RNA
aggtcagaccaacttcagt

SEQ ID NO: 1067 - RNA, 19 nt, synthetic construct
  source 1..19: mol_type = other RNA
ggtcagaccaacttcagct

SEQ ID NO: 1068 - RNA, 19 nt, synthetic construct
  source 1..19: mol_type = other RNA
gtcagaccaacttcagcca

SEQ ID NO: 1069 - RNA, 19 nt, synthetic construct
  source 1..19: mol_type = other RNA
ccaacttcagccgtggcta

SEQ ID NO: 1070 - RNA, 19 nt, synthetic construct
  source 1..19: mol_type = other RNA
caacttcagccgtggctgt

SEQ ID NO: 1071 - RNA, 19 nt, synthetic construct
  source 1..19: mol_type = other RNA
aacttcagccgtggctgct

SEQ ID NO: 1072 - RNA, 19 nt, synthetic construct
  source 1..19: mol_type = other RNA
acttcagccgtggctgcct

SEQ ID NO: 1073 - RNA, 19 nt, synthetic construct
  source 1..19: mol_type = other RNA
cttcagccgtggctgccta

SEQ ID NO: 1074 - RNA, 19 nt, synthetic construct
  source 1..19: mol_type = other RNA
ttcagccgtggctgcctga

SEQ ID NO: 1075 - RNA, 19 nt, synthetic construct
  source 1..19: mol_type = other RNA
tcagccgtggctgcctgaa

SEQ ID NO: 1076 - RNA, 19 nt, synthetic construct
  source 1..19: mol_type = other RNA
cagccgtggctgcctgaga

SEQ ID NO: 1077 - RNA, 19 nt, synthetic construct
  source 1..19: mol_type = other RNA
agccgtggctgcctgagat

SEQ ID NO: 1078 - RNA, 19 nt, synthetic construct
  source 1..19: mol_type = other RNA
gccgtggctgcctgagact

SEQ ID NO: 1079 - RNA, 19 nt, synthetic construct
  source 1..19: mol_type = other RNA
ccgtggctgcctgagacct

SEQ ID NO: 1080 - RNA, 19 nt, synthetic construct
  source 1..19: mol_type = other RNA
cgtggctgcctgagacctt

SEQ ID NO: 1081 - RNA, 19 nt, synthetic construct
  source 1..19: mol_type = other RNA
gtggctgcctgagacctca

SEQ ID NO: 1082 - RNA, 19 nt, synthetic construct
  source 1..19: mol_type = other RNA
tggctgcctgagacctcaa

SEQ ID NO: 1083 - RNA, 19 nt, synthetic construct
  source 1..19: mol_type = other RNA
ggctgcctgagacctcaat

SEQ ID NO: 1084 - RNA, 19 nt, synthetic construct
  source 1..19: mol_type = other RNA
gctgcctgagacctcaata

SEQ ID NO: 1085 - RNA, 19 nt, synthetic construct
  source 1..19: mol_type = other RNA
ctgcctgagacctcaatat

SEQ ID NO: 1086 - RNA, 19 nt, synthetic construct
  source 1..19: mol_type = other RNA
tgcctgagacctcaatact

SEQ ID NO: 1087 - RNA, 19 nt, synthetic construct
  source 1..19: mol_type = other RNA
gcctgagacctcaatacct

SEQ ID NO: 1088 - RNA, 19 nt, synthetic construct
  source 1..19: mol_type = other RNA
cctgagacctcaataccct

SEQ ID NO: 1089 - RNA, 19 nt, synthetic construct
  source 1..19: mol_type = other RNA
tgagacctcaataccccaa

SEQ ID NO: 1090 - RNA, 19 nt, synthetic construct
  source 1..19: mol_type = other RNA
gagacctcaataccccaaa

SEQ ID NO: 1091 - RNA, 19 nt, synthetic construct
  source 1..19: mol_type = other RNA
agacctcaataccccaagt

SEQ ID NO: 1092 - RNA, 19 nt, synthetic construct
  source 1..19: mol_type = other RNA
gacctcaataccccaagtt

SEQ ID NO: 1093 - RNA, 19 nt, synthetic construct
  source 1..19: mol_type = other RNA
acctcaataccccaagtct

SEQ ID NO: 1094 - RNA, 19 nt, synthetic construct
  source 1..19: mol_type = other RNA
cctcaataccccaagtcca

SEQ ID NO: 1095 - RNA, 19 nt, synthetic construct
  source 1..19: mol_type = other RNA
ctcaataccccaagtccat

SEQ ID NO: 1096 - RNA, 19 nt, synthetic construct
  source 1..19: mol_type = other RNA
tcaataccccaagtccact

SEQ ID NO: 1097 - RNA, 19 nt, synthetic construct
  source 1..19: mol_type = other RNA
caataccccaagtccacct

SEQ ID NO: 1098 - RNA, 19 nt, synthetic construct
  source 1..19: mol_type = other RNA
aataccccaagtccaccta

SEQ ID NO: 1099 - RNA, 19 nt, synthetic construct
  source 1..19: mol_type = other RNA
ataccccaagtccacctgt

SEQ ID NO: 1100 - RNA, 19 nt, synthetic construct
  source 1..19: mol_type = other RNA
taccccaagtccacctgct

SEQ ID NO: 1101 - RNA, 19 nt, synthetic construct
  source 1..19: mol_type = other RNA
ccccaagtccacctgccta

SEQ ID NO: 1102 - RNA, 19 nt, synthetic construct
  source 1..19: mol_type = other RNA
cccaagtccacctgcctat

SEQ ID NO: 1103 - RNA, 19 nt, synthetic construct
  source 1..19: mol_type = other RNA
ccaagtccacctgcctatt

SEQ ID NO: 1104 - RNA, 19 nt, synthetic construct
  source 1..19: mol_type = other RNA
caagtccacctgcctatct

SEQ ID NO: 1105 - RNA, 19 nt, synthetic construct
  source 1..19: mol_type = other RNA
aagtccacctgcctatcca

SEQ ID NO: 1106 - RNA, 19 nt, synthetic construct
  source 1..19: mol_type = other RNA
agtccacctgcctatccat

SEQ ID NO: 1107 - RNA, 19 nt, synthetic construct
  source 1..19: mol_type = other RNA
gtccacctgcctatccatt

SEQ ID NO: 1108 - RNA, 19 nt, synthetic construct
  source 1..19: mol_type = other RNA
tccacctgcctatccatct

SEQ ID NO: 1109 - RNA, 19 nt, synthetic construct
  source 1..19: mol_type = other RNA
ccacctgcctatccatcct

SEQ ID NO: 1110 - RNA, 19 nt, synthetic construct
  source 1..19: mol_type = other RNA
cacctgcctatccatccta

SEQ ID NO: 1111 - RNA, 19 nt, synthetic construct
  source 1..19: mol_type = other RNA
acctgcctatccatcctgt

SEQ ID NO: 1112 - RNA, 19 nt, synthetic construct
  source 1..19: mol_type = other RNA
cctgcctatccatcctgca

SEQ ID NO: 1113 - RNA, 19 nt, synthetic construct
  source 1..19: mol_type = other RNA
ctgcctatccatcctgcga

SEQ ID NO: 1114 - RNA, 19 nt, synthetic construct
  source 1..19: mol_type = other RNA
tgcctatccatcctgcgaa

SEQ ID NO: 1115 - RNA, 19 nt, synthetic construct
  source 1..19: mol_type = other RNA
gcctatccatcctgcgagt

SEQ ID NO: 1116 - RNA, 19 nt, synthetic construct
  source 1..19: mol_type = other RNA
cctatccatcctgcgagct

SEQ ID NO: 1117 - RNA, 19 nt, synthetic construct
  source 1..19: mol_type = other RNA
ctatccatcctgcgagctt

SEQ ID NO: 1118 - RNA, 19 nt, synthetic construct
  source 1..19: mol_type = other RNA
tatccatcctgcgagctct

SEQ ID NO: 1119 - RNA, 19 nt, synthetic construct
  source 1..19: mol_type = other RNA
atccatcctgcgagctcct

SEQ ID NO: 1120 - RNA, 19 nt, synthetic construct
  source 1..19: mol_type = other RNA
tccatcctgcgagctcctt

SEQ ID NO: 1121 - RNA, 19 nt, synthetic construct
  source 1..19: mol_type = other RNA
ccatcctgcgagctcctta

SEQ ID NO: 1122 - RNA, 19 nt, synthetic construct
  source 1..19: mol_type = other RNA
catcctgcgagctccttga

SEQ ID NO: 1123 - RNA, 19 nt, synthetic construct
  source 1..19: mol_type = other RNA
atcctgcgagctccttgga

SEQ ID NO: 1124 - RNA, 19 nt, synthetic construct
  source 1..19: mol_type = other RNA
tcctgcgagctccttgggt

SEQ ID NO: 1125 - RNA, 19 nt, synthetic construct
  source 1..19: mol_type = other RNA
cctgcgagctccttgggtt

SEQ ID NO: 1126 - RNA, 19 nt, synthetic construct
  source 1..19: mol_type = other RNA
ctgcgagctccttgggtct

SEQ ID NO: 1127 - RNA, 19 nt, synthetic construct
  source 1..19: mol_type = other RNA
tgcgagctccttgggtcct

SEQ ID NO: 1128 - RNA, 19 nt, synthetic construct
  source 1..19: mol_type = other RNA
gcgagctccttgggtccta

SEQ ID NO: 1129 - RNA, 19 nt, synthetic construct
  source 1..19: mol_type = other RNA
cgagctccttgggtcctgt

SEQ ID NO: 1130 - RNA, 19 nt, synthetic construct
  source 1..19: mol_type = other RNA
gagctccttgggtcctgca

SEQ ID NO: 1131 - RNA, 19 nt, synthetic construct
  source 1..19: mol_type = other RNA
agctccttgggtcctgcaa

SEQ ID NO: 1132 - RNA, 19 nt, synthetic construct
  source 1..19: mol_type = other RNA
gctccttgggtcctgcaat

SEQ ID NO: 1133 - RNA, 19 nt, synthetic construct
  source 1..19: mol_type = other RNA
ctccttgggtcctgcaatt

SEQ ID NO: 1134 - RNA, 19 nt, synthetic construct
  source 1..19: mol_type = other RNA
tccttgggtcctgcaatct

SEQ ID NO: 1135 - RNA, 19 nt, synthetic construct
  source 1..19: mol_type = other RNA
ccttgggtcctgcaatctt

SEQ ID NO: 1136 - RNA, 19 nt, synthetic construct
  source 1..19: mol_type = other RNA
cttgggtcctgcaatctct

SEQ ID NO: 1137 - RNA, 19 nt, synthetic construct
  source 1..19: mol_type = other RNA
ttgggtcctgcaatctcca

SEQ ID NO: 1138 - RNA, 19 nt, synthetic construct
  source 1..19: mol_type = other RNA
tgggtcctgcaatctccaa

SEQ ID NO: 1139 - RNA, 19 nt, synthetic construct
  source 1..19: mol_type = other RNA
gggtcctgcaatctccaga

SEQ ID NO: 1140 - RNA, 19 nt, synthetic construct
  source 1..19: mol_type = other RNA
ggtcctgcaatctccagga

SEQ ID NO: 1141 - RNA, 19 nt, synthetic construct
  source 1..19: mol_type = other RNA
gtcctgcaatctccagggt

SEQ ID NO: 1142 - RNA, 19 nt, synthetic construct
  source 1..19: mol_type = other RNA
cctgcaatctccagggcta

SEQ ID NO: 1143 - RNA, 19 nt, synthetic construct
  source 1..19: mol_type = other RNA
ctgcaatctccagggctgt

SEQ ID NO: 1144 - RNA, 19 nt, synthetic construct
  source 1..19: mol_type = other RNA
tgcaatctccagggctgct

SEQ ID NO: 1145 - RNA, 19 nt, synthetic construct
  source 1..19: mol_type = other RNA
ctccagggctgcccctgta

SEQ ID NO: 1146 - RNA, 19 nt, synthetic construct
  source 1..19: mol_type = other RNA
tccagggctgcccctgtaa

SEQ ID NO: 1147 - RNA, 19 nt, synthetic construct
  source 1..19: mol_type = other RNA
ccagggctgcccctgtaga

SEQ ID NO: 1148 - RNA, 19 nt, synthetic construct
  source 1..19: mol_type = other RNA
cagggctgcccctgtaggt

SEQ ID NO: 1149 - RNA, 19 nt, synthetic construct
  source 1..19: mol_type = other RNA
agggctgcccctgtaggtt

SEQ ID NO: 1150 - RNA, 19 nt, synthetic construct
  source 1..19: mol_type = other RNA
gggctgcccctgtaggtta

SEQ ID NO: 1151 - RNA, 19 nt, synthetic construct
  source 1..19: mol_type = other RNA
ggctgcccctgtaggttgt

SEQ ID NO: 1152 - RNA, 19 nt, synthetic construct
  source 1..19: mol_type = other RNA
gctgcccctgtaggttgct

SEQ ID NO: 1153 - RNA, 19 nt, synthetic construct
  source 1..19: mol_type = other RNA
ctgcccctgtaggttgctt

SEQ ID NO: 1154 - RNA, 19 nt, synthetic construct
  source 1..19: mol_type = other RNA
tgcccctgtaggttgctta

SEQ ID NO: 1155 - RNA, 19 nt, synthetic construct
  source 1..19: mol_type = other RNA
gcccctgtaggttgcttaa

SEQ ID NO: 1156 - RNA, 19 nt, synthetic construct
  source 1..19: mol_type = other RNA
cccctgtaggttgcttaaa

SEQ ID NO: 1157 - RNA, 19 nt, synthetic construct
  source 1..19: mol_type = other RNA
ccctgtaggttgcttaaaa

SEQ ID NO: 1158 - RNA, 19 nt, synthetic construct
  source 1..19: mol_type = other RNA
cctgtaggttgcttaaaaa

SEQ ID NO: 1159 - RNA, 19 nt, synthetic construct
  source 1..19: mol_type = other RNA
ctgtaggttgcttaaaaga

SEQ ID NO: 1160 - RNA, 19 nt, synthetic construct
  source 1..19: mol_type = other RNA
tgtaggttgcttaaaagga

SEQ ID NO: 1161 - RNA, 19 nt, synthetic construct
  source 1..19: mol_type = other RNA
gtaggttgcttaaaaggga

SEQ ID NO: 1162 - RNA, 19 nt, synthetic construct
  source 1..19: mol_type = other RNA
taggttgcttaaaagggat

SEQ ID NO: 1163 - RNA, 19 nt, synthetic construct
  source 1..19: mol_type = other RNA
aggttgcttaaaagggaca

SEQ ID NO: 1164 - RNA, 19 nt, synthetic construct
  source 1..19: mol_type = other RNA
ggttgcttaaaagggacaa

SEQ ID NO: 1165 - RNA, 19 nt, synthetic construct
  source 1..19: mol_type = other RNA
gttgcttaaaagggacagt

SEQ ID NO: 1166 - RNA, 19 nt, synthetic construct
  source 1..19: mol_type = other RNA
ttgcttaaaagggacagta

SEQ ID NO: 1167 - RNA, 19 nt, synthetic construct
  source 1..19: mol_type = other RNA
tgcttaaaagggacagtat

SEQ ID NO: 1168 - RNA, 19 nt, synthetic construct
  source 1..19: mol_type = other RNA
gcttaaaagggacagtatt

SEQ ID NO: 1169 - RNA, 19 nt, synthetic construct
  source 1..19: mol_type = other RNA
cttaaaagggacagtattt

SEQ ID NO: 1170 - RNA, 19 nt, synthetic construct
  source 1..19: mol_type = other RNA
ttaaaagggacagtattct

SEQ ID NO: 1171 - RNA, 19 nt, synthetic construct
  source 1..19: mol_type = other RNA
taaaagggacagtattctt

SEQ ID NO: 1172 - RNA, 19 nt, synthetic construct
  source 1..19: mol_type = other RNA
aaaagggacagtattctca

SEQ ID NO: 1173 - RNA, 19 nt, synthetic construct
  source 1..19: mol_type = other RNA
aaagggacagtattctcaa

SEQ ID NO: 1174 - RNA, 19 nt, synthetic construct
  source 1..19: mol_type = other RNA
aagggacagtattctcagt

SEQ ID NO: 1175 - RNA, 19 nt, synthetic construct
  source 1..19: mol_type = other RNA
agggacagtattctcagta

SEQ ID NO: 1176 - RNA, 19 nt, synthetic construct
  source 1..19: mol_type = other RNA
gggacagtattctcagtgt

SEQ ID NO: 1177 - RNA, 19 nt, synthetic construct
  source 1..19: mol_type = other RNA
ggacagtattctcagtgct

SEQ ID NO: 1178 - RNA, 19 nt, synthetic construct
  source 1..19: mol_type = other RNA
gacagtattctcagtgctt

SEQ ID NO: 1179 - RNA, 19 nt, synthetic construct
  source 1..19: mol_type = other RNA
acagtattctcagtgctct

SEQ ID NO: 1180 - RNA, 19 nt, synthetic construct
  source 1..19: mol_type = other RNA
cagtattctcagtgctctt

SEQ ID NO: 1181 - RNA, 19 nt, synthetic construct
  source 1..19: mol_type = other RNA
agtattctcagtgctctct

SEQ ID NO: 1182 - RNA, 19 nt, synthetic construct
  source 1..19: mol_type = other RNA
gtattctcagtgctctcct

SEQ ID NO: 1183 - RNA, 19 nt, synthetic construct
  source 1..19: mol_type = other RNA
tattctcagtgctctccta

SEQ ID NO: 1184 - RNA, 19 nt, synthetic construct
  source 1..19: mol_type = other RNA
attctcagtgctctcctat

SEQ ID NO: 1185 - RNA, 19 nt, synthetic construct
  source 1..19: mol_type = other RNA
ttctcagtgctctcctact

SEQ ID NO: 1186 - RNA, 19 nt, synthetic construct
  source 1..19: mol_type = other RNA
tctcagtgctctcctacct

SEQ ID NO: 1187 - RNA, 19 nt, synthetic construct
  source 1..19: mol_type = other RNA
ctcagtgctctcctaccct

SEQ ID NO: 1188 - RNA, 19 nt, synthetic construct
  source 1..19: mol_type = other RNA
gctctcctaccccacctca

SEQ ID NO: 1189 - RNA, 19 nt, synthetic construct
  source 1..19: mol_type = other RNA
ctctcctaccccacctcat

SEQ ID NO: 1190 - RNA, 19 nt, synthetic construct
  source 1..19: mol_type = other RNA
tctcctaccccacctcata

SEQ ID NO: 1191 - RNA, 19 nt, synthetic construct
  source 1..19: mol_type = other RNA
ctcctaccccacctcatgt

SEQ ID NO: 1192 - RNA, 19 nt, synthetic construct
  source 1..19: mol_type = other RNA
tcctaccccacctcatgct

SEQ ID NO: 1193 - RNA, 19 nt, synthetic construct
  source 1..19: mol_type = other RNA
cctaccccacctcatgcct

SEQ ID NO: 1194 - RNA, 19 nt, synthetic construct
  source 1..19: mol_type = other RNA
ctaccccacctcatgccta

SEQ ID NO: 1195 - RNA, 19 nt, synthetic construct
  source 1..19: mol_type = other RNA
taccccacctcatgcctga

SEQ ID NO: 1196 - RNA, 19 nt, synthetic construct
  source 1..19: mol_type = other RNA
cccctccaggcatgctggt

SEQ ID NO: 1197 - RNA, 19 nt, synthetic construct
  source 1..19: mol_type = other RNA
ccctccaggcatgctggct

SEQ ID NO: 1198 - RNA, 19 nt, synthetic construct
  source 1..19: mol_type = other RNA
cctccaggcatgctggcct

SEQ ID NO: 1199 - RNA, 19 nt, synthetic construct
  source 1..19: mol_type = other RNA
ctccaggcatgctggcctt

SEQ ID NO: 1200 - RNA, 19 nt, synthetic construct
  source 1..19: mol_type = other RNA
aggcatgctggcctcccaa

SEQ ID NO: 1201 - RNA, 19 nt, synthetic construct
  source 1..19: mol_type = other RNA
ggcatgctggcctcccaat

SEQ ID NO: 1202 - RNA, 19 nt, synthetic construct
  source 1..19: mol_type = other RNA
gcatgctggcctcccaata

SEQ ID NO: 1203 - RNA, 19 nt, synthetic construct
  source 1..19: mol_type = other RNA
catgctggcctcccaataa

SEQ ID NO: 1204 - RNA, 19 nt, synthetic construct
  source 1..19: mol_type = other RNA
atgctggcctcccaataaa

SEQ ID NO: 1205 - RNA, 19 nt, synthetic construct
  source 1..19: mol_type = other RNA
tgctggcctcccaataaaa

SEQ ID NO: 1206 - RNA, 19 nt, synthetic construct
  source 1..19: mol_type = other RNA
gctggcctcccaataaagt

SEQ ID NO: 1207 - RNA, 19 nt, synthetic construct
  source 1..19: mol_type = other RNA
ctggcctcccaataaagct

SEQ ID NO: 1208 - RNA, 19 nt, synthetic construct
  source 1..19: mol_type = other RNA
tggcctcccaataaagcta

SEQ ID NO: 1209 - RNA, 19 nt, synthetic construct
  source 1..19: mol_type = other RNA
ggcctcccaataaagctga

SEQ ID NO: 1210 - RNA, 19 nt, synthetic construct
  source 1..19: mol_type = other RNA
gcctcccaataaagctgga

SEQ ID NO: 1211 - RNA, 19 nt, synthetic construct
  source 1..19: mol_type = other RNA
cctcccaataaagctggat

SEQ ID NO: 1212 - RNA, 19 nt, synthetic construct
  source 1..19: mol_type = other RNA
ctcccaataaagctggaca

SEQ ID NO: 1213 - RNA, 19 nt, synthetic construct
  source 1..19: mol_type = other RNA
tcccaataaagctggacaa

SEQ ID NO: 1214 - RNA, 19 nt, synthetic construct
  source 1..19: mol_type = other RNA
cccaataaagctggacaaa

SEQ ID NO: 1215 - RNA, 19 nt, synthetic construct
  source 1..19: mol_type = other RNA
ccaataaagctggacaaga

SEQ ID NO: 1216 - RNA, 19 nt, synthetic construct
  source 1..19: mol_type = other RNA
caataaagctggacaagaa

SEQ ID NO: 1217 - RNA, 19 nt, synthetic construct
  source 1..19: mol_type = other RNA
aataaagctggacaagaaa

SEQ ID NO: 1218 - RNA, 19 nt, synthetic construct
  source 1..19: mol_type = other RNA
ataaagctggacaagaagt

SEQ ID NO: 1219 - RNA, 19 nt, synthetic construct
  source 1..19: mol_type = other RNA
taaagctggacaagaagct

SEQ ID NO: 1220 - RNA, 19 nt, synthetic construct
  source 1..19: mol_type = other RNA
aaagctggacaagaagcta

SEQ ID NO: 1221 - RNA, 19 nt, synthetic construct
  source 1..19: mol_type = other RNA
aagctggacaagaagctgt

SEQ ID NO: 1222 - RNA, 19 nt, synthetic construct
  source 1..19: mol_type = other RNA
agctggacaagaagctgct

SEQ ID NO: 1223 - RNA, 19 nt, synthetic construct
  source 1..19: mol_type = other RNA
gctggacaagaagctgcta

SEQ ID NO: 1224 - RNA, 19 nt, synthetic construct
  source 1..19: mol_type = other RNA
ctggacaagaagctgctat

SEQ ID NO: 1225 - RNA, 19 nt, synthetic construct
  source 1..19: mol_type = other RNA
tggacaagaagctgctata

SEQ ID NO: 1226 - RNA, 19 nt, synthetic construct
  source 1..19: mol_type = other RNA
ggacaagaagctgctatga

SEQ ID NO: 1227 - RNA, 23 nt, synthetic construct
  source 1..23: mol_type = other RNA
  modified_base 1: mod_base = OTHER; note = n is IB
  modified_base 23: mod_base = OTHER; note = n is IB
  modified_base 21: mod_base = i
nacgggacagtattctcagtnan

SEQ ID NO: 1228 - RNA, 21 nt, synthetic construct
  source 1..21: mol_type = other RNA
aagggacagtattctcagtgc

SEQ ID NO: 1229 - RNA, 19 nt, synthetic construct
  source 1..19: mol_type = other RNA
ttaaaagggacagtattct

SEQ ID NO: 1230 - RNA, 19 nt, synthetic construct
  source 1..19: mol_type = other RNA
aagggacagtattctcagt

SEQ ID NO: 1231 - RNA, 19 nt, synthetic construct
  source 1..19: mol_type = other RNA
ccaagtccacctgcctatt

SEQ ID NO: 1232 - RNA, 19 nt, synthetic construct
  source 1..19: mol_type = other RNA
ccgttaaggacaagttctt

SEQ ID NO: 1233 - RNA, 19 nt, synthetic construct
  source 1..19: mol_type = other RNA
cgaggatgcctcccttctt

SEQ ID NO: 1234 - RNA, 23 nt, synthetic construct
  source 1..23: mol_type = other RNA
  modified_base 1: mod_base = OTHER; note = n is IB
  modified_base 23: mod_base = OTHER; note = n is IB
  modified_base 21: mod_base = i
nacgggacagtattctcagtnan

SEQ ID NO: 1235 - RNA, 23 nt, synthetic construct
  source 1..23: mol_type = other RNA
  modified_base 1: mod_base = OTHER; note = n is STM1
  modified_base 23: mod_base = OTHER; note = n is STM1
naattaaaagggacagtattcan

SEQ ID NO: 1236 - RNA, 23 nt, synthetic construct
  source 1..23: mol_type = other RNA
  modified_base 1: mod_base = OTHER; note = n is IB
  modified_base 23: mod_base = OTHER; note = n is IB
naattaaaagggacagtattcan

SEQ ID NO: 1237 - RNA, 19 nt, synthetic construct
  source 1..19: mol_type = other RNA
ttaaaagggacagtattca

SEQ ID NO: 1238 - RNA, 23 nt, synthetic construct
  source 1..23: mol_type = other RNA
  modified_base 1: mod_base = OTHER; note = n is STM1
  modified_base 23: mod_base = OTHER; note = n is STM1
naaaagggacagtattctcagan

SEQ ID NO: 1239 - RNA, 23 nt, synthetic construct
  source 1..23: mol_type = other RNA
  modified_base 1: mod_base = OTHER; note = n is IB
  modified_base 23: mod_base = OTHER; note = n is IB
naaaagggacagtattctcagan

SEQ ID NO: 1240 - RNA, 19 nt, synthetic construct
  source 1..19: mol_type = other RNA
aagggacagtattctcaga

SEQ ID NO: 1241 - RNA, 21 nt, synthetic construct
  source 1..21: mol_type = other RNA
attcctggagcagctgccttt

SEQ ID NO: 1242 - RNA, 21 nt, synthetic construct
  source 1..21: mol_type = other RNA
tgttcctggagcagctgcctt

SEQ ID NO: 1243 - RNA, 21 nt, synthetic construct
  source 1..21: mol_type = other RNA
ttgttcctggagcagctgctt

SEQ ID NO: 1244 - RNA, 21 nt, synthetic construct
  source 1..21: mol_type = other RNA
tctgttcctggagcagctgtt

SEQ ID NO: 1245 - RNA, 21 nt, synthetic construct
  source 1..21: mol_type = other RNA
ttctgttcctggagcagcttt

SEQ ID NO: 1246 - RNA, 21 nt, synthetic construct
  source 1..21: mol_type = other RNA
tctctgttcctggagcagctt

SEQ ID NO: 1247 - RNA, 21 nt, synthetic construct
  source 1..21: mol_type = other RNA
tacctctgttcctggagcatt

SEQ ID NO: 1248 - RNA, 21 nt, synthetic construct
  source 1..21: mol_type = other RNA
tatggcacctctgttcctgtt

SEQ ID NO: 1249 - RNA, 21 nt, synthetic construct
  source 1..21: mol_type = other RNA
acatggcacctctgttccttt

SEQ ID NO: 1250 - RNA, 21 nt, synthetic construct
  source 1..21: mol_type = other RNA
tgcatggcacctctgttcctt

SEQ ID NO: 1251 - RNA, 21 nt, synthetic construct
  source 1..21: mol_type = other RNA
ttgcatggcacctctgttctt

SEQ ID NO: 1252 - RNA, 21 nt, synthetic construct
  source 1..21: mol_type = other RNA
actgcatggcacctctgtttt

SEQ ID NO: 1253 - RNA, 21 nt, synthetic construct
  source 1..21: mol_type = other RNA
aagtacccggggctgcatgtt

SEQ ID NO: 1254 - RNA, 21 nt, synthetic construct
  source 1..21: mol_type = other RNA
agagtacccggggctgcattt

SEQ ID NO: 1255 - RNA, 21 nt, synthetic construct
  source 1..21: mol_type = other RNA
aggagtacccggggctgcatt

SEQ ID NO: 1256 - RNA, 21 nt, synthetic construct
  source 1..21: mol_type = other RNA
aaggagtacccggggctgctt

SEQ ID NO: 1257 - RNA, 21 nt, synthetic construct
  source 1..21: mol_type = other RNA
taaggagtacccggggctgtt

SEQ ID NO: 1258 - RNA, 21 nt, synthetic construct
  source 1..21: mol_type = other RNA
acaaggagtacccggggcttt

SEQ ID NO: 1259 - RNA, 21 nt, synthetic construct
  source 1..21: mol_type = other RNA
aacaaggagtacccggggctt

SEQ ID NO: 1260 - RNA, 21 nt, synthetic construct
  source 1..21: mol_type = other RNA
taacaaggagtacccggggtt

SEQ ID NO: 1261 - RNA, 21 nt, synthetic construct
  source 1..21: mol_type = other RNA
acaacaaggagtacccgggtt

SEQ ID NO: 1262 - RNA, 21 nt, synthetic construct
  source 1..21: mol_type = other RNA
aacaacaaggagtacccggtt

SEQ ID NO: 1263 - RNA, 21 nt, synthetic construct
  source 1..21: mol_type = other RNA
taacaacaaggagtacccgtt

SEQ ID NO: 1264 - RNA, 21 nt, synthetic construct
  source 1..21: mol_type = other RNA
acaacaacaaggagtaccctt

SEQ ID NO: 1265 - RNA, 21 nt, synthetic construct
  source 1..21: mol_type = other RNA
agcaacaacaaggagtacctt

SEQ ID NO: 1266 - RNA, 21 nt, synthetic construct
  source 1..21: mol_type = other RNA
aggcaacaacaaggagtactt

SEQ ID NO: 1267 - RNA, 21 nt, synthetic construct
  source 1..21: mol_type = other RNA
aagggcaacaacaaggagttt

SEQ ID NO: 1268 - RNA, 21 nt, synthetic construct
  source 1..21: mol_type = other RNA
agagggcaacaacaaggagtt

SEQ ID NO: 1269 - RNA, 21 nt, synthetic construct
  source 1..21: mol_type = other RNA
aggagggcaacaacaaggatt

SEQ ID NO: 1270 - RNA, 21 nt, synthetic construct
  source 1..21: mol_type = other RNA
taggagggcaacaacaaggtt

SEQ ID NO: 1271 - RNA, 21 nt, synthetic construct
  source 1..21: mol_type = other RNA
tcaggagggcaacaacaagtt

SEQ ID NO: 1272 - RNA, 21 nt, synthetic construct
  source 1..21: mol_type = other RNA
accaggagggcaacaacaatt

SEQ ID NO: 1273 - RNA, 21 nt, synthetic construct
  source 1..21: mol_type = other RNA
tgccaggagggcaacaacatt

SEQ ID NO: 1274 - RNA, 21 nt, synthetic construct
  source 1..21: mol_type = other RNA
tcaggagcgccaggagggctt

SEQ ID NO: 1275 - RNA, 21 nt, synthetic construct
  source 1..21: mol_type = other RNA
aaggccaggagcgccaggatt

SEQ ID NO: 1276 - RNA, 21 nt, synthetic construct
  source 1..21: mol_type = other RNA
tagaggccaggagcgccagtt

SEQ ID NO: 1277 - RNA, 21 nt, synthetic construct
  source 1..21: mol_type = other RNA
acagaggccaggagcgccatt

SEQ ID NO: 1278 - RNA, 21 nt, synthetic construct
  source 1..21: mol_type = other RNA
agcagaggccaggagcgcctt

SEQ ID NO: 1279 - RNA, 21 nt, synthetic construct
  source 1..21: mol_type = other RNA
aggcagaggccaggagcgctt

SEQ ID NO: 1280 - RNA, 21 nt, synthetic construct
  source 1..21: mol_type = other RNA
aagctcgggcagaggccagtt

SEQ ID NO: 1281 - RNA, 21 nt, synthetic construct
  source 1..21: mol_type = other RNA
aaagctcgggcagaggccatt

SEQ ID NO: 1282 - RNA, 21 nt, synthetic construct
  source 1..21: mol_type = other RNA
tgaagctcgggcagaggcctt

SEQ ID NO: 1283 - RNA, 21 nt, synthetic construct
  source 1..21: mol_type = other RNA
ttgaagctcgggcagaggctt

SEQ ID NO: 1284 - RNA, 21 nt, synthetic construct
  source 1..21: mol_type = other RNA
tctgaagctcgggcagaggtt

SEQ ID NO: 1285 - RNA, 21 nt, synthetic construct
  source 1..21: mol_type = other RNA
ttctgaagctcgggcagagtt

SEQ ID NO: 1286 - RNA, 21 nt, synthetic construct
  source 1..21: mol_type = other RNA
tctctgaagctcgggcagatt

SEQ ID NO: 1287 - RNA, 21 nt, synthetic construct
  source 1..21: mol_type = other RNA
acctctgaagctcgggcagtt

SEQ ID NO: 1288 - RNA, 21 nt, synthetic construct
  source 1..21: mol_type = other RNA
agcctctgaagctcgggcatt

SEQ ID NO: 1289 - RNA, 21 nt, synthetic construct
  source 1..21: mol_type = other RNA
atcctcggcctctgaagcttt

SEQ ID NO: 1290 - RNA, 21 nt, synthetic construct
  source 1..21: mol_type = other RNA
tatcctcggcctctgaagctt

SEQ ID NO: 1291 - RNA, 21 nt, synthetic construct
  source 1..21: mol_type = other RNA
acatcctcggcctctgaagtt

SEQ ID NO: 1292 - RNA, 21 nt, synthetic construct
  source 1..21: mol_type = other RNA
agcatcctcggcctctgaatt

SEQ ID NO: 1293 - RNA, 21 nt, synthetic construct
  source 1..21: mol_type = other RNA
aggcatcctcggcctctgatt

SEQ ID NO: 1294 - RNA, 21 nt, synthetic construct
  source 1..21: mol_type = other RNA
aaggcatcctcggcctctgtt

SEQ ID NO: 1295 - RNA, 21 nt, synthetic construct
  source 1..21: mol_type = other RNA
agaggcatcctcggcctcttt

SEQ ID NO: 1296 - RNA, 21 nt, synthetic construct
  source 1..21: mol_type = other RNA
aggaggcatcctcggcctctt

SEQ ID NO: 1297 - RNA, 21 nt, synthetic construct
  source 1..21: mol_type = other RNA
aagggaggcatcctcggcctt

SEQ ID NO: 1298 - RNA, 21 nt, synthetic construct
  source 1..21: mol_type = other RNA
aaagggaggcatcctcggctt

SEQ ID NO: 1299 - RNA, 21 nt, synthetic construct
  source 1..21: mol_type = other RNA
agaagggaggcatcctcggtt

SEQ ID NO: 1300 - RNA, 21 nt, synthetic construct
  source 1..21: mol_type = other RNA
aagaagggaggcatcctcgtt

SEQ ID NO: 1301 - RNA, 21 nt, synthetic construct
  source 1..21: mol_type = other RNA
tgagaagggaggcatcctctt

SEQ ID NO: 1302 - RNA, 21 nt, synthetic construct
  source 1..21: mol_type = other RNA
ttgagaagggaggcatccttt

SEQ ID NO: 1303 - RNA, 21 nt, synthetic construct
  source 1..21: mol_type = other RNA
actgagaagggaggcatcctt

SEQ ID NO: 1304 - RNA, 21 nt, synthetic construct
  source 1..21: mol_type = other RNA
agctgagaagggaggcatctt

SEQ ID NO: 1305 - RNA, 21 nt, synthetic construct
  source 1..21: mol_type = other RNA
aagctgagaagggaggcattt

SEQ ID NO: 1306 - RNA, 21 nt, synthetic construct
  source 1..21: mol_type = other RNA
aaagctgagaagggaggcatt

SEQ ID NO: 1307 - RNA, 21 nt, synthetic construct
  source 1..21: mol_type = other RNA
tgaagctgagaagggaggctt

SEQ ID NO: 1308 - RNA, 21 nt, synthetic construct
  source 1..21: mol_type = other RNA
atgaagctgagaagggaggtt

SEQ ID NO: 1309 - RNA, 21 nt, synthetic construct
  source 1..21: mol_type = other RNA
tatgaagctgagaagggagtt

SEQ ID NO: 1310 - RNA, 21 nt, synthetic construct
  source 1..21: mol_type = other RNA
acatgaagctgagaagggatt

SEQ ID NO: 1311 - RNA, 21 nt, synthetic construct
  source 1..21: mol_type = other RNA
tgcatgaagctgagaagggtt

SEQ ID NO: 1312 - RNA, 21 nt, synthetic construct
  source 1..21: mol_type = other RNA
ttgcatgaagctgagaaggtt

SEQ ID NO: 1313 - RNA, 21 nt, synthetic construct
  source 1..21: mol_type = other RNA
tctgcatgaagctgagaagtt

SEQ ID NO: 1314 - RNA, 21 nt, synthetic construct
  source 1..21: mol_type = other RNA
tcctgcatgaagctgagaatt

SEQ ID NO: 1315 - RNA, 21 nt, synthetic construct
  source 1..21: mol_type = other RNA
accctgcatgaagctgagatt

SEQ ID NO: 1316 - RNA, 21 nt, synthetic construct
  source 1..21: mol_type = other RNA
aaccctgcatgaagctgagtt

SEQ ID NO: 1317 - RNA, 21 nt, synthetic construct
  source 1..21: mol_type = other RNA
taaccctgcatgaagctgatt

SEQ ID NO: 1318 - RNA, 21 nt, synthetic construct
  source 1..21: mol_type = other RNA
ataaccctgcatgaagctgtt

SEQ ID NO: 1319 - RNA, 21 nt, synthetic construct
  source 1..21: mol_type = other RNA
tgtaaccctgcatgaagcttt

SEQ ID NO: 1320 - RNA, 21 nt, synthetic construct
  source 1..21: mol_type = other RNA
atgtaaccctgcatgaagctt

SEQ ID NO: 1321 - RNA, 21 nt, synthetic construct
  source 1..21: mol_type = other RNA
tatgtaaccctgcatgaagtt

SEQ ID NO: 1322 - RNA, 21 nt, synthetic construct
  source 1..21: mol_type = other RNA
tcatgtaaccctgcatgaatt

SEQ ID NO: 1323 - RNA, 21 nt, synthetic construct
  source 1..21: mol_type = other RNA
ttcatgtaaccctgcatgatt

SEQ ID NO: 1324 - RNA, 21 nt, synthetic construct
  source 1..21: mol_type = other RNA
tttcatgtaaccctgcatgtt

SEQ ID NO: 1325 - RNA, 21 nt, synthetic construct
  source 1..21: mol_type = other RNA
acttcatgtaaccctgcattt

SEQ ID NO: 1326 - RNA, 21 nt, synthetic construct
  source 1..21: mol_type = other RNA
tgcttcatgtaaccctgcatt

SEQ ID NO: 1327 - RNA, 21 nt, synthetic construct
  source 1..21: mol_type = other RNA
atgcttcatgtaaccctgctt

SEQ ID NO: 1328 - RNA, 21 nt, synthetic construct
  source 1..21: mol_type = other RNA
tgtgcttcatgtaaccctgtt

SEQ ID NO: 1329 - RNA, 21 nt, synthetic construct
  source 1..21: mol_type = other RNA
acgtgcttcatgtaacccttt

SEQ ID NO: 1330 - RNA, 21 nt, synthetic construct
  source 1..21: mol_type = other RNA
agcgtgcttcatgtaaccctt

SEQ ID NO: 1331 - RNA, 21 nt, synthetic construct
  source 1..21: mol_type = other RNA
atggcgtgcttcatgtaactt

SEQ ID NO: 1332 - RNA, 21 nt, synthetic construct
  source 1..21: mol_type = other RNA
ttggtggcgtgcttcatgttt

SEQ ID NO: 1333 - RNA, 21 nt, synthetic construct
  source 1..21: mol_type = other RNA
tttggtggcgtgcttcatgtt

SEQ ID NO: 1334 - RNA, 21 nt, synthetic construct
  source 1..21: mol_type = other RNA
tcttggtggcgtgcttcattt

SEQ ID NO: 1335 - RNA, 21 nt, synthetic construct
  source 1..21: mol_type = other RNA
atcttggtggcgtgcttcatt

SEQ ID NO: 1336 - RNA, 21 nt, synthetic construct
  source 1..21: mol_type = other RNA
agtcttggtggcgtgcttctt

SEQ ID NO: 1337 - RNA, 21 nt, synthetic construct
  source 1..21: mol_type = other RNA
tggtcttggtggcgtgctttt

SEQ ID NO: 1338 - RNA, 21 nt, synthetic construct
  source 1..21: mol_type = other RNA
acggtcttggtggcgtgcttt

SEQ ID NO: 1339 - RNA, 21 nt, synthetic construct
  source 1..21: mol_type = other RNA
agcggtcttggtggcgtgctt

SEQ ID NO: 1340 - RNA, 21 nt, synthetic construct
  source 1..21: mol_type = other RNA
tttggcggtcttggtggcgtt

SEQ ID NO: 1341 - RNA, 21 nt, synthetic construct
  source 1..21: mol_type = other RNA
tcttggcggtcttggtggctt

SEQ ID NO: 1342 - RNA, 21 nt, synthetic construct
  source 1..21: mol_type = other RNA
tccttggcggtcttggtggtt

SEQ ID NO: 1343 - RNA, 21 nt, synthetic construct
  source 1..21: mol_type = other RNA
atccttggcggtcttggtgtt

SEQ ID NO: 1344 - RNA, 21 nt, synthetic construct
  source 1..21: mol_type = other RNA
tatccttggcggtcttggttt

SEQ ID NO: 1345 - RNA, 21 nt, synthetic construct
  source 1..21: mol_type = other RNA
acatccttggcggtcttggtt

SEQ ID NO: 1346 - RNA, 21 nt, synthetic construct
  source 1..21: mol_type = other RNA
tgcatccttggcggtcttgtt

SEQ ID NO: 1347 - RNA, 21 nt, synthetic construct
  source 1..21: mol_type = other RNA
atgcatccttggcggtctttt

SEQ ID NO: 1348 - RNA, 21 nt, synthetic construct
  source 1..21: mol_type = other RNA
agtgcatccttggcggtcttt

SEQ ID NO: 1349 - RNA, 21 nt, synthetic construct
  source 1..21: mol_type = other RNA
tagtgcatccttggcggtctt

SEQ ID NO: 1350 - RNA, 21 nt, synthetic construct
  source 1..21: mol_type = other RNA
tcagtgcatccttggcggttt

SEQ ID NO: 1351 - RNA, 21 nt, synthetic construct
  source 1..21: mol_type = other RNA
ttcagtgcatccttggcggtt

SEQ ID NO: 1352 - RNA, 21 nt, synthetic construct
  source 1..21: mol_type = other RNA
actcagtgcatccttggcgtt

SEQ ID NO: 1353 - RNA, 21 nt, synthetic construct
  source 1..21: mol_type = other RNA
tgctcagtgcatccttggctt

SEQ ID NO: 1354 - RNA, 21 nt, synthetic construct
  source 1..21: mol_type = other RNA
ttgctcagtgcatccttggtt

SEQ ID NO: 1355 - RNA, 21 nt, synthetic construct
  source 1..21: mol_type = other RNA
actgctcagtgcatccttgtt

SEQ ID NO: 1356 - RNA, 21 nt, synthetic construct
  source 1..21: mol_type = other RNA
tgctgctcagtgcatcctttt

SEQ ID NO: 1357 - RNA, 21 nt, synthetic construct
  source 1..21: mol_type = other RNA
acgctgctcagtgcatccttt

SEQ ID NO: 1358 - RNA, 21 nt, synthetic construct
  source 1..21: mol_type = other RNA
tacgctgctcagtgcatcctt

SEQ ID NO: 1359 - RNA, 21 nt, synthetic construct
  source 1..21: mol_type = other RNA
acacgctgctcagtgcatctt

SEQ ID NO: 1360 - RNA, 21 nt, synthetic construct
  source 1..21: mol_type = other RNA
tgcacgctgctcagtgcattt

SEQ ID NO: 1361 - RNA, 21 nt, synthetic construct
  source 1..21: mol_type = other RNA
ttgcacgctgctcagtgcatt

SEQ ID NO: 1362 - RNA, 21 nt, synthetic construct
  source 1..21: mol_type = other RNA
tctgcacgctgctcagtgctt

SEQ ID NO: 1363 - RNA, 21 nt, synthetic construct
  source 1..21: mol_type = other RNA
tcctgcacgctgctcagtgtt

SEQ ID NO: 1364 - RNA, 21 nt, synthetic construct
  source 1..21: mol_type = other RNA
ttcctgcacgctgctcagttt

SEQ ID NO: 1365 - RNA, 21 nt, synthetic construct
  source 1..21: mol_type = other RNA
actcctgcacgctgctcagtt

SEQ ID NO: 1366 - RNA, 21 nt, synthetic construct
  source 1..21: mol_type = other RNA
aactcctgcacgctgctcatt

SEQ ID NO: 1367 - RNA, 21 nt, synthetic construct
  source 1..21: mol_type = other RNA
agactcctgcacgctgctctt

SEQ ID NO: 1368 - RNA, 21 nt, synthetic construct
  source 1..21: mol_type = other RNA
aggactcctgcacgctgcttt

SEQ ID NO: 1369 - RNA, 21 nt, synthetic construct
  source 1..21: mol_type = other RNA
tgggactcctgcacgctgctt

SEQ ID NO: 1370 - RNA, 21 nt, synthetic construct
  source 1..21: mol_type = other RNA
ttgggactcctgcacgctgtt

SEQ ID NO: 1371 - RNA, 21 nt, synthetic construct
  source 1..21: mol_type = other RNA
tctgggactcctgcacgcttt

SEQ ID NO: 1372 - RNA, 21 nt, synthetic construct
  source 1..21: mol_type = other RNA
acctgggactcctgcacgctt

SEQ ID NO: 1373 - RNA, 21 nt, synthetic construct
  source 1..21: mol_type = other RNA
tacctgggactcctgcacgtt

SEQ ID NO: 1374 - RNA, 21 nt, synthetic construct
  source 1..21: mol_type = other RNA
tcacctgggactcctgcactt

SEQ ID NO: 1375 - RNA, 21 nt, synthetic construct
  source 1..21: mol_type = other RNA
accacctgggactcctgcatt

SEQ ID NO: 1376 - RNA, 21 nt, synthetic construct
  source 1..21: mol_type = other RNA
ttgctgggccacctgggactt

SEQ ID NO: 1377 - RNA, 21 nt, synthetic construct
  source 1..21: mol_type = other RNA
tctgctgggccacctgggatt

SEQ ID NO: 1378 - RNA, 21 nt, synthetic construct
  source 1..21: mol_type = other RNA
acctgctgggccacctgggtt

SEQ ID NO: 1379 - RNA, 21 nt, synthetic construct
  source 1..21: mol_type = other RNA
agcctgctgggccacctggtt

SEQ ID NO: 1380 - RNA, 21 nt, synthetic construct
  source 1..21: mol_type = other RNA
tggcctgctgggccacctgtt

SEQ ID NO: 1381 - RNA, 21 nt, synthetic construct
  source 1..21: mol_type = other RNA
ttggcctgctgggccaccttt

SEQ ID NO: 1382 - RNA, 21 nt, synthetic construct
  source 1..21: mol_type = other RNA
tctggcctgctgggccacctt

SEQ ID NO: 1383 - RNA, 21 nt, synthetic construct
  source 1..21: mol_type = other RNA
tcctggcctgctgggccactt

SEQ ID NO: 1384 - RNA, 21 nt, synthetic construct
  source 1..21: mol_type = other RNA
tacccagcccctggcctgctt

SEQ ID NO: 1385 - RNA, 21 nt, synthetic construct
  source 1..21: mol_type = other RNA
tcacccagcccctggcctgtt

SEQ ID NO: 1386 - RNA, 21 nt, synthetic construct
  source 1..21: mol_type = other RNA
atcacccagcccctggccttt

SEQ ID NO: 1387 - RNA, 21 nt, synthetic construct
  source 1..21: mol_type = other RNA
agtcacccagcccctggcctt

SEQ ID NO: 1388 - RNA, 21 nt, synthetic construct
  source 1..21: mol_type = other RNA
tggtcacccagcccctggctt

SEQ ID NO: 1389 - RNA, 21 nt, synthetic construct
  source 1..21: mol_type = other RNA
tcggtcacccagcccctggtt

SEQ ID NO: 1390 - RNA, 21 nt, synthetic construct
  source 1..21: mol_type = other RNA
atcggtcacccagcccctgtt

SEQ ID NO: 1391 - RNA, 21 nt, synthetic construct
  source 1..21: mol_type = other RNA
tatcggtcacccagccccttt

SEQ ID NO: 1392 - RNA, 21 nt, synthetic construct
  source 1..21: mol_type = other RNA
tcatcggtcacccagcccctt

SEQ ID NO: 1393 - RNA, 21 nt, synthetic construct
  source 1..21: mol_type = other RNA
accatcggtcacccagccctt

SEQ ID NO: 1394 - RNA, 21 nt, synthetic construct
  source 1..21: mol_type = other RNA
agccatcggtcacccagcctt

SEQ ID NO: 1395 - RNA, 21 nt, synthetic construct
  source 1..21: mol_type = other RNA
aagccatcggtcacccagctt

SEQ ID NO: 1396 - RNA, 21 nt, synthetic construct
  source 1..21: mol_type = other RNA
aaagccatcggtcacccagtt

SEQ ID NO: 1397 - RNA, 21 nt, synthetic construct
  source 1..21: mol_type = other RNA
tgaagccatcggtcacccatt

SEQ ID NO: 1398 - RNA, 21 nt, synthetic construct
  source 1..21: mol_type = other RNA
ttgaagccatcggtcaccctt

SEQ ID NO: 1399 - RNA, 21 nt, synthetic construct
  source 1..21: mol_type = other RNA
actgaagccatcggtcacctt

SEQ ID NO: 1400 - RNA, 21 nt, synthetic construct
  source 1..21: mol_type = other RNA
aactgaagccatcggtcactt

SEQ ID NO: 1401 - RNA, 21 nt, synthetic construct
  source 1..21: mol_type = other RNA
aaactgaagccatcggtcatt

SEQ ID NO: 1402 - RNA, 21 nt, synthetic construct
  source 1..21: mol_type = other RNA
agaactgaagccatcggtctt

SEQ ID NO: 1403 - RNA, 21 nt, synthetic construct
  source 1..21: mol_type = other RNA
aggaactgaagccatcggttt

SEQ ID NO: 1404 - RNA, 21 nt, synthetic construct
  source 1..21: mol_type = other RNA
agggaactgaagccatcggtt

SEQ ID NO: 1405 - RNA, 21 nt, synthetic construct
  source 1..21: mol_type = other RNA
tagggaactgaagccatcgtt

SEQ ID NO: 1406 - RNA, 21 nt, synthetic construct
  source 1..21: mol_type = other RNA
tcagggaactgaagccatctt

SEQ ID NO: 1407 - RNA, 21 nt, synthetic construct
  source 1..21: mol_type = other RNA
ttcagggaactgaagccattt

SEQ ID NO: 1408 - RNA, 21 nt, synthetic construct
  source 1..21: mol_type = other RNA
tttcagggaactgaagccatt

SEQ ID NO: 1409 - RNA, 21 nt, synthetic construct
  source 1..21: mol_type = other RNA
ttttcagggaactgaagcctt

SEQ ID NO: 1410 - RNA, 21 nt, synthetic construct
  source 1..21: mol_type = other RNA
tctttcagggaactgaagctt

SEQ ID NO: 1411 - RNA, 21 nt, synthetic construct
  source 1..21: mol_type = other RNA
atctttcagggaactgaagtt

SEQ ID NO: 1412 - RNA, 21 nt, synthetic construct
  source 1..21: mol_type = other RNA
agtctttcagggaactgaatt

SEQ ID NO: 1413 - RNA, 21 nt, synthetic construct
  source 1..21: mol_type = other RNA
tagtctttcagggaactgatt

SEQ ID NO: 1414 - RNA, 21 nt, synthetic construct
  source 1..21: mol_type = other RNA
atagtctttcagggaactgtt

SEQ ID NO: 1415 - RNA, 21 nt, synthetic construct
  source 1..21: mol_type = other RNA
agtagtctttcagggaacttt

SEQ ID NO: 1416 - RNA, 21 nt, synthetic construct
  source 1..21: mol_type = other RNA
tagtagtctttcagggaactt

SEQ ID NO: 1417 - RNA, 21 nt, synthetic construct
  source 1..21: mol_type = other RNA
tcagtagtctttcagggaatt

SEQ ID NO: 1418 - RNA, 21 nt, synthetic construct
  source 1..21: mol_type = other RNA
tccagtagtctttcagggatt

SEQ ID NO: 1419 - RNA, 21 nt, synthetic construct
  source 1..21: mol_type = other RNA
ttccagtagtctttcagggtt

SEQ ID NO: 1420 - RNA, 21 nt, synthetic construct
  source 1..21: mol_type = other RNA
actccagtagtctttcaggtt

SEQ ID NO: 1421 - RNA, 21 nt, synthetic construct
  source 1..21: mol_type = other RNA
tgctccagtagtctttcagtt

SEQ ID NO: 1422 - RNA, 21 nt, synthetic construct
  source 1..21: mol_type = other RNA
atgctccagtagtctttcatt

SEQ ID NO: 1423 - RNA, 21 nt, synthetic construct
  source 1..21: mol_type = other RNA
agtgctccagtagtctttctt

SEQ ID NO: 1424 - RNA, 21 nt, synthetic construct
  source 1..21: mol_type = other RNA
tggtgctccagtagtcttttt

SEQ ID NO: 1425 - RNA, 21 nt, synthetic construct
  source 1..21: mol_type = other RNA
aacggtgctccagtagtcttt

SEQ ID NO: 1426 - RNA, 21 nt, synthetic construct
  source 1..21: mol_type = other RNA
taacggtgctccagtagtctt

SEQ ID NO: 1427 - RNA, 21 nt, synthetic construct
  source 1..21: mol_type = other RNA
ttaacggtgctccagtagttt

SEQ ID NO: 1428 - RNA, 21 nt, synthetic construct
  source 1..21: mol_type = other RNA
tttaacggtgctccagtagtt

SEQ ID NO: 1429 - RNA, 21 nt, synthetic construct
  source 1..21: mol_type = other RNA
tcttaacggtgctccagtatt

SEQ ID NO: 1430 - RNA, 21 nt, synthetic construct
  source 1..21: mol_type = other RNA
tccttaacggtgctccagttt

SEQ ID NO: 1431 - RNA, 21 nt, synthetic construct
  source 1..21: mol_type = other RNA
atccttaacggtgctccagtt

SEQ ID NO: 1432 - RNA, 21 nt, synthetic construct
  source 1..21: mol_type = other RNA
tgtccttaacggtgctccatt

SEQ ID NO: 1433 - RNA, 21 nt, synthetic construct
  source 1..21: mol_type = other RNA
ttgtccttaacggtgctcctt

SEQ ID NO: 1434 - RNA, 21 nt, synthetic construct
  source 1..21: mol_type = other RNA
tttgtccttaacggtgctctt

SEQ ID NO: 1435 - RNA, 21 nt, synthetic construct
  source 1..21: mol_type = other RNA
acttgtccttaacggtgcttt

SEQ ID NO: 1436 - RNA, 21 nt, synthetic construct
  source 1..21: mol_type = other RNA
aacttgtccttaacggtgctt

SEQ ID NO: 1437 - RNA, 21 nt, synthetic construct
  source 1..21: mol_type = other RNA
aaacttgtccttaacggtgtt

SEQ ID NO: 1438 - RNA, 21 nt, synthetic construct
  source 1..21: mol_type = other RNA
agaacttgtccttaacggttt

SEQ ID NO: 1439 - RNA, 21 nt, synthetic construct
  source 1..21: mol_type = other RNA
aagaacttgtccttaacggtt

SEQ ID NO: 1440 - RNA, 21 nt, synthetic construct
  source 1..21: mol_type = other RNA
agagaacttgtccttaacgtt

SEQ ID NO: 1441 - RNA, 21 nt, synthetic construct
  source 1..21: mol_type = other RNA
tagagaacttgtccttaactt

SEQ ID NO: 1442 - RNA, 21 nt, synthetic construct
  source 1..21: mol_type = other RNA
tcagagaacttgtccttaatt

SEQ ID NO: 1443 - RNA, 21 nt, synthetic construct
  source 1..21: mol_type = other RNA
ttcagagaacttgtccttatt

SEQ ID NO: 1444 - RNA, 21 nt, synthetic construct
  source 1..21: mol_type = other RNA
actcagagaacttgtcctttt

SEQ ID NO: 1445 - RNA, 21 nt, synthetic construct
  source 1..21: mol_type = other RNA
aactcagagaacttgtccttt

SEQ ID NO: 1446 - RNA, 21 nt, synthetic construct
  source 1..21: mol_type = other RNA
aaactcagagaacttgtcctt

SEQ ID NO: 1447 - RNA, 21 nt, synthetic construct
  source 1..21: mol_type = other RNA
agaactcagagaacttgtctt

SEQ ID NO: 1448 - RNA, 21 nt, synthetic construct
  source 1..21: mol_type = other RNA
tagaactcagagaacttgttt

SEQ ID NO: 1449 - RNA, 21 nt, synthetic construct
  source 1..21: mol_type = other RNA
tcagaactcagagaacttgtt

SEQ ID NO: 1450 - RNA, 21 nt, synthetic construct
  source 1..21: mol_type = other RNA
tccagaactcagagaactttt

SEQ ID NO: 1451 - RNA, 21 nt, synthetic construct
  source 1..21: mol_type = other RNA
tcccagaactcagagaacttt

SEQ ID NO: 1452 - RNA, 21 nt, synthetic construct
  source 1..21: mol_type = other RNA
atcccagaactcagagaactt

SEQ ID NO: 1453 - RNA, 21 nt, synthetic construct
  source 1..21: mol_type = other RNA
aatcccagaactcagagaatt

SEQ ID NO: 1454 - RNA, 21 nt, synthetic construct
  source 1..21: mol_type = other RNA
aaatcccagaactcagagatt

SEQ ID NO: 1455 - RNA, 21 nt, synthetic construct
  source 1..21: mol_type = other RNA
taaatcccagaactcagagtt

SEQ ID NO: 1456 - RNA, 21 nt, synthetic construct
  source 1..21: mol_type = other RNA
tcaaatcccagaactcagatt

SEQ ID NO: 1457 - RNA, 21 nt, synthetic construct
  source 1..21: mol_type = other RNA
tccaaatcccagaactcagtt

SEQ ID NO: 1458 - RNA, 21 nt, synthetic construct
  source 1..21: mol_type = other RNA
atccaaatcccagaactcatt

SEQ ID NO: 1459 - RNA, 21 nt, synthetic construct
  source 1..21: mol_type = other RNA
agtccaaatcccagaactctt

SEQ ID NO: 1460 - RNA, 21 nt, synthetic construct
  source 1..21: mol_type = other RNA
aggtccaaatcccagaacttt

SEQ ID NO: 1461 - RNA, 21 nt, synthetic construct
  source 1..21: mol_type = other RNA
tagggtccaaatcccagaatt

SEQ ID NO: 1462 - RNA, 21 nt, synthetic construct
  source 1..21: mol_type = other RNA
tcagggtccaaatcccagatt

SEQ ID NO: 1463 - RNA, 21 nt, synthetic construct
  source 1..21: mol_type = other RNA
ttcagggtccaaatcccagtt

SEQ ID NO: 1464 - RNA, 21 nt, synthetic construct
  source 1..21: mol_type = other RNA
tctcagggtccaaatcccatt

SEQ ID NO: 1465 - RNA, 21 nt, synthetic construct
  source 1..21: mol_type = other RNA
acctcagggtccaaatccctt

SEQ ID NO: 1466 - RNA, 21 nt, synthetic construct
  source 1..21: mol_type = other RNA
aacctcagggtccaaatcctt

SEQ ID NO: 1467 - RNA, 21 nt, synthetic construct
  source 1..21: mol_type = other RNA
tgacctcagggtccaaatctt

SEQ ID NO: 1468 - RNA, 21 nt, synthetic construct
  source 1..21: mol_type = other RNA
ttgacctcagggtccaaattt

SEQ ID NO: 1469 - RNA, 21 nt, synthetic construct
  source 1..21: mol_type = other RNA
tctgacctcagggtccaaatt

SEQ ID NO: 1470 - RNA, 21 nt, synthetic construct
  source 1..21: mol_type = other RNA
atctgacctcagggtccaatt

SEQ ID NO: 1471 - RNA, 21 nt, synthetic construct
  source 1..21: mol_type = other RNA
agtctgacctcagggtccatt

SEQ ID NO: 1472 - RNA, 21 nt, synthetic construct
  source 1..21: mol_type = other RNA
tggtctgacctcagggtcctt

SEQ ID NO: 1473 - RNA, 21 nt, synthetic construct
  source 1..21: mol_type = other RNA
ttggtctgacctcagggtctt

SEQ ID NO: 1474 - RNA, 21 nt, synthetic construct
  source 1..21: mol_type = other RNA
attggtctgacctcagggttt

SEQ ID NO: 1475 - RNA, 21 nt, synthetic construct
  source 1..21: mol_type = other RNA
agttggtctgacctcagggtt

SEQ ID NO: 1476 - RNA, 21 nt, synthetic construct
  source 1..21: mol_type = other RNA
aagttggtctgacctcaggtt

SEQ ID NO: 1477 - RNA, 21 nt, synthetic construct
  source 1..21: mol_type = other RNA
aaagttggtctgacctcagtt

SEQ ID NO: 1478 - RNA, 21 nt, synthetic construct
  source 1..21: mol_type = other RNA
tgaagttggtctgacctcatt

SEQ ID NO: 1479 - RNA, 21 nt, synthetic construct
  source 1..21: mol_type = other RNA
ttgaagttggtctgacctctt

SEQ ID NO: 1480 - RNA, 21 nt, synthetic construct
  source 1..21: mol_type = other RNA
actgaagttggtctgaccttt

SEQ ID NO: 1481 - RNA, 21 nt, synthetic construct
  source 1..21: mol_type = other RNA
agctgaagttggtctgacctt

SEQ ID NO: 1482 - RNA, 21 nt, synthetic construct
  source 1..21: mol_type = other RNA
tggctgaagttggtctgactt

SEQ ID NO: 1483 - RNA, 21 nt, synthetic construct
  source 1..21: mol_type = other RNA
tagccacggctgaagttggtt

SEQ ID NO: 1484 - RNA, 21 nt, synthetic construct
  source 1..21: mol_type = other RNA
acagccacggctgaagttgtt

SEQ ID NO: 1485 - RNA, 21 nt, synthetic construct
  source 1..21: mol_type = other RNA
agcagccacggctgaagtttt

SEQ ID NO: 1486 - RNA, 21 nt, synthetic construct
  source 1..21: mol_type = other RNA
aggcagccacggctgaagttt

SEQ ID NO: 1487 - RNA, 21 nt, synthetic construct
  source 1..21: mol_type = other RNA
taggcagccacggctgaagtt

SEQ ID NO: 1488 - RNA, 21 nt, synthetic construct
  source 1..21: mol_type = other RNA
tcaggcagccacggctgaatt

SEQ ID NO: 1489 - RNA, 21 nt, synthetic construct
  source 1..21: mol_type = other RNA
ttcaggcagccacggctgatt

SEQ ID NO: 1490 - RNA, 21 nt, synthetic construct
  source 1..21: mol_type = other RNA
tctcaggcagccacggctgtt

SEQ ID NO: 1491 - RNA, 21 nt, synthetic construct
  source 1..21: mol_type = other RNA
atctcaggcagccacggcttt

SEQ ID NO: 1492 - RNA, 21 nt, synthetic construct
  source 1..21: mol_type = other RNA
agtctcaggcagccacggctt

SEQ ID NO: 1493 - RNA, 21 nt, synthetic construct
  source 1..21: mol_type = other RNA
aggtctcaggcagccacggtt

SEQ ID NO: 1494 - RNA, 21 nt, synthetic construct
  source 1..21: mol_type = other RNA
aaggtctcaggcagccacgtt

SEQ ID NO: 1495 - RNA, 21 nt, synthetic construct
  source 1..21: mol_type = other RNA
tgaggtctcaggcagccactt

SEQ ID NO: 1496 - RNA, 21 nt, synthetic construct
  source 1..21: mol_type = other RNA
ttgaggtctcaggcagccatt

SEQ ID NO: 1497 - RNA, 21 nt, synthetic construct
  source 1..21: mol_type = other RNA
attgaggtctcaggcagcctt

SEQ ID NO: 1498 - RNA, 21 nt, synthetic construct
  source 1..21: mol_type = other RNA
tattgaggtctcaggcagctt

SEQ ID NO: 1499 - RNA, 21 nt, synthetic construct
  source 1..21: mol_type = other RNA
atattgaggtctcaggcagtt

SEQ ID NO: 1500 - RNA, 21 nt, synthetic construct
  source 1..21: mol_type = other RNA
agtattgaggtctcaggcatt

SEQ ID NO: 1501 - RNA, 21 nt, synthetic construct
  source 1..21: mol_type = other RNA
aggtattgaggtctcaggctt

SEQ ID NO: 1502 - RNA, 21 nt, synthetic construct
  source 1..21: mol_type = other RNA
agggtattgaggtctcaggtt

SEQ ID NO: 1503 - RNA, 21 nt, synthetic construct
  source 1..21: mol_type = other RNA
ttggggtattgaggtctcatt

SEQ ID NO: 1504 - RNA, 21 nt, synthetic construct
  source 1..21: mol_type = other RNA
tttggggtattgaggtctctt

SEQ ID NO: 1505 - RNA, 21 nt, synthetic construct
  source 1..21: mol_type = other RNA
acttggggtattgaggtcttt

SEQ ID NO: 1506 - RNA, 21 nt, synthetic construct
  source 1..21: mol_type = other RNA
aacttggggtattgaggtctt

SEQ ID NO: 1507 - RNA, 21 nt, synthetic construct
  source 1..21: mol_type = other RNA
agacttggggtattgaggttt

SEQ ID NO: 1508 - RNA, 21 nt, synthetic construct
  source 1..21: mol_type = other RNA
tggacttggggtattgaggtt

SEQ ID NO: 1509 - RNA, 21 nt, synthetic construct
  source 1..21: mol_type = other RNA
atggacttggggtattgagtt

SEQ ID NO: 1510 - RNA, 21 nt, synthetic construct
  source 1..21: mol_type = other RNA
agtggacttggggtattgatt

SEQ ID NO: 1511 - RNA, 21 nt, synthetic construct
  source 1..21: mol_type = other RNA
aggtggacttggggtattgtt

SEQ ID NO: 1512 - RNA, 21 nt, synthetic construct
  source 1..21: mol_type = other RNA
taggtggacttggggtatttt

SEQ ID NO: 1513 - RNA, 21 nt, synthetic construct
  source 1..21: mol_type = other RNA
acaggtggacttggggtattt

SEQ ID NO: 1514 - RNA, 21 nt, synthetic construct
  source 1..21: mol_type = other RNA
agcaggtggacttggggtatt

SEQ ID NO: 1515 - RNA, 21 nt, synthetic construct
  source 1..21: mol_type = other RNA
taggcaggtggacttggggtt

SEQ ID NO: 1516 - RNA, 21 nt, synthetic construct
  source 1..21: mol_type = other RNA
ataggcaggtggacttgggtt

SEQ ID NO: 1517 - RNA, 21 nt, synthetic construct
  source 1..21: mol_type = other RNA
aataggcaggtggacttggtt

SEQ ID NO: 1518 - RNA, 21 nt, synthetic construct
  source 1..21: mol_type = other RNA
agataggcaggtggacttgtt

SEQ ID NO: 1519 - RNA, 21 nt, synthetic construct
  source 1..21: mol_type = other RNA
tggataggcaggtggactttt

SEQ ID NO: 1520 - RNA, 21 nt, synthetic construct
  source 1..21: mol_type = other RNA
atggataggcaggtggacttt

SEQ ID NO: 1521 - RNA, 21 nt, synthetic construct
  source 1..21: mol_type = other RNA
aatggataggcaggtggactt

SEQ ID NO: 1522 - RNA, 21 nt, synthetic construct
  source 1..21: mol_type = other RNA
agatggataggcaggtggatt

SEQ ID NO: 1523 - RNA, 21 nt, synthetic construct
  source 1..21: mol_type = other RNA
aggatggataggcaggtggtt

SEQ ID NO: 1524 - RNA, 21 nt, synthetic construct
  source 1..21: mol_type = other RNA
taggatggataggcaggtgtt

SEQ ID NO: 1525 - RNA, 21 nt, synthetic construct
  source 1..21: mol_type = other RNA
acaggatggataggcaggttt

SEQ ID NO: 1526 - RNA, 21 nt, synthetic construct
  source 1..21: mol_type = other RNA
tgcaggatggataggcaggtt

SEQ ID NO: 1527 - RNA, 21 nt, synthetic construct
  source 1..21: mol_type = other RNA
tcgcaggatggataggcagtt

SEQ ID NO: 1528 - RNA, 21 nt, synthetic construct
  source 1..21: mol_type = other RNA
ttcgcaggatggataggcatt

SEQ ID NO: 1529 - RNA, 21 nt, synthetic construct
  source 1..21: mol_type = other RNA
actcgcaggatggataggctt

SEQ ID NO: 1530 - RNA, 21 nt, synthetic construct
  source 1..21: mol_type = other RNA
agctcgcaggatggataggtt

SEQ ID NO: 1531 - RNA, 21 nt, synthetic construct
  source 1..21: mol_type = other RNA
aagctcgcaggatggatagtt

SEQ ID NO: 1532 - RNA, 21 nt, synthetic construct
  source 1..21: mol_type = other RNA
agagctcgcaggatggatatt

SEQ ID NO: 1533 - RNA, 21 nt, synthetic construct
  source 1..21: mol_type = other RNA
aggagctcgcaggatggattt

SEQ ID NO: 1534 - RNA, 21 nt, synthetic construct
  source 1..21: mol_type = other RNA
aaggagctcgcaggatggatt

SEQ ID NO: 1535 - RNA, 21 nt, synthetic construct
  source 1..21: mol_type = other RNA
taaggagctcgcaggatggtt

SEQ ID NO: 1536 - RNA, 21 nt, synthetic construct
  source 1..21: mol_type = other RNA
tcaaggagctcgcaggatgtt

SEQ ID NO: 1537 - RNA, 21 nt, synthetic construct
  source 1..21: mol_type = other RNA
tccaaggagctcgcaggattt

SEQ ID NO: 1538 - RNA, 21 nt, synthetic construct
  source 1..21: mol_type = other RNA
acccaaggagctcgcaggatt

SEQ ID NO: 1539 - RNA, 21 nt, synthetic construct
  source 1..21: mol_type = other RNA
aacccaaggagctcgcaggtt

SEQ ID NO: 1540 - RNA, 21 nt, synthetic construct
  source 1..21: mol_type = other RNA
agacccaaggagctcgcagtt

SEQ ID NO: 1541 - RNA, 21 nt, synthetic construct
  source 1..21: mol_type = other RNA
aggacccaaggagctcgcatt

SEQ ID NO: 1542 - RNA, 21 nt, synthetic construct
  source 1..21: mol_type = other RNA
taggacccaaggagctcgctt

SEQ ID NO: 1543 - RNA, 21 nt, synthetic construct
  source 1..21: mol_type = other RNA
acaggacccaaggagctcgtt

SEQ ID NO: 1544 - RNA, 21 nt, synthetic construct
  source 1..21: mol_type = other RNA
tgcaggacccaaggagctctt

SEQ ID NO: 1545 - RNA, 21 nt, synthetic construct
  source 1..21: mol_type = other RNA
ttgcaggacccaaggagcttt

SEQ ID NO: 1546 - RNA, 21 nt, synthetic construct
  source 1..21: mol_type = other RNA
attgcaggacccaaggagctt

SEQ ID NO: 1547 - RNA, 21 nt, synthetic construct
  source 1..21: mol_type = other RNA
aattgcaggacccaaggagtt

SEQ ID NO: 1548 - RNA, 21 nt, synthetic construct
  source 1..21: mol_type = other RNA
agattgcaggacccaaggatt

SEQ ID NO: 1549 - RNA, 21 nt, synthetic construct
  source 1..21: mol_type = other RNA
aagattgcaggacccaaggtt

SEQ ID NO: 1550 - RNA, 21 nt, synthetic construct
  source 1..21: mol_type = other RNA
agagattgcaggacccaagtt

SEQ ID NO: 1551 - RNA, 21 nt, synthetic construct
  source 1..21: mol_type = other RNA
tggagattgcaggacccaatt

SEQ ID NO: 1552 - RNA, 21 nt, synthetic construct
  source 1..21: mol_type = other RNA
ttggagattgcaggacccatt

SEQ ID NO: 1553 - RNA, 21 nt, synthetic construct
  source 1..21: mol_type = other RNA
tctggagattgcaggaccctt

SEQ ID NO: 1554 - RNA, 21 nt, synthetic construct
  source 1..21: mol_type = other RNA
tcctggagattgcaggacctt

SEQ ID NO: 1555 - RNA, 21 nt, synthetic construct
  source 1..21: mol_type = other RNA
accctggagattgcaggactt

SEQ ID NO: 1556 - RNA, 21 nt, synthetic construct
  source 1..21: mol_type = other RNA
tagccctggagattgcaggtt

SEQ ID NO: 1557 - RNA, 21 nt, synthetic construct
  source 1..21: mol_type = other RNA
acagccctggagattgcagtt

SEQ ID NO: 1558 - RNA, 21 nt, synthetic construct
  source 1..21: mol_type = other RNA
agcagccctggagattgcatt

SEQ ID NO: 1559 - RNA, 21 nt, synthetic construct
  source 1..21: mol_type = other RNA
tacaggggcagccctggagtt

SEQ ID NO: 1560 - RNA, 21 nt, synthetic construct
  source 1..21: mol_type = other RNA
ttacaggggcagccctggatt

SEQ ID NO: 1561 - RNA, 21 nt, synthetic construct
  source 1..21: mol_type = other RNA
tctacaggggcagccctggtt

SEQ ID NO: 1562 - RNA, 21 nt, synthetic construct
  source 1..21: mol_type = other RNA
acctacaggggcagccctgtt

SEQ ID NO: 1563 - RNA, 21 nt, synthetic construct
  source 1..21: mol_type = other RNA
aacctacaggggcagcccttt

SEQ ID NO: 1564 - RNA, 21 nt, synthetic construct
  source 1..21: mol_type = other RNA
taacctacaggggcagccctt

SEQ ID NO: 1565 - RNA, 21 nt, synthetic construct
  source 1..21: mol_type = other RNA
acaacctacaggggcagcctt

SEQ ID NO: 1566 - RNA, 21 nt, synthetic construct
  source 1..21: mol_type = other RNA
agcaacctacaggggcagctt

SEQ ID NO: 1567 - RNA, 21 nt, synthetic construct
  source 1..21: mol_type = other RNA
aagcaacctacaggggcagtt

SEQ ID NO: 1568 - RNA, 21 nt, synthetic construct
  source 1..21: mol_type = other RNA
taagcaacctacaggggcatt

SEQ ID NO: 1569 - RNA, 21 nt, synthetic construct
  source 1..21: mol_type = other RNA
ttaagcaacctacaggggctt

SEQ ID NO: 1570 - RNA, 21 nt, synthetic construct
  source 1..21: mol_type = other RNA
tttaagcaacctacaggggtt

SEQ ID NO: 1571 - RNA, 21 nt, synthetic construct
  source 1..21: mol_type = other RNA
ttttaagcaacctacagggtt

SEQ ID NO: 1572 - RNA, 21 nt, synthetic construct
  source 1..21: mol_type = other RNA
tttttaagcaacctacaggtt

SEQ ID NO: 1573 - RNA, 21 nt, synthetic construct
  source 1..21: mol_type = other RNA
tcttttaagcaacctacagtt

SEQ ID NO: 1574 - RNA, 21 nt, synthetic construct
  source 1..21: mol_type = other RNA
tccttttaagcaacctacatt

SEQ ID NO: 1575 - RNA, 21 nt, synthetic construct
  source 1..21: mol_type = other RNA
tcccttttaagcaacctactt

SEQ ID NO: 1576 - RNA, 21 nt, synthetic construct
  source 1..21: mol_type = other RNA
atcccttttaagcaacctatt

SEQ ID NO: 1577 - RNA, 21 nt, synthetic construct
  source 1..21: mol_type = other RNA
tgtcccttttaagcaaccttt

SEQ ID NO: 1578 - RNA, 21 nt, synthetic construct
  source 1..21: mol_type = other RNA
ttgtcccttttaagcaacctt

SEQ ID NO: 1579 - RNA, 21 nt, synthetic construct
  source 1..21: mol_type = other RNA
actgtcccttttaagcaactt

SEQ ID NO: 1580 - RNA, 21 nt, synthetic construct
  source 1..21: mol_type = other RNA
tactgtcccttttaagcaatt

SEQ ID NO: 1581 - RNA, 21 nt, synthetic construct
  source 1..21: mol_type = other RNA
atactgtcccttttaagcatt

SEQ ID NO: 1582 - RNA, 21 nt, synthetic construct
  source 1..21: mol_type = other RNA
aatactgtcccttttaagctt

SEQ ID NO: 1583 - RNA, 21 nt, synthetic construct
  source 1..21: mol_type = other RNA
aaatactgtcccttttaagtt

SEQ ID NO: 1584 - RNA, 21 nt, synthetic construct
  source 1..21: mol_type = other RNA
agaatactgtcccttttaatt

SEQ ID NO: 1585 - RNA, 21 nt, synthetic construct
  source 1..21: mol_type = other RNA
aagaatactgtcccttttatt

SEQ ID NO: 1586 - RNA, 21 nt, synthetic construct
  source 1..21: mol_type = other RNA
tgagaatactgtccctttttt

SEQ ID NO: 1587 - RNA, 21 nt, synthetic construct
  source 1..21: mol_type = other RNA
ttgagaatactgtcccttttt

SEQ ID NO: 1588 - RNA, 21 nt, synthetic construct
  source 1..21: mol_type = other RNA
actgagaatactgtccctttt

SEQ ID NO: 1589 - RNA, 21 nt, synthetic construct
  source 1..21: mol_type = other RNA
tactgagaatactgtcccttt

SEQ ID NO: 1590 - RNA, 21 nt, synthetic construct
  source 1..21: mol_type = other RNA
acactgagaatactgtccctt

SEQ ID NO: 1591 - RNA, 21 nt, synthetic construct
  source 1..21: mol_type = other RNA
agcactgagaatactgtcctt

SEQ ID NO: 1592 - RNA, 21 nt, synthetic construct
  source 1..21: mol_type = other RNA
aagcactgagaatactgtctt

SEQ ID NO: 1593 - RNA, 21 nt, synthetic construct
  source 1..21: mol_type = other RNA
agagcactgagaatactgttt

SEQ ID NO: 1594 - RNA, 21 nt, synthetic construct
  source 1..21: mol_type = other RNA
aagagcactgagaatactgtt

SEQ ID NO: 1595 - RNA, 21 nt, synthetic construct
  source 1..21: mol_type = other RNA
agagagcactgagaatacttt

SEQ ID NO: 1596 - RNA, 21 nt, synthetic construct
  source 1..21: mol_type = other RNA
aggagagcactgagaatactt

SEQ ID NO: 1597 - RNA, 21 nt, synthetic construct
  source 1..21: mol_type = other RNA
taggagagcactgagaatatt

SEQ ID NO: 1598 - RNA, 21 nt, synthetic construct
  source 1..21: mol_type = other RNA
ataggagagcactgagaattt

SEQ ID NO: 1599 - RNA, 21 nt, synthetic construct
  source 1..21: mol_type = other RNA
agtaggagagcactgagaatt

SEQ ID NO: 1600 - RNA, 21 nt, synthetic construct
  source 1..21: mol_type = other RNA
aggtaggagagcactgagatt

SEQ ID NO: 1601 - RNA, 21 nt, synthetic construct
  source 1..21: mol_type = other RNA
agggtaggagagcactgagtt

SEQ ID NO: 1602 - RNA, 21 nt, synthetic construct
  source 1..21: mol_type = other RNA
tgaggtggggtaggagagctt

SEQ ID NO: 1603 - RNA, 21 nt, synthetic construct
  source 1..21: mol_type = other RNA
atgaggtggggtaggagagtt

SEQ ID NO: 1604 - RNA, 21 nt, synthetic construct
  source 1..21: mol_type = other RNA
tatgaggtggggtaggagatt

SEQ ID NO: 1605 - RNA, 21 nt, synthetic construct
  source 1..21: mol_type = other RNA
acatgaggtggggtaggagtt

SEQ ID NO: 1606 - RNA, 21 nt, synthetic construct
  source 1..21: mol_type = other RNA
agcatgaggtggggtaggatt

SEQ ID NO: 1607 - RNA, 21 nt, synthetic construct
  source 1..21: mol_type = other RNA
aggcatgaggtggggtaggtt

SEQ ID NO: 1608 - RNA, 21 nt, synthetic construct
  source 1..21: mol_type = other RNA
taggcatgaggtggggtagtt

SEQ ID NO: 1609 - RNA, 21 nt, synthetic construct
  source 1..21: mol_type = other RNA
tcaggcatgaggtggggtatt

SEQ ID NO: 1610 - RNA, 21 nt, synthetic construct
  source 1..21: mol_type = other RNA
accagcatgcctggaggggtt

SEQ ID NO: 1611 - RNA, 21 nt, synthetic construct
  source 1..21: mol_type = other RNA
agccagcatgcctggagggtt

SEQ ID NO: 1612 - RNA, 21 nt, synthetic construct
  source 1..21: mol_type = other RNA
aggccagcatgcctggaggtt

SEQ ID NO: 1613 - RNA, 21 nt, synthetic construct
  source 1..21: mol_type = other RNA
aaggccagcatgcctggagtt

SEQ ID NO: 1614 - RNA, 21 nt, synthetic construct
  source 1..21: mol_type = other RNA
ttgggaggccagcatgccttt

SEQ ID NO: 1615 - RNA, 21 nt, synthetic construct
  source 1..21: mol_type = other RNA
attgggaggccagcatgcctt

SEQ ID NO: 1616 - RNA, 21 nt, synthetic construct
  source 1..21: mol_type = other RNA
tattgggaggccagcatgctt

SEQ ID NO: 1617 - RNA, 21 nt, synthetic construct
  source 1..21: mol_type = other RNA
ttattgggaggccagcatgtt

SEQ ID NO: 1618 - RNA, 21 nt, synthetic construct
  source 1..21: mol_type = other RNA
tttattgggaggccagcattt

SEQ ID NO: 1619 - RNA, 21 nt, synthetic construct
  source 1..21: mol_type = other RNA
ttttattgggaggccagcatt

SEQ ID NO: 1620 - RNA, 21 nt, synthetic construct
  source 1..21: mol_type = other RNA
actttattgggaggccagctt

SEQ ID NO: 1621 - RNA, 21 nt, synthetic construct
  source 1..21: mol_type = other RNA
agctttattgggaggccagtt

SEQ ID NO: 1622 - RNA, 21 nt, synthetic construct
  source 1..21: mol_type = other RNA
tagctttattgggaggccatt

SEQ ID NO: 1623 - RNA, 21 nt, synthetic construct
  source 1..21: mol_type = other RNA
tcagctttattgggaggcctt

SEQ ID NO: 1624 - RNA, 21 nt, synthetic construct
  source 1..21: mol_type = other RNA
tccagctttattgggaggctt

SEQ ID NO: 1625 - RNA, 21 nt, synthetic construct
  source 1..21: mol_type = other RNA
atccagctttattgggaggtt

SEQ ID NO: 1626 - RNA, 21 nt, synthetic construct
  source 1..21: mol_type = other RNA
tgtccagctttattgggagtt

SEQ ID NO: 1627 - RNA, 21 nt, synthetic construct
  source 1..21: mol_type = other RNA
ttgtccagctttattgggatt

SEQ ID NO: 1628 - RNA, 21 nt, synthetic construct
  source 1..21: mol_type = other RNA
tttgtccagctttattgggtt

SEQ ID NO: 1629 - RNA, 21 nt, synthetic construct
  source 1..21: mol_type = other RNA
tcttgtccagctttattggtt

SEQ ID NO: 1630 - RNA, 21 nt, synthetic construct
  source 1..21: mol_type = other RNA
ttcttgtccagctttattgtt

SEQ ID NO: 1631 - RNA, 21 nt, synthetic construct
  source 1..21: mol_type = other RNA
tttcttgtccagctttatttt

SEQ ID NO: 1632 - RNA, 21 nt, synthetic construct
  source 1..21: mol_type = other RNA
acttcttgtccagctttattt

SEQ ID NO: 1633 - RNA, 21 nt, synthetic construct
  source 1..21: mol_type = other RNA
agcttcttgtccagctttatt

SEQ ID NO: 1634 - RNA, 21 nt, synthetic construct
  source 1..21: mol_type = other RNA
tagcttcttgtccagcttttt

SEQ ID NO: 1635 - RNA, 21 nt, synthetic construct
  source 1..21: mol_type = other RNA
acagcttcttgtccagctttt

SEQ ID NO: 1636 - RNA, 21 nt, synthetic construct
  source 1..21: mol_type = other RNA
agcagcttcttgtccagcttt

SEQ ID NO: 1637 - RNA, 21 nt, synthetic construct
  source 1..21: mol_type = other RNA
tagcagcttcttgtccagctt

SEQ ID NO: 1638 - RNA, 21 nt, synthetic construct
  source 1..21: mol_type = other RNA
atagcagcttcttgtccagtt

SEQ ID NO: 1639 - RNA, 21 nt, synthetic construct
  source 1..21: mol_type = other RNA
tatagcagcttcttgtccatt

SEQ ID NO: 1640 - RNA, 21 nt, synthetic construct
  source 1..21: mol_type = other RNA
tcatagcagcttcttgtcctt

SEQ ID NO: 1641 - RNA, 21 nt, synthetic construct
  source 1..21: mol_type = other RNA
tcactgagaatactgtcccgt

SEQ ID NO: 1642 - RNA, 23 nt, synthetic construct
  source 1..23: mol_type = other RNA
gcactgagaatactgtccctttt

SEQ ID NO: 1643 - RNA, 21 nt, synthetic construct
  source 1..21: mol_type = other RNA
agaatactgtcccttttaatt

SEQ ID NO: 1644 - RNA, 21 nt, synthetic construct
  source 1..21: mol_type = other RNA
actgagaatactgtccctttt

SEQ ID NO: 1645 - RNA, 21 nt, synthetic construct
  source 1..21: mol_type = other RNA
aataggcaggtggacttggtt

SEQ ID NO: 1646 - RNA, 21 nt, synthetic construct
  source 1..21: mol_type = other RNA
aagaacttgtccttaacggtt

SEQ ID NO: 1647 - RNA, 21 nt, synthetic construct
  source 1..21: mol_type = other RNA
aagaagggaggcatcctcgtt

SEQ ID NO: 1648 - RNA, 21 nt, synthetic construct
  source 1..21: mol_type = other RNA
tcactgagaatactgtcccgt

SEQ ID NO: 1649 - RNA, 21 nt, synthetic construct
  source 1..21: mol_type = other RNA
  modified_base 1: mod_base = OTHER; note = t is VPU
tgaatactgtcccttttaatt

SEQ ID NO: 1650 - RNA, 21 nt, synthetic construct
  source 1..21: mol_type = other RNA
  modified_base 1: mod_base = OTHER; note = n is CP1a-U
ngaatactgtcccttttaatt

SEQ ID NO: 1651 - RNA, 21 nt, synthetic construct
  source 1..21: mol_type = other RNA
  modified_base 1: mod_base = OTHER; note = n is CP1a-U
nctgagaatactgtccctttt

SEQ ID NO: 1652 - RNA, 21 nt, synthetic construct
  source 1..21: mol_type = other RNA
  modified_base 1: mod_base = OTHER; note = n is CP1a-U
  modified_base 7: mod_base = OTHER; note = n is PCN-A
nctgagnatactgtccctttt

SEQ ID NO: 1653 - RNA, 21 nt, synthetic construct
  source 1..21: mol_type = other RNA
  modified_base 2: mod_base = OTHER; note = g is dG
  modified_base 5: mod_base = OTHER; note = t is dT
  modified_base 7: mod_base = OTHER; note = c is dC
  modified_base 12: mod_base = OTHER; note = c is dC
tgaatactgtcccttttaatt

SEQ ID NO: 1654 - RNA, 21 nt, synthetic construct
  source 1..21: mol_type = other RNA
tgaatactgtcccttttaatt

SEQ ID NO: 1655 - RNA, 23 nt, synthetic construct
  source 1..23: mol_type = other RNA
  modified_base 1: mod_base = OTHER; note = n is STM1
  modified_base 23: mod_base = OTHER; note = n is STM1
naaaagggacagtattctcagan

SEQ ID NO: 1656 - RNA, 23 nt, synthetic construct
  source 1..23: mol_type = other RNA
  modified_base 1: mod_base = OTHER; note = n is STM1
  modified_base 23: mod_base = OTHER; note = n is STM1
naattaaaagggacagtattcan

SEQ ID NO: 1657 - RNA, 23 nt, synthetic construct
  source 1..23: mol_type = other RNA
  modified_base 1: mod_base = OTHER; note = n is STM1
  modified_base 23: mod_base = OTHER; note = n is STM1
naattaaaagggacagtattcan

SEQ ID NO: 1658 - RNA, 23 nt, synthetic construct
  source 1..23: mol_type = other RNA
  modified_base 1: mod_base = OTHER; note = n is IB
  modified_base 23: mod_base = OTHER; note = n is IB
naattaaaagggacagtattcan

SEQ ID NO: 1659 - RNA, 19 nt, synthetic construct
  source 1..19: mol_type = other RNA
ttaaaagggacagtattca

SEQ ID NO: 1660 - RNA, 23 nt, synthetic construct
  source 1..23: mol_type = other RNA
  modified_base 1: mod_base = OTHER; note = n is IB
  modified_base 23: mod_base = OTHER; note = n is IB
naaaagggacagtattctcagan

SEQ ID NO: 1661 - RNA, 19 nt, synthetic construct
  source 1..19: mol_type = other RNA
aagggacagtattctcaga

SEQ ID NO: 1662 - RNA, 23 nt, synthetic construct
  source 1..23: mol_type = other RNA
  modified_base 1: mod_base = OTHER; note = n is IB
  modified_base 23: mod_base = OTHER; note = n is IB
naaaagggacagtattctcagan

SEQ ID NO: 1663 - RNA, 19 nt, synthetic construct
  source 1..19: mol_type = other RNA
aagggacagtattctcaga

SEQ ID NO: 1664 - DNA, 20 bp, synthetic construct
  source 1..20: mol_type = other DNA
acgtggacatccgcaaagac

SEQ ID NO: 1665 - DNA, 20 bp, synthetic construct
  source 1..20: mol_type = other DNA
tcttcattgtgctgggtgcc

SEQ ID NO: 1666 - DNA, 25 bp, synthetic construct
  source 1..25: mol_type = other DNA
aacacagtgctgtctggcggcacca

SEQ ID NO: 1667 - DNA, 20 bp, synthetic construct
  source 1..20: mol_type = other DNA
tgcctcccttctcagcttca

SEQ ID NO: 1668 - DNA, 20 bp, synthetic construct
  source 1..20: mol_type = other DNA
gggaactgaagccatcggtc

SEQ ID NO: 1669 - DNA, 25 bp, synthetic construct
  source 1..25: mol_type = other DNA
atgaagcacgccaccaagaccgcca

SEQ ID NO: 1670 - DNA, 20 bp, synthetic construct
  source 1..20: mol_type = other DNA
acgtggacatccgcaaagac

SEQ ID NO: 1671 - DNA, 20 bp, synthetic construct
  source 1..20: mol_type = other DNA
tcttcattgtgctgggtgcc

SEQ ID NO: 1672 - DNA, 25 bp, synthetic construct
  source 1..25: mol_type = other DNA
aacacagtgctgtctggcggcacca

SEQ ID NO: 1673 - DNA, 20 bp, synthetic construct
  source 1..20: mol_type = other DNA
tgcctcccttctcagcttca

SEQ ID NO: 1674 - DNA, 20 bp, synthetic construct
  source 1..20: mol_type = other DNA
gggaactgaagccatcggtc

SEQ ID NO: 1675 - DNA, 25 bp, synthetic construct
  source 1..25: mol_type = other DNA
atgaagcacgccaccaagaccgcca

SEQ ID NO: 1676 - DNA, 20 bp, synthetic construct
  source 1..20: mol_type = other DNA
tcaagatcgtcagcaacgcc

SEQ ID NO: 1677 - DNA, 20 bp, synthetic construct
  source 1..20: mol_type = other DNA
acagtcttctgggtggcagt

SEQ ID NO: 1678 - DNA, 25 bp, synthetic construct
  source 1..25: mol_type = other DNA
accaactgcttagcacccctggcca

SEQ ID NO: 1679 - DNA, 20 bp, synthetic construct
  source 1..20: mol_type = other DNA
gcctgcctgctctgttcatc

SEQ ID NO: 1680 - DNA, 21 bp, synthetic construct
  source 1..21: mol_type = other DNA
aagccaagaagggaggtgtcc

SEQ ID NO: 1681 - DNA, 27 bp, synthetic construct
  source 1..27: mol_type = other DNA
ttgttgctgccgtgctgtcactcctgg